European Patent Application EP 4 733 399 A1, published April 29, 2026. Title: 一种无相分离转录因子介导启始阶段重编程使细胞年轻化的方法. Applicant: 深圳菁童生命科学有限公司. The sequence listing filed with the application follows.

SEQUENCE LISTING (65 sequences)

SEQ ID NO: 1 - DNA, 1080 bp, Homo sapiens
  source 1..1080: mol_type = genomic DNA
atggctggccacctggcctctgacttcgccttctctcccccacctggcggcggcggtgacggccccggaggacccgagcctggatgggtggaccctagaacctggctgtcattccagggacctcctggcggacccggcatcggacctggcgtcgggcccggcagcgaggtgtggggcatacctccctgccctcccccctacgagttctgcgggggcatggcctactgtggcccccaggtcggggtcggcctggtgccccagggcggcctcgaaaccagccagcccgagggcgaggctggtgtcggagtggagagcaactccgacggggccagcccagagccatgcaccgtgactcccggcgcagtgaagctggaaaaggagaagctggagcagaatcctgaggagtctcaggacatcaaggcgctccagaaggagctggagcagttcgcgaagctgctgaagcagaagcggatcacgctggggtacacccaggccgacgtcggcctgaccctgggcgtcctgttcggcaaggtgttcagccagaccaccatctgccggttcgaggccctgcagcttagcttcaagaacatgtgcaagctgcgcccacttctgcagaagtgggtggaggaggcggataacaacgagaacctgcaggagatctgcaaggccgagacgctggtgcaggccaggaagcgaaagcggacctccatcgagaaccgcgttcgcgggaacctggagaacctgttcctgcagtgtcccaagcctacactgcagcagatctctcacatagcccagcagctgggcctggagaaggatgtggtgcgagtgtggttctgcaatcggaggcagaagggcaagcgctcttcctccgattacgcccagagggaggacttcgaggcggcggggtcccccttcagcggcggccccgtgtccttccctctggcccccgggccacacttcgggactcccggctacggcagcccacacttcaccgcgctgtacagcagcgtgccattccctgagggggaggccttcccccccgtgagcgtgacgacgctgggcagccccatgcacagcaat

SEQ ID NO: 2 - protein, 360 aa, Homo sapiens
MAGHLASDFAFSPPPGGGGDGPGGPEPGWVDPRTWLSFQGPPGGPGIGPGVGPGSEVWGIPPCPPPYEFCGGMAYCGPQVGVGLVPQGGLETSQPEGEAGVGVESNSDGASPEPCTVTPGAVKLEKEKLEQNPEESQDIKALQKELEQFAKLLKQKRITLGYTQADVGLTLGVLFGKVFSQTTICRFEALQLSFKNMCKLRPLLQKWVEEADNNENLQEICKAETLVQARKRKRTSIENRVRGNLENLFLQCPKPTLQQISHIAQQLGLEKDVVRVWFCNRRQKGKRSSSDYAQREDFEAAGSPFSGGPVSFPLAPGPHFGTPGYGSPHFTALYSSVPFPEGEAFPPVSVTTLGSPMHSN

SEQ ID NO: 3 - DNA, 1080 bp, synthetic construct
  source 1..1080: mol_type = other DNA
atggctggccacctggcctctgccttcgccttctctcccccacctggcggcggcggtgccggccccggaggacccgcccctggatgggtggcccctagaacctggctgtcattccagggacctcctggcggacccggcatcggacctggcgtcgggcccggcagcgccgtgtggggcatacctccctgccctcccccctacgccttctgcgggggcatggcctactgtggcccccaggtcggggtcggcctggtgccccagggcggcctcgccaccagccagcccgccggcgccgctggtgtcggagtggccagcaactccgccggggccagcccagccccatgcaccgtgactcccggcgcagtgaagctggccaaggccaagctggcccagaatcctgccgcctctcaggccatcaaggcgctccagaaggagctggagcagttcgcgaagctgctgaagcagaagcggatcacgctggggtacacccaggccgacgtcggcctgaccctgggcgtcctgttcggcaaggtgttcagccagaccaccatctgccggttcgaggccctgcagcttagcttcaagaacatgtgcaagctgcgcccacttctgcagaagtgggtggaggaggcggataacaacgagaacctgcaggagatctgcaaggccgagacgctggtgcaggccaggaagcgaaagcggacctccatcgagaaccgcgttcgcgggaacctggagaacctgttcctgcagtgtcccaagcctacactgcagcagatctctcacatagcccagcagctgggcctggagaaggatgtggtgcgagtgtggttctgcaatcggaggcagaagggcaagcgctcttcctccgcctacgcccagagggccgccttcgccgcggcggggtcccccttcagcggcggccccgtgtccttccctctggcccccgggccacacttcgggactcccggctacggcagcccacacttcaccgcgctgtacagcagcgtgccattccctgccggggccgccttcccccccgtgagcgtgacgacgctgggcagccccatgcacagcaat

SEQ ID NO: 4 - protein, 360 aa, synthetic construct
MAGHLASAFAFSPPPGGGGAGPGGPAPGWVAPRTWLSFQGPPGGPGIGPGVGPGSAVWGIPPCPPPYAFCGGMAYCGPQVGVGLVPQGGLATSQPAGAAGVGVASNSAGASPAPCTVTPGAVKLAKAKLAQNPAASQAIKALQKELEQFAKLLKQKRITLGYTQADVGLTLGVLFGKVFSQTTICRFEALQLSFKNMCKLRPLLQKWVEEADNNENLQEICKAETLVQARKRKRTSIENRVRGNLENLFLQCPKPTLQQISHIAQQLGLEKDVVRVWFCNRRQKGKRSSSAYAQRAAFAAAGSPFSGGPVSFPLAPGPHFGTPGYGSPHFTALYSSVPFPAGAAFPPVSVTTLGSPMHSN

SEQ ID NO: 5 - protein, 360 aa, synthetic construct
MAGHLASAFAFSPPPGGGGAGPGGPAPGWVAPRTWLSFQGPPGGPGIGPGVGPGSAVWGIPPCPPPYAFCGGMAYCGPQVGVGLVPQGGLATSQPAGAAGVGVASNSAGASPAPCTVTPGAVKLAKAKLAQNPAASQDIKALQKELEQFAKLLKQKRITLGYTQADVGLTLGVLFGKVFSQTTICRFEALQLSFKNMCKLRPLLQKWVEEADNNENLQEICKAETLVQARKRKRTSIENRVRGNLENLFLQCPKPTLQQISHIAQQLGLEKDVVRVWFCNRRQKGKRSSSAYAQRAAFAAAGSPFSGGPVSFPLAPGPHFGTPGYGSPHFTALYSSVPFPAGAAFPPVSVTTLGSPMHSN

SEQ ID NO: 6 - protein, 360 aa, synthetic construct
MAGHLASAFAFSPPPGGGGAGPGGPAPGWVAPRTWLSFQGPPGGPGIGPGVGPGSAVWGIPPCPPPYAFCGGMAYCGPQVGVGLVPQGGLATSQPAGAAGVGVASNSAGASPAPCTVTPGAVKLAKAKLAQNPAASQDIKALQKELEQFAKLLKQKRITLGYTQADVGLTLGVLFGKVFSQTTICRFEALQLSFKNMCKLRPLLQKWVEEADNNENLQEICKAETLVQARKRKRTSIENRVRGNLENLFLQCPKPTLQQISHIAQQLGLEKDVVRVWFCNRRQKGKRSSSDYAQRAAFAAAGSPFSGGPVSFPLAPGPHFGTPGYGSPHFTALYSSVPFPAGAAFPPVSVTTLGSPMHSN

SEQ ID NO: 7 - protein, 360 aa, synthetic construct
MAGHLASAFAFSPPPGGGGAGPGGPAPGWVAPRTWLSFQGPPGGPGIGPGVGPGSAVWGIPPCPPPYAFCGGMAYCGPQVGVGLVPQGGLATSQPAGAAGVGVASNSAGASPAPCTVTPGAVKLAKAKLAQNPAASQAIKALQKALEQFAKLLKQKRITLGYTQADVGLTLGVLFGKVFSQTTICRFEALQLSFKNMCKLRPLLQKWVEEADNNENLQEICKAETLVQARKRKRTSIENRVRGNLENLFLQCPKPTLQQISHIAQQLGLEKDVVRVWFCNRRQKGKRSSSAYAQRAAFAAAGSPFSGGPVSFPLAPGPHFGTPGYGSPHFTALYSSVPFPAGAAFPPVSVTTLGSPMHSN

SEQ ID NO: 8 - protein, 360 aa, synthetic construct
MAGHLASAFAFSPPPGGGGAGPGGPAPGWVAPRTWLSFQGPPGGPGIGPGVGPGSAVWGIPPCPPPYAFCGGMAYCGPQVGVGLVPQGGLATSQPAGAAGVGVASNSAGASPAPCTVTPGAVKLAKAKLAQNPAASQAIKALQKELEQFAKLLKQKRITLGYTQADVGLTLGVLFGKVFSQTTICRFEALQLSFKNMCKLRPLLQKWVEEADNNENLQEICKAETLVQARKRKRTSIENRVRGNLENLFLQCPKPTLQQISHIAQQLGLEKDVVRVWFCNRRQKGKRSSSDYAQRAAFAAAGSPFSGGPVSFPLAPGPHFGTPGYGSPHFTALYSSVPFPAGAAFPPVSVTTLGSPMHSN

SEQ ID NO: 9 - protein, 360 aa, synthetic construct
MAGHLASAFAFSPPPGGGGAGPGGPAPGWVAPRTWLSFQGPPGGPGIGPGVGPGSAVWGIPPCPPPYAFCGGMAYCGPQVGVGLVPQGGLATSQPAGAAGVGVASNSAGASPAPCTVTPGAVKLAKAKLAQNPAASQAIKALQKELEQFAKLLKQKRITLGYTQADVGLTLGVLFGKVFSQTTICRFEALQLSFKNMCKLRPLLQKWVEEADNNENLQEICKAETLVQARKRKRTSIENRVRGNLENLFLQCPKPTLQQISHIAQQLGLEKAVVRVWFCNRRQKGKRSSSAYAQRAAFAAAGSPFSGGPVSFPLAPGPHFGTPGYGSPHFTALYSSVPFPAGAAFPPVSVTTLGSPMHSN

SEQ ID NO: 10 - protein, 360 aa, synthetic construct
MAGHLASAFAFSPPPGGGGAGPGGPAPGWVAPRTWLSFQGPPGGPGIGPGVGPGSAVWGIPPCPPPYAFCGGMAYCGPQVGVGLVPQGGLATSQPAGAAGVGVASNSAGASPAPCTVTPGAVKLAKAKLAQNPAASQAIKALQKALEQFAKLLKQKRITLGYTQADVGLTLGVLFGKVFSQTTICRFEALQLSFKNMCKLRPLLQKWVEEADNNENLQEICKAETLVQARKRKRTSIENRVRGNLENLFLQCPKPTLQQISHIAQQLGLEKAVVRVWFCNRRQKGKRSSSAYAQRAAFAAAGSPFSGGPVSFPLAPGPHFGTPGYGSPHFTALYSSVPFPAGAAFPPVSVTTLGSPMHSN

SEQ ID NO: 11 - DNA, 1317 bp, Homo sapiens
  source 1..1317: mol_type = genomic DNA
atgcccctgaatgtgtccttcaccaaccgcaactatgatctggactatgactctgtgcagccttacttctactgcgatgaggaggagaacttctaccagcagcagcagcagagcgaactgcagccacccgccccatccgaggatatctggaagaagttcgagctgctgccgacccctcctctcagcccctccaggaggagcgggctgtgcagtcccagctacgtggctgtgacccccttctccctgcgcggcgacaacgacggcgggggggggagcttcagcaccgctgaccagctggagatggtcaccgagctgctgggtggcgacatggtcaaccagagcttcatctgcgaccctgatgatgagacattcatcaagaacatcatcatccaggactgcatgtggtccggcttctcggccgctgccaagctggtcagcgagaagctggccagctaccaggccgcccggaaggattccgggtcgcctaaccccgccaggggccacagcgtctgctccacgagcagcctgtacctgcaggatctgagcgccgccgccagcgagtgcatagatccttcagtggtgttcccatacccactgaacgacagcagctctcccaagagctgcgcctcgcaggacagcagcgccttcagcccctcgtccgactcgctgctgtccagcaccgagtcgagcccccagggctctcctgagcccctggtgctgcacgaggagacccctcctaccacctcctcggactccgaggaggagcaggaggatgaggaagagatcgacgtggtcagcgtggagaagcgccaggctcctggcaagcgcagcgagtctggcagcccctccgccgggggccacagcaagcccccgcacagcccgctggtgctgaagcggtgtcacgtgagcacccaccagcataactatgctgcgcctccttccaccaggaaggactaccccgctgccaagcgggtgaagctggatagcgtccgggtgctgaggcagatcagcaataaccgtaagtgcacctcccccaggagcagtgacacagaggagaacgtgaagaggcggactcacaacgttctggagcgccagcgccggaacgagctgaagcggtccttcttcgctctgagggaccagatcccagagctggagaacaatgagaaggcaccgaaggtggtcatcctgaagaaggccaccgcgtatatcctgagcgtgcaggctgaggagcagaagctgatcagcgaggaggacttgctgaggaagcggcgcgagcagctgaaacacaagctggagcagctgcgaaacagctgcgcc

SEQ ID NO: 12 - protein, 454 aa, Homo sapiens
MDFFRVVENQQPPATMPLNVSFTNRNYDLDYDSVQPYFYCDEEENFYQQQQQSELQPPAPSEDIWKKFELLPTPPLSPSRRSGLCSPSYVAVTPFSLRGDNDGGGGSFSTADQLEMVTELLGGDMVNQSFICDPDDETFIKNIIIQDCMWSGFSAAAKLVSEKLASYQAARKDSGSPNPARGHSVCSTSSLYLQDLSAAASECIDPSVVFPYPLNDSSSPKSCASQDSSAFSPSSDSLLSSTESSPQGSPEPLVLHEETPPTTSSDSEEEQEDEEEIDVVSVEKRQAPGKRSESGSPSAGGHSKPPHSPLVLKRCHVSTHQHNYAAPPSTRKDYPAAKRVKLDSVRVLRQISNNRKCTSPRSSDTEENVKRRTHNVLERQRRNELKRSFFALRDQIPELENNEKAPKVVILKKATAYILSVQAEEQKLISEEDLLRKRREQLKHKLEQLRNSCA

SEQ ID NO: 13 - DNA, 1317 bp, synthetic construct
  source 1..1317: mol_type = other DNA
atgcccctgaatgtgtccttcaccaaccgcaactatgatctggactatgactctgtgcagccttacttctactgcgatgaggaggagaacttctaccagcagcagcagcagagcgaactgcagccacccgccccatccgaggatatctggaggaggttcgagctgctgccgacccctcctctcagcccctccaggaggagcgggctgtgcagtcccagctacgtggctgtgacccccttctccctgcgcggcgacaacgacggcgggggggggagcttcagcaccgctgaccagctggagatggtcaccgagctgctgggtggcgacatggtcaaccagagcttcatctgcgaccctgatgatgagacattcatcaggaacatcatcatccaggactgcatgtggtccggcttctcggccgctgccaggctggtcagcgagaggctggccagctaccaggccgcccggagggattccgggtcgcctaaccccgccaggggccacagcgtctgctccacgagcagcctgtacctgcaggatctgagcgccgccgccagcgagtgcatagatccttcagtggtgttcccatacccactgaacgacagcagctctcccaggagctgcgcctcgcaggacagcagcgccttcagcccctcgtccgactcgctgctgtccagcaccgagtcgagcccccagggctctcctgagcccctggtgctgcacgaggagacccctcctaccacctcctcggactccgaggaggagcaggaggatgaggaagagatcgacgtggtcagcgtggagaggcgccaggctcctggcaggcgcagcgagtctggcagcccctccgccgggggccacagcaggcccccgcacagcccgctggtgctgaggcggtgtcacgtgagcacccaccagcataactatgctgcgcctccttccaccaggagggactaccccgctgccaggcgggtgaggctggatagcgtccgggtgctgaggcagatcagcaataaccgtaggtgcacctcccccaggagcagtgacacagaggagaacgtgaggaggcggactcacaacgttctggagcgccagcgccggaacgagctgaggcggtccttcttcgctctgagggaccagatcccagagctggagaacaatgagagggcaccgagggtggtcatcctgaggagggccaccgcgtatatcctgagcgtgcaggctgaggagcagaggctgatcagcgaggaggacttgctgaggaggcggcgcgagcagctgaggcacaggctggagcagctgcgaaacagctgcgcc

SEQ ID NO: 14 - protein, 439 aa, synthetic construct
MPLNVSFTNRNYDLDYDSVQPYFYCDEEENFYQQQQQSELQPPAPSEDIWRRFELLPTPPLSPSRRSGLCSPSYVAVTPFSLRGDNDGGGGSFSTADQLEMVTELLGGDMVNQSFICDPDDETFIRNIIIQDCMWSGFSAAARLVSERLASYQAARRDSGSPNPARGHSVCSTSSLYLQDLSAAASECIDPSVVFPYPLNDSSSPRSCASQDSSAFSPSSDSLLSSTESSPQGSPEPLVLHEETPPTTSSDSEEEQEDEEEIDVVSVERRQAPGRRSESGSPSAGGHSRPPHSPLVLRRCHVSTHQHNYAAPPSTRRDYPAARRVRLDSVRVLRQISNNRRCTSPRSSDTEENVRRRTHNVLERQRRNELRRSFFALRDQIPELENNERAPRVVILRRATAYILSVQAEEQRLISEEDLLRRRREQLRHRLEQLRNSCA

SEQ ID NO: 15 - protein, 439 aa, synthetic construct
MPLNVSFTNRNYDLDYDSVQPYFYCDEEENFYQQQQQSELQPPAPSEDIWKKFELLPTPPLSPSRRSGLCSPSYVAVTPFSLRGDNDGGGGSFSTADQLEMVTELLGGDMVNQSFICDPDDETFIKNIIIQDCMWSGFSAAAKLVSEKLASYQAARKDSGSPNPARGHSVCSTSSLYLQDLSAAASECIDPSVVFPYPLNDSSSPKSCASQDSSAFSPSSDSLLSSTESSPQGSPEPLVLHEETPPTTSSDSEEEQEDEEEIDVVSVEKRQAPGKRSESGSPSAGGHSKPPHSPLVLKRCHVSTHQHNYAAPPSTRKDYPAAKRVKLDSVRVLRQISNNRKCTSPRSSDTEENVKRRTHNVLERQRRNELKRSFFALRDQIPELENNEKAPKVVILKKATAYILSVQAEEQKLISEEDLLRKRREQLKHKLEQLRNSCA

SEQ ID NO: 16 - protein, 439 aa, synthetic construct
MPLNVSFTNRNYDLDYDSVQPYFYCDEEENFYQQQQQSELQPPAPSEDIWRRFELLPTPPLSPSKKSGLCSPSYVAVTPFSLRGDNDGGGGSFSTADQLEMVTELLGGDMVNQSFICDPDDETFIRNIIIQDCMWSGFSAAARLVSERLASYQAARRDSGSPNPARGHSVCSTSSLYLQDLSAAASECIDPSVVFPYPLNDSSSPRSCASQDSSAFSPSSDSLLSSTESSPQGSPEPLVLHEETPPTTSSDSEEEQEDEEEIDVVSVERRQAPGRRSESGSPSAGGHSRPPHSPLVLRRCHVSTHQHNYAAPPSTRRDYPAARRVRLDSVRVLRQISNNRRCTSPRSSDTEENVRRRTHNVLERQRRNELRRSFFALRDQIPELENNERAPRVVILRRATAYILSVQAEEQRLISEEDLLRRRREQLRHRLEQLRNSCA

SEQ ID NO: 17 - protein, 439 aa, synthetic construct
MPLNVSFTNRNYDLDYDSVQPYFYCDEEENFYQQQQQSELQPPAPSEDIWRRFELLPTPPLSPSRRSGLCSPSYVAVTPFSLRGDNDGGGGSFSTADQLEMVTELLGGDMVNQSFICDPDDETFIRNIIIQDCMWSGFSAAARLVSERLASYQAARRDSGSPNPARGHSVCSTSSLYLQDLSAAASECIDPSVVFPYPLNDSSSPRSCASQDSSAFSPSSDSLLSSTESSPQGSPEPLVLHEETPPTTSSDSEEEQEDEEEIDVVSVERRQAPGRRSESGSPSAGGHSRPPHSPLVLKKCHVSTHQHNYAAPPSTRRDYPAARRVRLDSVRVLRQISNNRRCTSPRSSDTEENVRRRTHNVLERQRRNELRRSFFALRDQIPELENNERAPRVVILRRATAYILSVQAEEQRLISEEDLLRRRREQLRHRLEQLRNSCA

SEQ ID NO: 18 - protein, 439 aa, synthetic construct
MPLNVSFTNRNYDLDYDSVQPYFYCDEEENFYQQQQQSELQPPAPSEDIWRRFELLPTPPLSPSRRSGLCSPSYVAVTPFSLRGDNDGGGGSFSTADQLEMVTELLGGDMVNQSFICDPDDETFIRNIIIQDCMWSGFSAAARLVSERLASYQAARRDSGSPNPARGHSVCSTSSLYLQDLSAAASECIDPSVVFPYPLNDSSSPRSCASQDSSAFSPSSDSLLSSTESSPQGSPEPLVLHEETPPTTSSDSEEEQEDEEEIDVVSVEKRQAPGRRSESGSPSAGGHSRPPHSPLVLRRCHVSTHQHNYAAPPSTRRDYPAARRVRLDSVRVLRQISNNRRCTSPRSSDTEENVRRRTHNVLERQRRNELRRSFFALRDQIPELENNERAPRVVILRRATAYILSVQAEEQRLISEEDLLRRRREQLRHRLEQLRNSCA

SEQ ID NO: 19 - protein, 439 aa, synthetic construct
MPLNVSFTNRNYDLDYDSVQPYFYCDEEENFYQQQQQSELQPPAPSEDIWKRFELLPTPPLSPSRRSGLCSPSYVAVTPFSLRGDNDGGGGSFSTADQLEMVTELLGGDMVNQSFICDPDDETFIRNIIIQDCMWSGFSAAARLVSERLASYQAARRDSGSPNPARGHSVCSTSSLYLQDLSAAASECIDPSVVFPYPLNDSSSPRSCASQDSSAFSPSSDSLLSSTESSPQGSPEPLVLHEETPPTTSSDSEEEQEDEEEIDVVSVERRQAPGRRSESGSPSAGGHSKPPHSPLVLRRCHVSTHQHNYAAPPSTRRDYPAARRVRLDSVRVLRQISNNRRCTSPRSSDTEENVRRRTHNVLERQRRNELRRSFFALRDQIPELENNERAPRVVILRRATAYILSVQAEEQRLISEEDLLKRRREQLRHRLEQLRNSCA

SEQ ID NO: 20 - protein, 439 aa, synthetic construct
MPLNVSFTNRNYDLDYDSVQPYFYCDEEENFYQQQQQSELQPPAPSEDIWRRFELLPTPPLSPSRRSGLCSPSYVAVTPFSLRGDNDGGGGSFSTADQLEMVTELLGGDMVNQSFICDPDDETFIKNIIIQDCMWSGFSAAAKLVSEKLASYQAARKDSGSPNPARGHSVCSTSSLYLQDLSAAASECIDPSVVFPYPLNDSSSPKSCASQDSSAFSPSSDSLLSSTESSPQGSPEPLVLHEETPPTTSSDSEEEQEDEEEIDVVSVEKRQAPGRRSESGSPSAGGHSRPPHSPLVLKRCHVSTHQHNYAAPPSTRKDYPAAKRVKLDSVRVLRQISNNRKCTSPRSSDTEENVKRRTHNVLERQRRNELKRSFFALRDQIPELENNEKAPKVVILKKATAYILSVQAEEQKLISEEDLLRKRREQLKHKLEQLRNSCA

SEQ ID NO: 21 - DNA, 1410 bp, synthetic construct
  source 1..1410: mol_type = other DNA
atggccgtgtccgacgccctgctgccctcattcagcaccttcgcctcaggccccgctggcagagaaaagacactgagacaggctggagcccctaacaaccgctggcgcgaggagctgagtcacatgaaacgcctgccccctgtcctgcctgggcggccatacgacctggccgccgccacggtggccaccgacctggagtcaggcggggccggagccgcctgtggcggctccaacctggcgcccctgccccgcagggagactgaggagttcaacgatctgctggatctggacttcatcctcagtaactctctgacccaccccccagagagtgttgctgctaccgtgagcagcagcgccagcgcgagctctagcagcagccctagcagctccgggcctgccagtgcccccagcacctgcagcttcacctaccccatcagggccggtaacgaccctggtgtggcccccggcggcaccgggggcggactcctgtacggccgggagtccgcccccccgcccaccgcccccttcaacctggcggacatcaacgatgtgagcccctccgggggcttcgtcgccgagctgctgcggccagagctcgaccctgtgtacatccccccacagcagccgcagcccccgggcggcggcctgatggggaagttcgtgctcaaggccagcctgagcgcacccggctctgagtacggaagcccctccgtgatcagtgtgagcaagggaagccccgacggctcacaccccgtggttgtggccccctacaacggcgggccgccacggacctgccccaagatcaagcaggaggcagtgagcagctgcacccatctgggtgcggggccaccactgtccaacggccaccgccccgctgcccatgacttccctctgggcaggcagctgcccagcaggaccacccctacgctgggcctggaggaggtcctgtcctccagggactgccacccggccctgcccctgcccccggggttccacccccaccccggacccaactaccccagcttcctgcctgaccagatgcagccgcaggttccgcccctgcattaccaggagctgatgcccccgggcagctgcatgcccgaggagcctaagcctaagcggggccggcgcagctggccccgcaagcggaccgccacccacacttgcgattacgccgggtgcggcaagacctacacaaagagttcgcacctgaaggcccacctgcgaactcacacgggcgagaagccctaccactgcgactgggacgggtgcggctggaagttcgcccggtccgatgagctgacccggcactatcggaagcacaccgggcacaggcccttccagtgccagaagtgtgaccgggccttcagccggtcagaccatctggcactgcacatgaagcgccacttc

SEQ ID NO: 22 - protein, 470 aa, synthetic construct
MAVSDALLPSFSTFASGPAGREKTLRQAGAPNNRWREELSHMKRLPPVLPGRPYDLAAATVATDLESGGAGAACGGSNLAPLPRRETEEFNDLLDLDFILSNSLTHPPESVAATVSSSASASSSSSPSSSGPASAPSTCSFTYPIRAGNDPGVAPGGTGGGLLYGRESAPPPTAPFNLADINDVSPSGGFVAELLRPELDPVYIPPQQPQPPGGGLMGKFVLKASLSAPGSEYGSPSVISVSKGSPDGSHPVVVAPYNGGPPRTCPKIKQEAVSSCTHLGAGPPLSNGHRPAAHDFPLGRQLPSRTTPTLGLEEVLSSRDCHPALPLPPGFHPHPGPNYPSFLPDQMQPQVPPLHYQELMPPGSCMPEEPKPKRGRRSWPRKRTATHTCDYAGCGKTYTKSSHLKAHLRTHTGEKPYHCDWDGCGWKFARSDELTRHYRKHTGHRPFQCQKCDRAFSRSDHLALHMKRHF

SEQ ID NO: 23 - DNA, 954 bp, Homo sapiens
  source 1..954: mol_type = genomic DNA
atgtacaacatgatggagacagagctgaagccccccgggcctcagcagaccagcggcggcggcgggggcaactccaccgccgccgctgctgggggcaaccagaagaacagccccgatagggtgaagcgccctatgaacgccttcatggtgtggtcccgcggccagcgccgtaagatggctcaggagaaccctaagatgcacaactccgagatcagcaagcggctgggcgcggagtggaagctgctgtcggagaccgagaagcggccattcatcgacgaggccaagaggcttcgtgccctgcacatgaaggagcatcctgactacaagtaccggccccgccggaagaccaagacactgatgaagaaggacaagtacaccttgcctgggggcctgctggcccccgggggcaactccatggcttccggcgtgggcgtgggagccggtctaggcgctggcgtgaaccagcgcatggactcctacgctcacatgaacggctggagcaacgggtcctacagcatgatgcaggaccagttgggctacccccagcaccctgggctgaacgcccatggggctgcccagatgcagcccatgcatcggtacgacgtgagtgccctgcagtacaactccatgacatctagccagacctacatgaacgggagtcccacctacagcatgagctatagccagcaggggaccccaggcatggccctggggtccatgggctccgtggtgaagtcggaggccagctcctcacctcccgtggtgacaagctcctcccacagccgggccccctgccaggctggggatctgagggacatgatctccatgtacctcccgggcgccgaggtgcccgagcctgctgctcccagcaggctgcatatgagccagcattaccagtccgggcccgtgcccggcactgccatcaatgggacactgccactgtcccatatgtga

SEQ ID NO: 24 - protein, 317 aa, Homo sapiens
MYNMMETELKPPGPQQTSGGGGGNSTAAAAGGNQKNSPDRVKRPMNAFMVWSRGQRRKMAQENPKMHNSEISKRLGAEWKLLSETEKRPFIDEAKRLRALHMKEHPDYKYRPRRKTKTLMKKDKYTLPGGLLAPGGNSMASGVGVGAGLGAGVNQRMDSYAHMNGWSNGSYSMMQDQLGYPQHPGLNAHGAAQMQPMHRYDVSALQYNSMTSSQTYMNGSPTYSMSYSQQGTPGMALGSMGSVVKSEASSSPPVVTSSSHSRAPCQAGDLRDMISMYLPGAEVPEPAAPSRLHMSQHYQSGPVPGTAINGTLPLSHM

SEQ ID NO: 25 - DNA, 66 bp, synthetic construct
  source 1..66: mol_type = other DNA
ggaagcggagccacgaacttctctctgttaaagcaagcaggagatgttgaagaaaaccccgggcct

SEQ ID NO: 26 - DNA, 63 bp, synthetic construct
  source 1..63: mol_type = other DNA
ggaagcggagagggcaggggaagtcttctaacatgcggggacgtggaggaaaatcccggcccc

SEQ ID NO: 27 - DNA, 69 bp, synthetic construct
  source 1..69: mol_type = other DNA
ggaagcggacagtgtactaattatgctctcttgaaattggctggagatgttgagagcaacccaggtccc

SEQ ID NO: 28 - DNA, 4959 bp, synthetic construct
  source 1..4959: mol_type = other DNA
atggctggccacctggcctctgccttcgccttctctcccccacctggcggcggcggtgccggccccggaggacccgcccctggatgggtggcccctagaacctggctgtcattccagggacctcctggcggacccggcatcggacctggcgtcgggcccggcagcgccgtgtggggcatacctccctgccctcccccctacgccttctgcgggggcatggcctactgtggcccccaggtcggggtcggcctggtgccccagggcggcctcgccaccagccagcccgccggcgccgctggtgtcggagtggccagcaactccgccggggccagcccagccccatgcaccgtgactcccggcgcagtgaagctggccaaggccaagctggcccagaatcctgccgcctctcaggccatcaaggcgctccagaaggagctggagcagttcgcgaagctgctgaagcagaagcggatcacgctggggtacacccaggccgacgtcggcctgaccctgggcgtcctgttcggcaaggtgttcagccagaccaccatctgccggttcgaggccctgcagcttagcttcaagaacatgtgcaagctgcgcccacttctgcagaagtgggtggaggaggcggataacaacgagaacctgcaggagatctgcaaggccgagacgctggtgcaggccaggaagcgaaagcggacctccatcgagaaccgcgttcgcgggaacctggagaacctgttcctgcagtgtcccaagcctacactgcagcagatctctcacatagcccagcagctgggcctggagaaggatgtggtgcgagtgtggttctgcaatcggaggcagaagggcaagcgctcttcctccgcctacgcccagagggccgccttcgccgcggcggggtcccccttcagcggcggccccgtgtccttccctctggcccccgggccacacttcgggactcccggctacggcagcccacacttcaccgcgctgtacagcagcgtgccattccctgccggggccgccttcccccccgtgagcgtgacgacgctgggcagccccatgcacagcaatggaagcggagccacgaacttctctctgttaaagcaagcaggagatgttgaagaaaaccccgggcctatggccgtgtccgacgccctgctgccctcattcagcaccttcgcctcaggccccgctggcagagaaaagacactgagacaggctggagcccctaacaaccgctggcgcgaggagctgagtcacatgaaacgcctgccccctgtcctgcctgggcggccatacgacctggccgccgccacggtggccaccgacctggagtcaggcggggccggagccgcctgtggcggctccaacctggcgcccctgccccgcagggagactgaggagttcaacgatctgctggatctggacttcatcctcagtaactctctgacccaccccccagagagtgttgctgctaccgtgagcagcagcgccagcgcgagctctagcagcagccctagcagctccgggcctgccagtgcccccagcacctgcagcttcacctaccccatcagggccggtaacgaccctggtgtggcccccggcggcaccgggggcggactcctgtacggccgggagtccgcccccccgcccaccgcccccttcaacctggcggacatcaacgatgtgagcccctccgggggcttcgtcgccgagctgctgcggccagagctcgaccctgtgtacatccccccacagcagccgcagcccccgggcggcggcctgatggggaagttcgtgctcaaggccagcctgagcgcacccggctctgagtacggaagcccctccgtgatcagtgtgagcaagggaagccccgacggctcacaccccgtggttgtggccccctacaacggcgggccgccacggacctgccccaagatcaagcaggaggcagtgagcagctgcacccatctgggtgcggggccaccactgtccaacggccaccgccccgctgcccatgacttccctctgggcaggcagctgcccagcaggaccacccctacgctgggcctggaggaggtcctgtcctccagggactgccacccggccctgcccctgcccccggggttccacccccaccccggacccaactaccccagcttcctgcctgaccagatgcagccgcaggttccgcccctgcattaccaggagctgatgcccccgggcagctgcatgcccgaggagcctaagcctaagcggggccggcgcagctggccccgcaagcggaccgccacccacacttgcgattacgccgggtgcggcaagacctacacaaagagttcgcacctgaaggcccacctgcgaactcacacgggcgagaagccctaccactgcgactgggacgggtgcggctggaagttcgcccggtccgatgagctgacccggcactatcggaagcacaccgggcacaggcccttccagtgccagaagtgtgaccgggccttcagccggtcagaccatctggcactgcacatgaagcgccacttcggaagcggagagggcaggggaagtcttctaacatgcggggacgtggaggaaaatcccggccccatgcccctgaatgtgtccttcaccaaccgcaactatgatctggactatgactctgtgcagccttacttctactgcgatgaggaggagaacttctaccagcagcagcagcagagcgaactgcagccacccgccccatccgaggatatctggaggaggttcgagctgctgccgacccctcctctcagcccctccaggaggagcgggctgtgcagtcccagctacgtggctgtgacccccttctccctgcgcggcgacaacgacggcgggggggggagcttcagcaccgctgaccagctggagatggtcaccgagctgctgggtggcgacatggtcaaccagagcttcatctgcgaccctgatgatgagacattcatcaggaacatcatcatccaggactgcatgtggtccggcttctcggccgctgccaggctggtcagcgagaggctggccagctaccaggccgcccggagggattccgggtcgcctaaccccgccaggggccacagcgtctgctccacgagcagcctgtacctgcaggatctgagcgccgccgccagcgagtgcatagatccttcagtggtgttcccatacccactgaacgacagcagctctcccaggagctgcgcctcgcaggacagcagcgccttcagcccctcgtccgactcgctgctgtccagcaccgagtcgagcccccagggctctcctgagcccctggtgctgcacgaggagacccctcctaccacctcctcggactccgaggaggagcaggaggatgaggaagagatcgacgtggtcagcgtggagaggcgccaggctcctggcaggcgcagcgagtctggcagcccctccgccgggggccacagcaggcccccgcacagcccgctggtgctgaggcggtgtcacgtgagcacccaccagcataactatgctgcgcctccttccaccaggagggactaccccgctgccaggcgggtgaggctggatagcgtccgggtgctgaggcagatcagcaataaccgtaggtgcacctcccccaggagcagtgacacagaggagaacgtgaggaggcggactcacaacgttctggagcgccagcgccggaacgagctgaggcggtccttcttcgctctgagggaccagatcccagagctggagaacaatgagagggcaccgagggtggtcatcctgaggagggccaccgcgtatatcctgagcgtgcaggctgaggagcagaggctgatcagcgaggaggacttgctgaggaggcggcgcgagcagctgaggcacaggctggagcagctgcgaaacagctgcgccggaagcggacagtgtactaattatgctctcttgaaattggctggagatgttgagagcaacccaggtcccatgtacaacatgatggagacagagctgaagccccccgggcctcagcagaccagcggcggcggcgggggcaactccaccgccgccgctgctgggggcaaccagaagaacagccccgatagggtgaagcgccctatgaacgccttcatggtgtggtcccgcggccagcgccgtaagatggctcaggagaaccctaagatgcacaactccgagatcagcaagcggctgggcgcggagtggaagctgctgtcggagaccgagaagcggccattcatcgacgaggccaagaggcttcgtgccctgcacatgaaggagcatcctgactacaagtaccggccccgccggaagaccaagacactgatgaagaaggacaagtacaccttgcctgggggcctgctggcccccgggggcaactccatggcttccggcgtgggcgtgggagccggtctaggcgctggcgtgaaccagcgcatggactcctacgctcacatgaacggctggagcaacgggtcctacagcatgatgcaggaccagttgggctacccccagcaccctgggctgaacgcccatggggctgcccagatgcagcccatgcatcggtacgacgtgagtgccctgcagtacaactccatgacatctagccagacctacatgaacgggagtcccacctacagcatgagctatagccagcaggggaccccaggcatggccctggggtccatgggctccgtggtgaagtcggaggccagctcctcacctcccgtggtgacaagctcctcccacagccgggccccctgccaggctggggatctgagggacatgatctccatgtacctcccgggcgccgaggtgcccgagcctgctgctcccagcaggctgcatatgagccagcattaccagtccgggcccgtgcccggcactgccatcaatgggacactgccactgtcccatatgtga

SEQ ID NO: 29 - DNA, 4959 bp, synthetic construct
  source 1..4959: mol_type = other DNA
atggctggccacctggcctctgacttcgccttctctcccccacctggcggcggcggtgacggccccggaggacccgagcctggatgggtggaccctagaacctggctgtcattccagggacctcctggcggacccggcatcggacctggcgtcgggcccggcagcgaggtgtggggcatacctccctgccctcccccctacgagttctgcgggggcatggcctactgtggcccccaggtcggggtcggcctggtgccccagggcggcctcgaaaccagccagcccgagggcgaggctggtgtcggagtggagagcaactccgacggggccagcccagagccatgcaccgtgactcccggcgcagtgaagctggaaaaggagaagctggagcagaatcctgaggagtctcaggacatcaaggcgctccagaaggagctggagcagttcgcgaagctgctgaagcagaagcggatcacgctggggtacacccaggccgacgtcggcctgaccctgggcgtcctgttcggcaaggtgttcagccagaccaccatctgccggttcgaggccctgcagcttagcttcaagaacatgtgcaagctgcgcccacttctgcagaagtgggtggaggaggcggataacaacgagaacctgcaggagatctgcaaggccgagacgctggtgcaggccaggaagcgaaagcggacctccatcgagaaccgcgttcgcgggaacctggagaacctgttcctgcagtgtcccaagcctacactgcagcagatctctcacatagcccagcagctgggcctggagaaggatgtggtgcgagtgtggttctgcaatcggaggcagaagggcaagcgctcttcctccgattacgcccagagggaggacttcgaggcggcggggtcccccttcagcggcggccccgtgtccttccctctggcccccgggccacacttcgggactcccggctacggcagcccacacttcaccgcgctgtacagcagcgtgccattccctgagggggaggccttcccccccgtgagcgtgacgacgctgggcagccccatgcacagcaatggaagcggagccacgaacttctctctgttaaagcaagcaggagatgttgaagaaaaccccgggcctatggccgtgtccgacgccctgctgccctcattcagcaccttcgcctcaggccccgctggcagagaaaagacactgagacaggctggagcccctaacaaccgctggcgcgaggagctgagtcacatgaaacgcctgccccctgtcctgcctgggcggccatacgacctggccgccgccacggtggccaccgacctggagtcaggcggggccggagccgcctgtggcggctccaacctggcgcccctgccccgcagggagactgaggagttcaacgatctgctggatctggacttcatcctcagtaactctctgacccaccccccagagagtgttgctgctaccgtgagcagcagcgccagcgcgagctctagcagcagccctagcagctccgggcctgccagtgcccccagcacctgcagcttcacctaccccatcagggccggtaacgaccctggtgtggcccccggcggcaccgggggcggactcctgtacggccgggagtccgcccccccgcccaccgcccccttcaacctggcggacatcaacgatgtgagcccctccgggggcttcgtcgccgagctgctgcggccagagctcgaccctgtgtacatccccccacagcagccgcagcccccgggcggcggcctgatggggaagttcgtgctcaaggccagcctgagcgcacccggctctgagtacggaagcccctccgtgatcagtgtgagcaagggaagccccgacggctcacaccccgtggttgtggccccctacaacggcgggccgccacggacctgccccaagatcaagcaggaggcagtgagcagctgcacccatctgggtgcggggccaccactgtccaacggccaccgccccgctgcccatgacttccctctgggcaggcagctgcccagcaggaccacccctacgctgggcctggaggaggtcctgtcctccagggactgccacccggccctgcccctgcccccggggttccacccccaccccggacccaactaccccagcttcctgcctgaccagatgcagccgcaggttccgcccctgcattaccaggagctgatgcccccgggcagctgcatgcccgaggagcctaagcctaagcggggccggcgcagctggccccgcaagcggaccgccacccacacttgcgattacgccgggtgcggcaagacctacacaaagagttcgcacctgaaggcccacctgcgaactcacacgggcgagaagccctaccactgcgactgggacgggtgcggctggaagttcgcccggtccgatgagctgacccggcactatcggaagcacaccgggcacaggcccttccagtgccagaagtgtgaccgggccttcagccggtcagaccatctggcactgcacatgaagcgccacttcggaagcggagagggcaggggaagtcttctaacatgcggggacgtggaggaaaatcccggccccatgcccctgaatgtgtccttcaccaaccgcaactatgatctggactatgactctgtgcagccttacttctactgcgatgaggaggagaacttctaccagcagcagcagcagagcgaactgcagccacccgccccatccgaggatatctggaagaagttcgagctgctgccgacccctcctctcagcccctccaggaggagcgggctgtgcagtcccagctacgtggctgtgacccccttctccctgcgcggcgacaacgacggcgggggggggagcttcagcaccgctgaccagctggagatggtcaccgagctgctgggtggcgacatggtcaaccagagcttcatctgcgaccctgatgatgagacattcatcaagaacatcatcatccaggactgcatgtggtccggcttctcggccgctgccaagctggtcagcgagaagctggccagctaccaggccgcccggaaggattccgggtcgcctaaccccgccaggggccacagcgtctgctccacgagcagcctgtacctgcaggatctgagcgccgccgccagcgagtgcatagatccttcagtggtgttcccatacccactgaacgacagcagctctcccaagagctgcgcctcgcaggacagcagcgccttcagcccctcgtccgactcgctgctgtccagcaccgagtcgagcccccagggctctcctgagcccctggtgctgcacgaggagacccctcctaccacctcctcggactccgaggaggagcaggaggatgaggaagagatcgacgtggtcagcgtggagaagcgccaggctcctggcaagcgcagcgagtctggcagcccctccgccgggggccacagcaagcccccgcacagcccgctggtgctgaagcggtgtcacgtgagcacccaccagcataactatgctgcgcctccttccaccaggaaggactaccccgctgccaagcgggtgaagctggatagcgtccgggtgctgaggcagatcagcaataaccgtaagtgcacctcccccaggagcagtgacacagaggagaacgtgaagaggcggactcacaacgttctggagcgccagcgccggaacgagctgaagcggtccttcttcgctctgagggaccagatcccagagctggagaacaatgagaaggcaccgaaggtggtcatcctgaagaaggccaccgcgtatatcctgagcgtgcaggctgaggagcagaagctgatcagcgaggaggacttgctgaggaagcggcgcgagcagctgaaacacaagctggagcagctgcgaaacagctgcgccggaagcggacagtgtactaattatgctctcttgaaattggctggagatgttgagagcaacccaggtcccatgtacaacatgatggagacagagctgaagccccccgggcctcagcagaccagcggcggcggcgggggcaactccaccgccgccgctgctgggggcaaccagaagaacagccccgatagggtgaagcgccctatgaacgccttcatggtgtggtcccgcggccagcgccgtaagatggctcaggagaaccctaagatgcacaactccgagatcagcaagcggctgggcgcggagtggaagctgctgtcggagaccgagaagcggccattcatcgacgaggccaagaggcttcgtgccctgcacatgaaggagcatcctgactacaagtaccggccccgccggaagaccaagacactgatgaagaaggacaagtacaccttgcctgggggcctgctggcccccgggggcaactccatggcttccggcgtgggcgtgggagccggtctaggcgctggcgtgaaccagcgcatggactcctacgctcacatgaacggctggagcaacgggtcctacagcatgatgcaggaccagttgggctacccccagcaccctgggctgaacgcccatggggctgcccagatgcagcccatgcatcggtacgacgtgagtgccctgcagtacaactccatgacatctagccagacctacatgaacgggagtcccacctacagcatgagctatagccagcaggggaccccaggcatggccctggggtccatgggctccgtggtgaagtcggaggccagctcctcacctcccgtggtgacaagctcctcccacagccgggccccctgccaggctggggatctgagggacatgatctccatgtacctcccgggcgccgaggtgcccgagcctgctgctcccagcaggctgcatatgagccagcattaccagtccgggcccgtgcccggcactgccatcaatgggacactgccactgtcccatatgtga

SEQ ID NO: 30 - DNA, 3939 bp, synthetic construct
  source 1..3939: mol_type = other DNA
atggctggccacctggcctctgccttcgccttctctcccccacctggcggcggcggtgccggccccggaggacccgcccctggatgggtggcccctagaacctggctgtcattccagggacctcctggcggacccggcatcggacctggcgtcgggcccggcagcgccgtgtggggcatacctccctgccctcccccctacgccttctgcgggggcatggcctactgtggcccccaggtcggggtcggcctggtgccccagggcggcctcgccaccagccagcccgccggcgccgctggtgtcggagtggccagcaactccgccggggccagcccagccccatgcaccgtgactcccggcgcagtgaagctggccaaggccaagctggcccagaatcctgccgcctctcaggccatcaaggcgctccagaaggagctggagcagttcgcgaagctgctgaagcagaagcggatcacgctggggtacacccaggccgacgtcggcctgaccctgggcgtcctgttcggcaaggtgttcagccagaccaccatctgccggttcgaggccctgcagcttagcttcaagaacatgtgcaagctgcgcccacttctgcagaagtgggtggaggaggcggataacaacgagaacctgcaggagatctgcaaggccgagacgctggtgcaggccaggaagcgaaagcggacctccatcgagaaccgcgttcgcgggaacctggagaacctgttcctgcagtgtcccaagcctacactgcagcagatctctcacatagcccagcagctgggcctggagaaggatgtggtgcgagtgtggttctgcaatcggaggcagaagggcaagcgctcttcctccgcctacgcccagagggccgccttcgccgcggcggggtcccccttcagcggcggccccgtgtccttccctctggcccccgggccacacttcgggactcccggctacggcagcccacacttcaccgcgctgtacagcagcgtgccattccctgccggggccgccttcccccccgtgagcgtgacgacgctgggcagccccatgcacagcaatggaagcggagccacgaacttctctctgttaaagcaagcaggagatgttgaagaaaaccccgggcctatggccgtgtccgacgccctgctgccctcattcagcaccttcgcctcaggccccgctggcagagaaaagacactgagacaggctggagcccctaacaaccgctggcgcgaggagctgagtcacatgaaacgcctgccccctgtcctgcctgggcggccatacgacctggccgccgccacggtggccaccgacctggagtcaggcggggccggagccgcctgtggcggctccaacctggcgcccctgccccgcagggagactgaggagttcaacgatctgctggatctggacttcatcctcagtaactctctgacccaccccccagagagtgttgctgctaccgtgagcagcagcgccagcgcgagctctagcagcagccctagcagctccgggcctgccagtgcccccagcacctgcagcttcacctaccccatcagggccggtaacgaccctggtgtggcccccggcggcaccgggggcggactcctgtacggccgggagtccgcccccccgcccaccgcccccttcaacctggcggacatcaacgatgtgagcccctccgggggcttcgtcgccgagctgctgcggccagagctcgaccctgtgtacatccccccacagcagccgcagcccccgggcggcggcctgatggggaagttcgtgctcaaggccagcctgagcgcacccggctctgagtacggaagcccctccgtgatcagtgtgagcaagggaagccccgacggctcacaccccgtggttgtggccccctacaacggcgggccgccacggacctgccccaagatcaagcaggaggcagtgagcagctgcacccatctgggtgcggggccaccactgtccaacggccaccgccccgctgcccatgacttccctctgggcaggcagctgcccagcaggaccacccctacgctgggcctggaggaggtcctgtcctccagggactgccacccggccctgcccctgcccccggggttccacccccaccccggacccaactaccccagcttcctgcctgaccagatgcagccgcaggttccgcccctgcattaccaggagctgatgcccccgggcagctgcatgcccgaggagcctaagcctaagcggggccggcgcagctggccccgcaagcggaccgccacccacacttgcgattacgccgggtgcggcaagacctacacaaagagttcgcacctgaaggcccacctgcgaactcacacgggcgagaagccctaccactgcgactgggacgggtgcggctggaagttcgcccggtccgatgagctgacccggcactatcggaagcacaccgggcacaggcccttccagtgccagaagtgtgaccgggccttcagccggtcagaccatctggcactgcacatgaagcgccacttcggaagcggagagggcaggggaagtcttctaacatgcggggacgtggaggaaaatcccggccccatgcccctgaatgtgtccttcaccaaccgcaactatgatctggactatgactctgtgcagccttacttctactgcgatgaggaggagaacttctaccagcagcagcagcagagcgaactgcagccacccgccccatccgaggatatctggaggaggttcgagctgctgccgacccctcctctcagcccctccaggaggagcgggctgtgcagtcccagctacgtggctgtgacccccttctccctgcgcggcgacaacgacggcgggggggggagcttcagcaccgctgaccagctggagatggtcaccgagctgctgggtggcgacatggtcaaccagagcttcatctgcgaccctgatgatgagacattcatcaggaacatcatcatccaggactgcatgtggtccggcttctcggccgctgccaggctggtcagcgagaggctggccagctaccaggccgcccggagggattccgggtcgcctaaccccgccaggggccacagcgtctgctccacgagcagcctgtacctgcaggatctgagcgccgccgccagcgagtgcatagatccttcagtggtgttcccatacccactgaacgacagcagctctcccaggagctgcgcctcgcaggacagcagcgccttcagcccctcgtccgactcgctgctgtccagcaccgagtcgagcccccagggctctcctgagcccctggtgctgcacgaggagacccctcctaccacctcctcggactccgaggaggagcaggaggatgaggaagagatcgacgtggtcagcgtggagaggcgccaggctcctggcaggcgcagcgagtctggcagcccctccgccgggggccacagcaggcccccgcacagcccgctggtgctgaggcggtgtcacgtgagcacccaccagcataactatgctgcgcctccttccaccaggagggactaccccgctgccaggcgggtgaggctggatagcgtccgggtgctgaggcagatcagcaataaccgtaggtgcacctcccccaggagcagtgacacagaggagaacgtgaggaggcggactcacaacgttctggagcgccagcgccggaacgagctgaggcggtccttcttcgctctgagggaccagatcccagagctggagaacaatgagagggcaccgagggtggtcatcctgaggagggccaccgcgtatatcctgagcgtgcaggctgaggagcagaggctgatcagcgaggaggacttgctgaggaggcggcgcgagcagctgaggcacaggctggagcagctgcgaaacagctgcgcctga

SEQ ID NO: 31 - DNA, 3939 bp, synthetic construct
  source 1..3939: mol_type = other DNA
atggctggccacctggcctctgacttcgccttctctcccccacctggcggcggcggtgacggccccggaggacccgagcctggatgggtggaccctagaacctggctgtcattccagggacctcctggcggacccggcatcggacctggcgtcgggcccggcagcgaggtgtggggcatacctccctgccctcccccctacgagttctgcgggggcatggcctactgtggcccccaggtcggggtcggcctggtgccccagggcggcctcgaaaccagccagcccgagggcgaggctggtgtcggagtggagagcaactccgacggggccagcccagagccatgcaccgtgactcccggcgcagtgaagctggaaaaggagaagctggagcagaatcctgaggagtctcaggacatcaaggcgctccagaaggagctggagcagttcgcgaagctgctgaagcagaagcggatcacgctggggtacacccaggccgacgtcggcctgaccctgggcgtcctgttcggcaaggtgttcagccagaccaccatctgccggttcgaggccctgcagcttagcttcaagaacatgtgcaagctgcgcccacttctgcagaagtgggtggaggaggcggataacaacgagaacctgcaggagatctgcaaggccgagacgctggtgcaggccaggaagcgaaagcggacctccatcgagaaccgcgttcgcgggaacctggagaacctgttcctgcagtgtcccaagcctacactgcagcagatctctcacatagcccagcagctgggcctggagaaggatgtggtgcgagtgtggttctgcaatcggaggcagaagggcaagcgctcttcctccgattacgcccagagggaggacttcgaggcggcggggtcccccttcagcggcggccccgtgtccttccctctggcccccgggccacacttcgggactcccggctacggcagcccacacttcaccgcgctgtacagcagcgtgccattccctgagggggaggccttcccccccgtgagcgtgacgacgctgggcagccccatgcacagcaatggaagcggagccacgaacttctctctgttaaagcaagcaggagatgttgaagaaaaccccgggcctatggccgtgtccgacgccctgctgccctcattcagcaccttcgcctcaggccccgctggcagagaaaagacactgagacaggctggagcccctaacaaccgctggcgcgaggagctgagtcacatgaaacgcctgccccctgtcctgcctgggcggccatacgacctggccgccgccacggtggccaccgacctggagtcaggcggggccggagccgcctgtggcggctccaacctggcgcccctgccccgcagggagactgaggagttcaacgatctgctggatctggacttcatcctcagtaactctctgacccaccccccagagagtgttgctgctaccgtgagcagcagcgccagcgcgagctctagcagcagccctagcagctccgggcctgccagtgcccccagcacctgcagcttcacctaccccatcagggccggtaacgaccctggtgtggcccccggcggcaccgggggcggactcctgtacggccgggagtccgcccccccgcccaccgcccccttcaacctggcggacatcaacgatgtgagcccctccgggggcttcgtcgccgagctgctgcggccagagctcgaccctgtgtacatccccccacagcagccgcagcccccgggcggcggcctgatggggaagttcgtgctcaaggccagcctgagcgcacccggctctgagtacggaagcccctccgtgatcagtgtgagcaagggaagccccgacggctcacaccccgtggttgtggccccctacaacggcgggccgccacggacctgccccaagatcaagcaggaggcagtgagcagctgcacccatctgggtgcggggccaccactgtccaacggccaccgccccgctgcccatgacttccctctgggcaggcagctgcccagcaggaccacccctacgctgggcctggaggaggtcctgtcctccagggactgccacccggccctgcccctgcccccggggttccacccccaccccggacccaactaccccagcttcctgcctgaccagatgcagccgcaggttccgcccctgcattaccaggagctgatgcccccgggcagctgcatgcccgaggagcctaagcctaagcggggccggcgcagctggccccgcaagcggaccgccacccacacttgcgattacgccgggtgcggcaagacctacacaaagagttcgcacctgaaggcccacctgcgaactcacacgggcgagaagccctaccactgcgactgggacgggtgcggctggaagttcgcccggtccgatgagctgacccggcactatcggaagcacaccgggcacaggcccttccagtgccagaagtgtgaccgggccttcagccggtcagaccatctggcactgcacatgaagcgccacttcggaagcggagagggcaggggaagtcttctaacatgcggggacgtggaggaaaatcccggccccatgcccctgaatgtgtccttcaccaaccgcaactatgatctggactatgactctgtgcagccttacttctactgcgatgaggaggagaacttctaccagcagcagcagcagagcgaactgcagccacccgccccatccgaggatatctggaagaagttcgagctgctgccgacccctcctctcagcccctccaggaggagcgggctgtgcagtcccagctacgtggctgtgacccccttctccctgcgcggcgacaacgacggcgggggggggagcttcagcaccgctgaccagctggagatggtcaccgagctgctgggtggcgacatggtcaaccagagcttcatctgcgaccctgatgatgagacattcatcaagaacatcatcatccaggactgcatgtggtccggcttctcggccgctgccaagctggtcagcgagaagctggccagctaccaggccgcccggaaggattccgggtcgcctaaccccgccaggggccacagcgtctgctccacgagcagcctgtacctgcaggatctgagcgccgccgccagcgagtgcatagatccttcagtggtgttcccatacccactgaacgacagcagctctcccaagagctgcgcctcgcaggacagcagcgccttcagcccctcgtccgactcgctgctgtccagcaccgagtcgagcccccagggctctcctgagcccctggtgctgcacgaggagacccctcctaccacctcctcggactccgaggaggagcaggaggatgaggaagagatcgacgtggtcagcgtggagaagcgccaggctcctggcaagcgcagcgagtctggcagcccctccgccgggggccacagcaagcccccgcacagcccgctggtgctgaagcggtgtcacgtgagcacccaccagcataactatgctgcgcctccttccaccaggaaggactaccccgctgccaagcgggtgaagctggatagcgtccgggtgctgaggcagatcagcaataaccgtaagtgcacctcccccaggagcagtgacacagaggagaacgtgaagaggcggactcacaacgttctggagcgccagcgccggaacgagctgaagcggtccttcttcgctctgagggaccagatcccagagctggagaacaatgagaaggcaccgaaggtggtcatcctgaagaaggccaccgcgtatatcctgagcgtgcaggctgaggagcagaagctgatcagcgaggaggacttgctgaggaagcggcgcgagcagctgaaacacaagctggagcagctgcgaaacagctgcgcctga

SEQ ID NO: 32 - DNA, 3573 bp, synthetic construct
  source 1..3573: mol_type = other DNA
atggctggccacctggcctctgccttcgccttctctcccccacctggcggcggcggtgccggccccggaggacccgcccctggatgggtggcccctagaacctggctgtcattccagggacctcctggcggacccggcatcggacctggcgtcgggcccggcagcgccgtgtggggcatacctccctgccctcccccctacgccttctgcgggggcatggcctactgtggcccccaggtcggggtcggcctggtgccccagggcggcctcgccaccagccagcccgccggcgccgctggtgtcggagtggccagcaactccgccggggccagcccagccccatgcaccgtgactcccggcgcagtgaagctggccaaggccaagctggcccagaatcctgccgcctctcaggccatcaaggcgctccagaaggagctggagcagttcgcgaagctgctgaagcagaagcggatcacgctggggtacacccaggccgacgtcggcctgaccctgggcgtcctgttcggcaaggtgttcagccagaccaccatctgccggttcgaggccctgcagcttagcttcaagaacatgtgcaagctgcgcccacttctgcagaagtgggtggaggaggcggataacaacgagaacctgcaggagatctgcaaggccgagacgctggtgcaggccaggaagcgaaagcggacctccatcgagaaccgcgttcgcgggaacctggagaacctgttcctgcagtgtcccaagcctacactgcagcagatctctcacatagcccagcagctgggcctggagaaggatgtggtgcgagtgtggttctgcaatcggaggcagaagggcaagcgctcttcctccgcctacgcccagagggccgccttcgccgcggcggggtcccccttcagcggcggccccgtgtccttccctctggcccccgggccacacttcgggactcccggctacggcagcccacacttcaccgcgctgtacagcagcgtgccattccctgccggggccgccttcccccccgtgagcgtgacgacgctgggcagccccatgcacagcaatggaagcggagccacgaacttctctctgttaaagcaagcaggagatgttgaagaaaaccccgggcctatggccgtgtccgacgccctgctgccctcattcagcaccttcgcctcaggccccgctggcagagaaaagacactgagacaggctggagcccctaacaaccgctggcgcgaggagctgagtcacatgaaacgcctgccccctgtcctgcctgggcggccatacgacctggccgccgccacggtggccaccgacctggagtcaggcggggccggagccgcctgtggcggctccaacctggcgcccctgccccgcagggagactgaggagttcaacgatctgctggatctggacttcatcctcagtaactctctgacccaccccccagagagtgttgctgctaccgtgagcagcagcgccagcgcgagctctagcagcagccctagcagctccgggcctgccagtgcccccagcacctgcagcttcacctaccccatcagggccggtaacgaccctggtgtggcccccggcggcaccgggggcggactcctgtacggccgggagtccgcccccccgcccaccgcccccttcaacctggcggacatcaacgatgtgagcccctccgggggcttcgtcgccgagctgctgcggccagagctcgaccctgtgtacatccccccacagcagccgcagcccccgggcggcggcctgatggggaagttcgtgctcaaggccagcctgagcgcacccggctctgagtacggaagcccctccgtgatcagtgtgagcaagggaagccccgacggctcacaccccgtggttgtggccccctacaacggcgggccgccacggacctgccccaagatcaagcaggaggcagtgagcagctgcacccatctgggtgcggggccaccactgtccaacggccaccgccccgctgcccatgacttccctctgggcaggcagctgcccagcaggaccacccctacgctgggcctggaggaggtcctgtcctccagggactgccacccggccctgcccctgcccccggggttccacccccaccccggacccaactaccccagcttcctgcctgaccagatgcagccgcaggttccgcccctgcattaccaggagctgatgcccccgggcagctgcatgcccgaggagcctaagcctaagcggggccggcgcagctggccccgcaagcggaccgccacccacacttgcgattacgccgggtgcggcaagacctacacaaagagttcgcacctgaaggcccacctgcgaactcacacgggcgagaagccctaccactgcgactgggacgggtgcggctggaagttcgcccggtccgatgagctgacccggcactatcggaagcacaccgggcacaggcccttccagtgccagaagtgtgaccgggccttcagccggtcagaccatctggcactgcacatgaagcgccacttcggaagcggagagggcaggggaagtcttctaacatgcggggacgtggaggaaaatcccggccccatgtacaacatgatggagacagagctgaagccccccgggcctcagcagaccagcggcggcggcgggggcaactccaccgccgccgctgctgggggcaaccagaagaacagccccgatagggtgaagcgccctatgaacgccttcatggtgtggtcccgcggccagcgccgtaagatggctcaggagaaccctaagatgcacaactccgagatcagcaagcggctgggcgcggagtggaagctgctgtcggagaccgagaagcggccattcatcgacgaggccaagaggcttcgtgccctgcacatgaaggagcatcctgactacaagtaccggccccgccggaagaccaagacactgatgaagaaggacaagtacaccttgcctgggggcctgctggcccccgggggcaactccatggcttccggcgtgggcgtgggagccggtctaggcgctggcgtgaaccagcgcatggactcctacgctcacatgaacggctggagcaacgggtcctacagcatgatgcaggaccagttgggctacccccagcaccctgggctgaacgcccatggggctgcccagatgcagcccatgcatcggtacgacgtgagtgccctgcagtacaactccatgacatctagccagacctacatgaacgggagtcccacctacagcatgagctatagccagcaggggaccccaggcatggccctggggtccatgggctccgtggtgaagtcggaggccagctcctcacctcccgtggtgacaagctcctcccacagccgggccccctgccaggctggggatctgagggacatgatctccatgtacctcccgggcgccgaggtgcccgagcctgctgctcccagcaggctgcatatgagccagcattaccagtccgggcccgtgcccggcactgccatcaatgggacactgccactgtcccatatgtga

SEQ ID NO: 33 - DNA, 3573 bp, synthetic construct
  source 1..3573: mol_type = other DNA
atggctggccacctggcctctgacttcgccttctctcccccacctggcggcggcggtgacggccccggaggacccgagcctggatgggtggaccctagaacctggctgtcattccagggacctcctggcggacccggcatcggacctggcgtcgggcccggcagcgaggtgtggggcatacctccctgccctcccccctacgagttctgcgggggcatggcctactgtggcccccaggtcggggtcggcctggtgccccagggcggcctcgaaaccagccagcccgagggcgaggctggtgtcggagtggagagcaactccgacggggccagcccagagccatgcaccgtgactcccggcgcagtgaagctggaaaaggagaagctggagcagaatcctgaggagtctcaggacatcaaggcgctccagaaggagctggagcagttcgcgaagctgctgaagcagaagcggatcacgctggggtacacccaggccgacgtcggcctgaccctgggcgtcctgttcggcaaggtgttcagccagaccaccatctgccggttcgaggccctgcagcttagcttcaagaacatgtgcaagctgcgcccacttctgcagaagtgggtggaggaggcggataacaacgagaacctgcaggagatctgcaaggccgagacgctggtgcaggccaggaagcgaaagcggacctccatcgagaaccgcgttcgcgggaacctggagaacctgttcctgcagtgtcccaagcctacactgcagcagatctctcacatagcccagcagctgggcctggagaaggatgtggtgcgagtgtggttctgcaatcggaggcagaagggcaagcgctcttcctccgattacgcccagagggaggacttcgaggcggcggggtcccccttcagcggcggccccgtgtccttccctctggcccccgggccacacttcgggactcccggctacggcagcccacacttcaccgcgctgtacagcagcgtgccattccctgagggggaggccttcccccccgtgagcgtgacgacgctgggcagccccatgcacagcaatggaagcggagccacgaacttctctctgttaaagcaagcaggagatgttgaagaaaaccccgggcctatggccgtgtccgacgccctgctgccctcattcagcaccttcgcctcaggccccgctggcagagaaaagacactgagacaggctggagcccctaacaaccgctggcgcgaggagctgagtcacatgaaacgcctgccccctgtcctgcctgggcggccatacgacctggccgccgccacggtggccaccgacctggagtcaggcggggccggagccgcctgtggcggctccaacctggcgcccctgccccgcagggagactgaggagttcaacgatctgctggatctggacttcatcctcagtaactctctgacccaccccccagagagtgttgctgctaccgtgagcagcagcgccagcgcgagctctagcagcagccctagcagctccgggcctgccagtgcccccagcacctgcagcttcacctaccccatcagggccggtaacgaccctggtgtggcccccggcggcaccgggggcggactcctgtacggccgggagtccgcccccccgcccaccgcccccttcaacctggcggacatcaacgatgtgagcccctccgggggcttcgtcgccgagctgctgcggccagagctcgaccctgtgtacatccccccacagcagccgcagcccccgggcggcggcctgatggggaagttcgtgctcaaggccagcctgagcgcacccggctctgagtacggaagcccctccgtgatcagtgtgagcaagggaagccccgacggctcacaccccgtggttgtggccccctacaacggcgggccgccacggacctgccccaagatcaagcaggaggcagtgagcagctgcacccatctgggtgcggggccaccactgtccaacggccaccgccccgctgcccatgacttccctctgggcaggcagctgcccagcaggaccacccctacgctgggcctggaggaggtcctgtcctccagggactgccacccggccctgcccctgcccccggggttccacccccaccccggacccaactaccccagcttcctgcctgaccagatgcagccgcaggttccgcccctgcattaccaggagctgatgcccccgggcagctgcatgcccgaggagcctaagcctaagcggggccggcgcagctggccccgcaagcggaccgccacccacacttgcgattacgccgggtgcggcaagacctacacaaagagttcgcacctgaaggcccacctgcgaactcacacgggcgagaagccctaccactgcgactgggacgggtgcggctggaagttcgcccggtccgatgagctgacccggcactatcggaagcacaccgggcacaggcccttccagtgccagaagtgtgaccgggccttcagccggtcagaccatctggcactgcacatgaagcgccacttcggaagcggagagggcaggggaagtcttctaacatgcggggacgtggaggaaaatcccggccccatgtacaacatgatggagacagagctgaagccccccgggcctcagcagaccagcggcggcggcgggggcaactccaccgccgccgctgctgggggcaaccagaagaacagccccgatagggtgaagcgccctatgaacgccttcatggtgtggtcccgcggccagcgccgtaagatggctcaggagaaccctaagatgcacaactccgagatcagcaagcggctgggcgcggagtggaagctgctgtcggagaccgagaagcggccattcatcgacgaggccaagaggcttcgtgccctgcacatgaaggagcatcctgactacaagtaccggccccgccggaagaccaagacactgatgaagaaggacaagtacaccttgcctgggggcctgctggcccccgggggcaactccatggcttccggcgtgggcgtgggagccggtctaggcgctggcgtgaaccagcgcatggactcctacgctcacatgaacggctggagcaacgggtcctacagcatgatgcaggaccagttgggctacccccagcaccctgggctgaacgcccatggggctgcccagatgcagcccatgcatcggtacgacgtgagtgccctgcagtacaactccatgacatctagccagacctacatgaacgggagtcccacctacagcatgagctatagccagcaggggaccccaggcatggccctggggtccatgggctccgtggtgaagtcggaggccagctcctcacctcccgtggtgacaagctcctcccacagccgggccccctgccaggctggggatctgagggacatgatctccatgtacctcccgggcgccgaggtgcccgagcctgctgctcccagcaggctgcatatgagccagcattaccagtccgggcccgtgcccggcactgccatcaatgggacactgccactgtcccatatgtga

SEQ ID NO: 34 - DNA, 11788 bp, synthetic construct
  source 1..11788: mol_type = other DNA
aatgtagtcttatgcaatactcttgtagtcttgcaacatggtaacgatgagttagcaacatgccttacaaggagagaaaaagcaccgtgcatgccgattggtggaagtaaggtggtacgatcgtgccttattaggaaggcaacagacgggtctgacatggattggacgaaccactgaattgccgcattgcagagatattgtatttaagtgcctagctcgatacataaacgggtctctctggttagaccagatctgagcctgggagctctctggctaactagggaacccactgcttaagcctcaataaagcttgccttgagtgcttcaagtagtgtgtgcccgtctgttgtgtgactctggtaactagagatccctcagacccttttagtcagtgtggaaaatctctagcagtggcgcccgaacagggacttgaaagcgaaagggaaaccagaggagctctctcgacgcaggactcggcttgctgaagcgcgcacggcaagaggcgaggggcggcgactggtgagtacgccaaaaattttgactagcggaggctagaaggagagagatgggtgcgagagcgtcagtattaagcgggggagaattagatcgcgatgggaaaaaattcggttaaggccagggggaaagaaaaaatataaattaaaacatatagtatgggcaagcagggagctagaacgattcgcagttaatcctggcctgttagaaacatcagaaggctgtagacaaatactgggacagctacaaccatcccttcagacaggatcagaagaacttagatcattatataatacagtagcaaccctctattgtgtgcatcaaaggatagagataaaagacaccaaggaagctttagacaagatagaggaagagcaaaacaaaagtaagaccaccgcacagcaagcggccgctgatcttcagacctggaggaggagatatgagggacaattggagaagtgaattatataaatataaagtagtaaaaattgaaccattaggagtagcacccaccaaggcaaagagaagagtggtgcagagagaaaaaagagcagtgggaataggagctttgttccttgggttcttgggagcagcaggaagcactatgggcgcagcgtcaatgacgctgacggtacaggccagacaattattgtctggtatagtgcagcagcagaacaatttgctgagggctattgaggcgcaacagcatctgttgcaactcacagtctggggcatcaagcagctccaggcaagaatcctggctgtggaaagatacctaaaggatcaacagctcctggggatttggggttgctctggaaaactcatttgcaccactgctgtgccttggaatgctagttggagtaataaatctctggaacagatttggaatcacacgacctggatggagtgggacagagaaattaacaattacacaagcttaatacactccttaattgaagaatcgcaaaaccagcaagaaaagaatgaacaagaattattggaattagataaatgggcaagtttgtggaattggtttaacataacaaattggctgtggtatataaaattattcataatgatagtaggaggcttggtaggtttaagaatagtttttgctgtactttctatagtgaatagagttaggcagggatattcaccattatcgtttcagacccacctcccaaccccgaggggacccgacaggcccgaaggaatagaagaagaaggtggagagagagacagagacagatccattcgattagtgaacggatctcgacggtatcgctagcttttaaaagaaaaggggggattggggggtacagtgcaggggaaagaatagtagacataatagcaacagacatacaaactaaagaattacaaaaacaaattacaaaaattcaaaattttactagtgattatcggattgataatcgaattcaccggttttactccctatcagtgatagagaacgtatgaagagtttactccctatcagtgatagagaacgtatgcagactttactccctatcagtgatagagaacgtataaggagtttactccctatcagtgatagagaacgtatgaccagtttactccctatcagtgatagagaacgtatctacagtttactccctatcagtgatagagaacgtatatccagtttactccctatcagtgatagagaacgtataagctttaggcgtgtacggtgggcgcctataaaagcagagctcgtttagtgaaccgtcagatcgcctggagcaattccacaacacttttgtcttataccaactttccgtaccacttcctaccctcgtaaactcgaggccgccaccatggctggccacctggcctctgacttcgccttctctcccccacctggcggcggcggtgacggccccggaggacccgagcctggatgggtggaccctagaacctggctgtcattccagggacctcctggcggacccggcatcggacctggcgtcgggcccggcagcgaggtgtggggcatacctccctgccctcccccctacgagttctgcgggggcatggcctactgtggcccccaggtcggggtcggcctggtgccccagggcggcctcgaaaccagccagcccgagggcgaggctggtgtcggagtggagagcaactccgacggggccagcccagagccatgcaccgtgactcccggcgcagtgaagctggaaaaggagaagctggagcagaatcctgaggagtctcaggacatcaaggcgctccagaaggagctggagcagttcgcgaagctgctgaagcagaagcggatcacgctggggtacacccaggccgacgtcggcctgaccctgggcgtcctgttcggcaaggtgttcagccagaccaccatctgccggttcgaggccctgcagcttagcttcaagaacatgtgcaagctgcgcccacttctgcagaagtgggtggaggaggcggataacaacgagaacctgcaggagatctgcaaggccgagacgctggtgcaggccaggaagcgaaagcggacctccatcgagaaccgcgttcgcgggaacctggagaacctgttcctgcagtgtcccaagcctacactgcagcagatctctcacatagcccagcagctgggcctggagaaggatgtggtgcgagtgtggttctgcaatcggaggcagaagggcaagcgctcttcctccgattacgcccagagggaggacttcgaggcggcggggtcccccttcagcggcggccccgtgtccttccctctggcccccgggccacacttcgggactcccggctacggcagcccacacttcaccgcgctgtacagcagcgtgccattccctgagggggaggccttcccccccgtgagcgtgacgacgctgggcagccccatgcacagcaatggaagcggagccacgaacttctctctgttaaagcaagcaggagatgttgaagaaaaccccgggcctatggccgtgtccgacgccctgctgccctcattcagcaccttcgcctcaggccccgctggcagagaaaagacactgagacaggctggagcccctaacaaccgctggcgcgaggagctgagtcacatgaaacgcctgccccctgtcctgcctgggcggccatacgacctggccgccgccacggtggccaccgacctggagtcaggcggggccggagccgcctgtggcggctccaacctggcgcccctgccccgcagggagactgaggagttcaacgatctgctggatctggacttcatcctcagtaactctctgacccaccccccagagagtgttgctgctaccgtgagcagcagcgccagcgcgagctctagcagcagccctagcagctccgggcctgccagtgcccccagcacctgcagcttcacctaccccatcagggccggtaacgaccctggtgtggcccccggcggcaccgggggcggactcctgtacggccgggagtccgcccccccgcccaccgcccccttcaacctggcggacatcaacgatgtgagcccctccgggggcttcgtcgccgagctgctgcggccagagctcgaccctgtgtacatccccccacagcagccgcagcccccgggcggcggcctgatggggaagttcgtgctcaaggccagcctgagcgcacccggctctgagtacggaagcccctccgtgatcagtgtgagcaagggaagccccgacggctcacaccccgtggttgtggccccctacaacggcgggccgccacggacctgccccaagatcaagcaggaggcagtgagcagctgcacccatctgggtgcggggccaccactgtccaacggccaccgccccgctgcccatgacttccctctgggcaggcagctgcccagcaggaccacccctacgctgggcctggaggaggtcctgtcctccagggactgccacccggccctgcccctgcccccggggttccacccccaccccggacccaactaccccagcttcctgcctgaccagatgcagccgcaggttccgcccctgcattaccaggagctgatgcccccgggcagctgcatgcccgaggagcctaagcctaagcggggccggcgcagctggccccgcaagcggaccgccacccacacttgcgattacgccgggtgcggcaagacctacacaaagagttcgcacctgaaggcccacctgcgaactcacacgggcgagaagccctaccactgcgactgggacgggtgcggctggaagttcgcccggtccgatgagctgacccggcactatcggaagcacaccgggcacaggcccttccagtgccagaagtgtgaccgggccttcagccggtcagaccatctggcactgcacatgaagcgccacttcggaagcggagagggcaggggaagtcttctaacatgcggggacgtggaggaaaatcccggccccatgcccctgaatgtgtccttcaccaaccgcaactatgatctggactatgactctgtgcagccttacttctactgcgatgaggaggagaacttctaccagcagcagcagcagagcgaactgcagccacccgccccatccgaggatatctggaagaagttcgagctgctgccgacccctcctctcagcccctccaggaggagcgggctgtgcagtcccagctacgtggctgtgacccccttctccctgcgcggcgacaacgacggcgggggggggagcttcagcaccgctgaccagctggagatggtcaccgagctgctgggtggcgacatggtcaaccagagcttcatctgcgaccctgatgatgagacattcatcaagaacatcatcatccaggactgcatgtggtccggcttctcggccgctgccaagctggtcagcgagaagctggccagctaccaggccgcccggaaggattccgggtcgcctaaccccgccaggggccacagcgtctgctccacgagcagcctgtacctgcaggatctgagcgccgccgccagcgagtgcatagatccttcagtggtgttcccatacccactgaacgacagcagctctcccaagagctgcgcctcgcaggacagcagcgccttcagcccctcgtccgactcgctgctgtccagcaccgagtcgagcccccagggctctcctgagcccctggtgctgcacgaggagacccctcctaccacctcctcggactccgaggaggagcaggaggatgaggaagagatcgacgtggtcagcgtggagaagcgccaggctcctggcaagcgcagcgagtctggcagcccctccgccgggggccacagcaagcccccgcacagcccgctggtgctgaagcggtgtcacgtgagcacccaccagcataactatgctgcgcctccttccaccaggaaggactaccccgctgccaagcgggtgaagctggatagcgtccgggtgctgaggcagatcagcaataaccgtaagtgcacctcccccaggagcagtgacacagaggagaacgtgaagaggcggactcacaacgttctggagcgccagcgccggaacgagctgaagcggtccttcttcgctctgagggaccagatcccagagctggagaacaatgagaaggcaccgaaggtggtcatcctgaagaaggccaccgcgtatatcctgagcgtgcaggctgaggagcagaagctgatcagcgaggaggacttgctgaggaagcggcgcgagcagctgaaacacaagctggagcagctgcgaaacagctgcgcctgaggcgcgccgataatcaacctctggattacaaaatttgtgaaagattgactggtattcttaactatgttgctccttttacgctatgtggatacgctgctttaatgcctttgtatcatgctattgcttcccgtatggctttcattttctcctccttgtataaatcctggttgctgtctctttatgaggagttgtggcccgttgtcaggcaacgtggcgtggtgtgcactgtgtttgctgacgcaacccccactggttggggcattgccaccacctgtcagctcctttccgggactttcgctttccccctccctattgccacggcggaactcatcgccgcctgccttgcccgctgctggacaggggctcggctgttgggcactgacaattccgtggtgttgtcggggaagctgacgtcctttccatggctgctcgcctgtgttgccacctggattctgcgcgggacgtccttctgctacgtcccttcggccctcaatccagcggaccttccttcccgcggcctgctgccggctctgcggcctcttccgcgtcttcgccttcgccctcagacgagtcggatctccctttgggccgcctccccgcatcgggaattcccgcggttcgaacgcgatcgcgcgttgacattgattattgactagttattaatagtaatcaattacggggtcattagttcatagcccatatatggagttccgcgttacataacttacggtaaatggcccgcctggctgaccgcccaacgacccccgcccattgacgtcaataatgacgtatgttcccatagtaacgccaatagggactttccattgacgtcaatgggtggagtatttacggtaaactgcccacttggcagtacatcaagtgtatcatatgccaagtacgccccctattgacgtcaatgacggtaaatggcccgcctggcattatgcccagtacatgaccttatgggactttcctacttggcagtacatctacgtattagtcatcgctattaccatggtgatgcggttttggcagtacatcaatgggcgtggatagcggtttgactcacggggatttccaagtctccaccccattgacgtcaatgggagtttgttttggcaccaaaatcaacgggactttccaaaatgtcgtaacaactccgccccattgacgcaaatgggcggtaggcgtgtacggtgggaggtctatataagcagagctgccgccaccatggtgagcaagggcgaggagctgttcaccggggtggtgcccatcctggtcgagctggacggcgacgtaaacggccacaagttcagcgtgtccggcgagggcgagggcgatgccacctacggcaagctgaccctgaagttcatctgcaccaccggcaagctgcccgtgccctggcccaccctcgtgaccaccctgacctacggcgtgcagtgcttcagccgctaccccgaccacatgaagcagcacgacttcttcaagtccgccatgcccgaaggctacgtccaggagcgcaccatcttcttcaaggacgacggcaactacaagacccgcgccgaggtgaagttcgagggcgacaccctggtgaaccgcatcgagctgaagggcatcgacttcaaggaggacggcaacatcctggggcacaagctggagtacaactacaacagccacaacgtctatatcatggccgacaagcagaagaacggcatcaaggtgaacttcaagatccgccacaacatcgaggacggcagcgtgcagctcgccgaccactaccagcagaacacccccatcggcgacggccccgtgctgctgcccgacaaccactacctgagcacccagtccgccctgagcaaagaccccaacgagaagcgcgatcacatggtcctgctggagttcgtgaccgccgccgggatcactctcggcatggacgagctgtacaagtaaggtacctttaagaccaatgacttacaaggcagctgtagatcttagccactttttaaaagaaaaggggggactggaagggctaattcactcccaacgaagacaagatctgctttttgcttgtactgggtctctctggttagaccagatctgagcctgggagctctctggctaactagggaacccactgcttaagcctcaataaagcttgccttgagtgcttcaagtagtgtgtgcccgtctgttgtgtgactctggtaactagagatccctcagacccttttagtcagtgtggaaaatctctagcagtagtagttcatgtcatcttattattcagtatttataacttgcaaagaaatgaatatcagagagtgagaggaacttgtttattgcagcttataatggttacaaataaagcaatagcatcacaaatttcacaaataaagcatttttttcactgcattctagttgtggtttgtccaaactcatcaatgtatcttatcatgtctggctctagctatcccgcccctaactccgcccatcccgcccctaactccgcccagttccgcccattctccgccccatggctgactaattttttttatttatgcagaggccgaggccgcctcggcctctgagctattccagaagtagtgaggaggcttttttggaggcctagggacgtacccaattcgccctatagtgagtcgtattacgcgcgctcactggccgtcgttttacaacgtcgtgactgggaaaaccctggcgttacccaacttaatcgccttgcagcacatccccctttcgccagctggcgtaatagcgaagaggcccgcaccgatcgcccttcccaacagttgcgcagcctgaatggcgaatgggacgcgccctgtagcggcgcattaagcgcggcgggtgtggtggttacgcgcagcgtgaccgctacacttgccagcgccctagcgcccgctcctttcgctttcttcccttcctttctcgccacgttcgccggctttccccgtcaagctctaaatcgggggctccctttagggttccgatttagtgctttacggcacctcgaccccaaaaaacttgattagggtgatggttcacgtagtgggccatcgccctgatagacggtttttcgccctttgacgttggagtccacgttctttaatagtggactcttgttccaaactggaacaacactcaaccctatctcggtctattcttttgatttataagggattttgccgatttcggcctattggttaaaaaatgagctgatttaacaaaaatttaacgcgaattttaacaaaatattaacgcttacaatttaggtggcacttttcggggaaatgtgcgcggaacccctatttgtttatttttctaaatacattcaaatatgtatccgctcatgagacaataaccctgataaatgcttcaataatattgaaaaaggaagagtatgagtattcaacatttccgtgtcgcccttattcccttttttgcggcattttgccttcctgtttttgctcacccagaaacgctggtgaaagtaaaagatgctgaagatcagttgggtgcacgagtgggttacatcgaactggatctcaacagcggtaagatccttgagagttttcgccccgaagaacgttttccaatgatgagcacttttaaagttctgctatgtggcgcggtattatcccgtattgacgccgggcaagagcaactcggtcgccgcatacactattctcagaatgacttggttgagtactcaccagtcacagaaaagcatcttacggatggcatgacagtaagagaattatgcagtgctgccataaccatgagtgataacactgcggccaacttacttctgacaacgatcggaggaccgaaggagctaaccgcttttttgcacaacatgggggatcatgtaactcgccttgatcgttgggaaccggagctgaatgaagccataccaaacgacgagcgtgacaccacgatgcctgtagcaatggcaacaacgttgcgcaaactattaactggcgaactacttactctagcttcccggcaacaattaatagactggatggaggcggataaagttgcaggaccacttctgcgctcggcccttccggctggctggtttattgctgataaatctggagccggtgagcgtgggtctcgcggtatcattgcagcactggggccagatggtaagccctcccgtatcgtagttatctacacgacggggagtcaggcaactatggatgaacgaaatagacagatcgctgagataggtgcctcactgattaagcattggtaactgtcagaccaagtttactcatatatactttagattgatttaaaacttcatttttaatttaaaaggatctaggtgaagatcctttttgataatctcatgaccaaaatcccttaacgtgagttttcgttccactgagcgtcagaccccgtagaaaagatcaaaggatcttcttgagatcctttttttctgcgcgtaatctgctgcttgcaaacaaaaaaaccaccgctaccagcggtggtttgtttgccggatcaagagctaccaactctttttccgaaggtaactggcttcagcagagcgcagataccaaatactgttcttctagtgtagccgtagttaggccaccacttcaagaactctgtagcaccgcctacatacctcgctctgctaatcctgttaccagtggctgctgccagtggcgataagtcgtgtcttaccgggttggactcaagacgatagttaccggataaggcgcagcggtcgggctgaacggggggttcgtgcacacagcccagcttggagcgaacgacctacaccgaactgagatacctacagcgtgagctatgagaaagcgccacgcttcccgaagggagaaaggcggacaggtatccggtaagcggcagggtcggaacaggagagcgcacgagggagcttccagggggaaacgcctggtatctttatagtcctgtcgggtttcgccacctctgacttgagcgtcgatttttgtgatgctcgtcaggggggcggagcctatggaaaaacgccagcaacgcggcctttttacggttcctggccttttgctggccttttgctcacatgttctttcctgcgttatcccctgattctgtggataaccgtattaccgcctttgagtgagctgataccgctcgccgcagccgaacgaccgagcgcagcgagtcagtgagcgaggaagcggaagagcgcccaatacgcaaaccgcctctccccgcgcgttggccgattcattaatgcagctggcacgacaggtttcccgactggaaagcgggcagtgagcgcaacgcaattaatgtgagttagctcactcattaggcaccccaggctttacactttatgcttccggctcgtatgttgtgtggaattgtgagcggataacaatttcacacaggaaacagctatgaccatgattacgccaagcgcgcaattaaccctcactaaagggaacaaaagctggagctgcaagctt

SEQ ID NO: 35 - DNA, 11788 bp, synthetic construct
  source 1..11788: mol_type = other DNA
aatgtagtcttatgcaatactcttgtagtcttgcaacatggtaacgatgagttagcaacatgccttacaaggagagaaaaagcaccgtgcatgccgattggtggaagtaaggtggtacgatcgtgccttattaggaaggcaacagacgggtctgacatggattggacgaaccactgaattgccgcattgcagagatattgtatttaagtgcctagctcgatacataaacgggtctctctggttagaccagatctgagcctgggagctctctggctaactagggaacccactgcttaagcctcaataaagcttgccttgagtgcttcaagtagtgtgtgcccgtctgttgtgtgactctggtaactagagatccctcagacccttttagtcagtgtggaaaatctctagcagtggcgcccgaacagggacttgaaagcgaaagggaaaccagaggagctctctcgacgcaggactcggcttgctgaagcgcgcacggcaagaggcgaggggcggcgactggtgagtacgccaaaaattttgactagcggaggctagaaggagagagatgggtgcgagagcgtcagtattaagcgggggagaattagatcgcgatgggaaaaaattcggttaaggccagggggaaagaaaaaatataaattaaaacatatagtatgggcaagcagggagctagaacgattcgcagttaatcctggcctgttagaaacatcagaaggctgtagacaaatactgggacagctacaaccatcccttcagacaggatcagaagaacttagatcattatataatacagtagcaaccctctattgtgtgcatcaaaggatagagataaaagacaccaaggaagctttagacaagatagaggaagagcaaaacaaaagtaagaccaccgcacagcaagcggccgctgatcttcagacctggaggaggagatatgagggacaattggagaagtgaattatataaatataaagtagtaaaaattgaaccattaggagtagcacccaccaaggcaaagagaagagtggtgcagagagaaaaaagagcagtgggaataggagctttgttccttgggttcttgggagcagcaggaagcactatgggcgcagcgtcaatgacgctgacggtacaggccagacaattattgtctggtatagtgcagcagcagaacaatttgctgagggctattgaggcgcaacagcatctgttgcaactcacagtctggggcatcaagcagctccaggcaagaatcctggctgtggaaagatacctaaaggatcaacagctcctggggatttggggttgctctggaaaactcatttgcaccactgctgtgccttggaatgctagttggagtaataaatctctggaacagatttggaatcacacgacctggatggagtgggacagagaaattaacaattacacaagcttaatacactccttaattgaagaatcgcaaaaccagcaagaaaagaatgaacaagaattattggaattagataaatgggcaagtttgtggaattggtttaacataacaaattggctgtggtatataaaattattcataatgatagtaggaggcttggtaggtttaagaatagtttttgctgtactttctatagtgaatagagttaggcagggatattcaccattatcgtttcagacccacctcccaaccccgaggggacccgacaggcccgaaggaatagaagaagaaggtggagagagagacagagacagatccattcgattagtgaacggatctcgacggtatcgctagcttttaaaagaaaaggggggattggggggtacagtgcaggggaaagaatagtagacataatagcaacagacatacaaactaaagaattacaaaaacaaattacaaaaattcaaaattttactagtgattatcggattgataatcgaattcaccggttttactccctatcagtgatagagaacgtatgaagagtttactccctatcagtgatagagaacgtatgcagactttactccctatcagtgatagagaacgtataaggagtttactccctatcagtgatagagaacgtatgaccagtttactccctatcagtgatagagaacgtatctacagtttactccctatcagtgatagagaacgtatatccagtttactccctatcagtgatagagaacgtataagctttaggcgtgtacggtgggcgcctataaaagcagagctcgtttagtgaaccgtcagatcgcctggagcaattccacaacacttttgtcttataccaactttccgtaccacttcctaccctcgtaaactcgaggccgccaccatggctggccacctggcctctgccttcgccttctctcccccacctggcggcggcggtgccggccccggaggacccgcccctggatgggtggcccctagaacctggctgtcattccagggacctcctggcggacccggcatcggacctggcgtcgggcccggcagcgccgtgtggggcatacctccctgccctcccccctacgccttctgcgggggcatggcctactgtggcccccaggtcggggtcggcctggtgccccagggcggcctcgccaccagccagcccgccggcgccgctggtgtcggagtggccagcaactccgccggggccagcccagccccatgcaccgtgactcccggcgcagtgaagctggccaaggccaagctggcccagaatcctgccgcctctcaggccatcaaggcgctccagaaggagctggagcagttcgcgaagctgctgaagcagaagcggatcacgctggggtacacccaggccgacgtcggcctgaccctgggcgtcctgttcggcaaggtgttcagccagaccaccatctgccggttcgaggccctgcagcttagcttcaagaacatgtgcaagctgcgcccacttctgcagaagtgggtggaggaggcggataacaacgagaacctgcaggagatctgcaaggccgagacgctggtgcaggccaggaagcgaaagcggacctccatcgagaaccgcgttcgcgggaacctggagaacctgttcctgcagtgtcccaagcctacactgcagcagatctctcacatagcccagcagctgggcctggagaaggatgtggtgcgagtgtggttctgcaatcggaggcagaagggcaagcgctcttcctccgcctacgcccagagggccgccttcgccgcggcggggtcccccttcagcggcggccccgtgtccttccctctggcccccgggccacacttcgggactcccggctacggcagcccacacttcaccgcgctgtacagcagcgtgccattccctgccggggccgccttcccccccgtgagcgtgacgacgctgggcagccccatgcacagcaatggaagcggagccacgaacttctctctgttaaagcaagcaggagatgttgaagaaaaccccgggcctatggccgtgtccgacgccctgctgccctcattcagcaccttcgcctcaggccccgctggcagagaaaagacactgagacaggctggagcccctaacaaccgctggcgcgaggagctgagtcacatgaaacgcctgccccctgtcctgcctgggcggccatacgacctggccgccgccacggtggccaccgacctggagtcaggcggggccggagccgcctgtggcggctccaacctggcgcccctgccccgcagggagactgaggagttcaacgatctgctggatctggacttcatcctcagtaactctctgacccaccccccagagagtgttgctgctaccgtgagcagcagcgccagcgcgagctctagcagcagccctagcagctccgggcctgccagtgcccccagcacctgcagcttcacctaccccatcagggccggtaacgaccctggtgtggcccccggcggcaccgggggcggactcctgtacggccgggagtccgcccccccgcccaccgcccccttcaacctggcggacatcaacgatgtgagcccctccgggggcttcgtcgccgagctgctgcggccagagctcgaccctgtgtacatccccccacagcagccgcagcccccgggcggcggcctgatggggaagttcgtgctcaaggccagcctgagcgcacccggctctgagtacggaagcccctccgtgatcagtgtgagcaagggaagccccgacggctcacaccccgtggttgtggccccctacaacggcgggccgccacggacctgccccaagatcaagcaggaggcagtgagcagctgcacccatctgggtgcggggccaccactgtccaacggccaccgccccgctgcccatgacttccctctgggcaggcagctgcccagcaggaccacccctacgctgggcctggaggaggtcctgtcctccagggactgccacccggccctgcccctgcccccggggttccacccccaccccggacccaactaccccagcttcctgcctgaccagatgcagccgcaggttccgcccctgcattaccaggagctgatgcccccgggcagctgcatgcccgaggagcctaagcctaagcggggccggcgcagctggccccgcaagcggaccgccacccacacttgcgattacgccgggtgcggcaagacctacacaaagagttcgcacctgaaggcccacctgcgaactcacacgggcgagaagccctaccactgcgactgggacgggtgcggctggaagttcgcccggtccgatgagctgacccggcactatcggaagcacaccgggcacaggcccttccagtgccagaagtgtgaccgggccttcagccggtcagaccatctggcactgcacatgaagcgccacttcggaagcggagagggcaggggaagtcttctaacatgcggggacgtggaggaaaatcccggccccatgcccctgaatgtgtccttcaccaaccgcaactatgatctggactatgactctgtgcagccttacttctactgcgatgaggaggagaacttctaccagcagcagcagcagagcgaactgcagccacccgccccatccgaggatatctggaggaggttcgagctgctgccgacccctcctctcagcccctccaggaggagcgggctgtgcagtcccagctacgtggctgtgacccccttctccctgcgcggcgacaacgacggcgggggggggagcttcagcaccgctgaccagctggagatggtcaccgagctgctgggtggcgacatggtcaaccagagcttcatctgcgaccctgatgatgagacattcatcaggaacatcatcatccaggactgcatgtggtccggcttctcggccgctgccaggctggtcagcgagaggctggccagctaccaggccgcccggagggattccgggtcgcctaaccccgccaggggccacagcgtctgctccacgagcagcctgtacctgcaggatctgagcgccgccgccagcgagtgcatagatccttcagtggtgttcccatacccactgaacgacagcagctctcccaggagctgcgcctcgcaggacagcagcgccttcagcccctcgtccgactcgctgctgtccagcaccgagtcgagcccccagggctctcctgagcccctggtgctgcacgaggagacccctcctaccacctcctcggactccgaggaggagcaggaggatgaggaagagatcgacgtggtcagcgtggagaggcgccaggctcctggcaggcgcagcgagtctggcagcccctccgccgggggccacagcaggcccccgcacagcccgctggtgctgaggcggtgtcacgtgagcacccaccagcataactatgctgcgcctccttccaccaggagggactaccccgctgccaggcgggtgaggctggatagcgtccgggtgctgaggcagatcagcaataaccgtaggtgcacctcccccaggagcagtgacacagaggagaacgtgaggaggcggactcacaacgttctggagcgccagcgccggaacgagctgaggcggtccttcttcgctctgagggaccagatcccagagctggagaacaatgagagggcaccgagggtggtcatcctgaggagggccaccgcgtatatcctgagcgtgcaggctgaggagcagaggctgatcagcgaggaggacttgctgaggaggcggcgcgagcagctgaggcacaggctggagcagctgcgaaacagctgcgcctgaggcgcgccgataatcaacctctggattacaaaatttgtgaaagattgactggtattcttaactatgttgctccttttacgctatgtggatacgctgctttaatgcctttgtatcatgctattgcttcccgtatggctttcattttctcctccttgtataaatcctggttgctgtctctttatgaggagttgtggcccgttgtcaggcaacgtggcgtggtgtgcactgtgtttgctgacgcaacccccactggttggggcattgccaccacctgtcagctcctttccgggactttcgctttccccctccctattgccacggcggaactcatcgccgcctgccttgcccgctgctggacaggggctcggctgttgggcactgacaattccgtggtgttgtcggggaagctgacgtcctttccatggctgctcgcctgtgttgccacctggattctgcgcgggacgtccttctgctacgtcccttcggccctcaatccagcggaccttccttcccgcggcctgctgccggctctgcggcctcttccgcgtcttcgccttcgccctcagacgagtcggatctccctttgggccgcctccccgcatcgggaattcccgcggttcgaacgcgatcgcgcgttgacattgattattgactagttattaatagtaatcaattacggggtcattagttcatagcccatatatggagttccgcgttacataacttacggtaaatggcccgcctggctgaccgcccaacgacccccgcccattgacgtcaataatgacgtatgttcccatagtaacgccaatagggactttccattgacgtcaatgggtggagtatttacggtaaactgcccacttggcagtacatcaagtgtatcatatgccaagtacgccccctattgacgtcaatgacggtaaatggcccgcctggcattatgcccagtacatgaccttatgggactttcctacttggcagtacatctacgtattagtcatcgctattaccatggtgatgcggttttggcagtacatcaatgggcgtggatagcggtttgactcacggggatttccaagtctccaccccattgacgtcaatgggagtttgttttggcaccaaaatcaacgggactttccaaaatgtcgtaacaactccgccccattgacgcaaatgggcggtaggcgtgtacggtgggaggtctatataagcagagctgccgccaccatggtgagcaagggcgaggagctgttcaccggggtggtgcccatcctggtcgagctggacggcgacgtaaacggccacaagttcagcgtgtccggcgagggcgagggcgatgccacctacggcaagctgaccctgaagttcatctgcaccaccggcaagctgcccgtgccctggcccaccctcgtgaccaccctgacctacggcgtgcagtgcttcagccgctaccccgaccacatgaagcagcacgacttcttcaagtccgccatgcccgaaggctacgtccaggagcgcaccatcttcttcaaggacgacggcaactacaagacccgcgccgaggtgaagttcgagggcgacaccctggtgaaccgcatcgagctgaagggcatcgacttcaaggaggacggcaacatcctggggcacaagctggagtacaactacaacagccacaacgtctatatcatggccgacaagcagaagaacggcatcaaggtgaacttcaagatccgccacaacatcgaggacggcagcgtgcagctcgccgaccactaccagcagaacacccccatcggcgacggccccgtgctgctgcccgacaaccactacctgagcacccagtccgccctgagcaaagaccccaacgagaagcgcgatcacatggtcctgctggagttcgtgaccgccgccgggatcactctcggcatggacgagctgtacaagtaaggtacctttaagaccaatgacttacaaggcagctgtagatcttagccactttttaaaagaaaaggggggactggaagggctaattcactcccaacgaagacaagatctgctttttgcttgtactgggtctctctggttagaccagatctgagcctgggagctctctggctaactagggaacccactgcttaagcctcaataaagcttgccttgagtgcttcaagtagtgtgtgcccgtctgttgtgtgactctggtaactagagatccctcagacccttttagtcagtgtggaaaatctctagcagtagtagttcatgtcatcttattattcagtatttataacttgcaaagaaatgaatatcagagagtgagaggaacttgtttattgcagcttataatggttacaaataaagcaatagcatcacaaatttcacaaataaagcatttttttcactgcattctagttgtggtttgtccaaactcatcaatgtatcttatcatgtctggctctagctatcccgcccctaactccgcccatcccgcccctaactccgcccagttccgcccattctccgccccatggctgactaattttttttatttatgcagaggccgaggccgcctcggcctctgagctattccagaagtagtgaggaggcttttttggaggcctagggacgtacccaattcgccctatagtgagtcgtattacgcgcgctcactggccgtcgttttacaacgtcgtgactgggaaaaccctggcgttacccaacttaatcgccttgcagcacatccccctttcgccagctggcgtaatagcgaagaggcccgcaccgatcgcccttcccaacagttgcgcagcctgaatggcgaatgggacgcgccctgtagcggcgcattaagcgcggcgggtgtggtggttacgcgcagcgtgaccgctacacttgccagcgccctagcgcccgctcctttcgctttcttcccttcctttctcgccacgttcgccggctttccccgtcaagctctaaatcgggggctccctttagggttccgatttagtgctttacggcacctcgaccccaaaaaacttgattagggtgatggttcacgtagtgggccatcgccctgatagacggtttttcgccctttgacgttggagtccacgttctttaatagtggactcttgttccaaactggaacaacactcaaccctatctcggtctattcttttgatttataagggattttgccgatttcggcctattggttaaaaaatgagctgatttaacaaaaatttaacgcgaattttaacaaaatattaacgcttacaatttaggtggcacttttcggggaaatgtgcgcggaacccctatttgtttatttttctaaatacattcaaatatgtatccgctcatgagacaataaccctgataaatgcttcaataatattgaaaaaggaagagtatgagtattcaacatttccgtgtcgcccttattcccttttttgcggcattttgccttcctgtttttgctcacccagaaacgctggtgaaagtaaaagatgctgaagatcagttgggtgcacgagtgggttacatcgaactggatctcaacagcggtaagatccttgagagttttcgccccgaagaacgttttccaatgatgagcacttttaaagttctgctatgtggcgcggtattatcccgtattgacgccgggcaagagcaactcggtcgccgcatacactattctcagaatgacttggttgagtactcaccagtcacagaaaagcatcttacggatggcatgacagtaagagaattatgcagtgctgccataaccatgagtgataacactgcggccaacttacttctgacaacgatcggaggaccgaaggagctaaccgcttttttgcacaacatgggggatcatgtaactcgccttgatcgttgggaaccggagctgaatgaagccataccaaacgacgagcgtgacaccacgatgcctgtagcaatggcaacaacgttgcgcaaactattaactggcgaactacttactctagcttcccggcaacaattaatagactggatggaggcggataaagttgcaggaccacttctgcgctcggcccttccggctggctggtttattgctgataaatctggagccggtgagcgtgggtctcgcggtatcattgcagcactggggccagatggtaagccctcccgtatcgtagttatctacacgacggggagtcaggcaactatggatgaacgaaatagacagatcgctgagataggtgcctcactgattaagcattggtaactgtcagaccaagtttactcatatatactttagattgatttaaaacttcatttttaatttaaaaggatctaggtgaagatcctttttgataatctcatgaccaaaatcccttaacgtgagttttcgttccactgagcgtcagaccccgtagaaaagatcaaaggatcttcttgagatcctttttttctgcgcgtaatctgctgcttgcaaacaaaaaaaccaccgctaccagcggtggtttgtttgccggatcaagagctaccaactctttttccgaaggtaactggcttcagcagagcgcagataccaaatactgttcttctagtgtagccgtagttaggccaccacttcaagaactctgtagcaccgcctacatacctcgctctgctaatcctgttaccagtggctgctgccagtggcgataagtcgtgtcttaccgggttggactcaagacgatagttaccggataaggcgcagcggtcgggctgaacggggggttcgtgcacacagcccagcttggagcgaacgacctacaccgaactgagatacctacagcgtgagctatgagaaagcgccacgcttcccgaagggagaaaggcggacaggtatccggtaagcggcagggtcggaacaggagagcgcacgagggagcttccagggggaaacgcctggtatctttatagtcctgtcgggtttcgccacctctgacttgagcgtcgatttttgtgatgctcgtcaggggggcggagcctatggaaaaacgccagcaacgcggcctttttacggttcctggccttttgctggccttttgctcacatgttctttcctgcgttatcccctgattctgtggataaccgtattaccgcctttgagtgagctgataccgctcgccgcagccgaacgaccgagcgcagcgagtcagtgagcgaggaagcggaagagcgcccaatacgcaaaccgcctctccccgcgcgttggccgattcattaatgcagctggcacgacaggtttcccgactggaaagcgggcagtgagcgcaacgcaattaatgtgagttagctcactcattaggcaccccaggctttacactttatgcttccggctcgtatgttgtgtggaattgtgagcggataacaatttcacacaggaaacagctatgaccatgattacgccaagcgcgcaattaaccctcactaaagggaacaaaagctggagctgcaagctt

SEQ ID NO: 36 - DNA, 11492 bp, synthetic construct
  source 1..11492: mol_type = other DNA
aatgtagtcttatgcaatactcttgtagtcttgcaacatggtaacgatgagttagcaacatgccttacaaggagagaaaaagcaccgtgcatgccgattggtggaagtaaggtggtacgatcgtgccttattaggaaggcaacagacgggtctgacatggattggacgaaccactgaattgccgcattgcagagatattgtatttaagtgcctagctcgatacataaacgggtctctctggttagaccagatctgagcctgggagctctctggctaactagggaacccactgcttaagcctcaataaagcttgccttgagtgcttcaagtagtgtgtgcccgtctgttgtgtgactctggtaactagagatccctcagacccttttagtcagtgtggaaaatctctagcagtggcgcccgaacagggacttgaaagcgaaagggaaaccagaggagctctctcgacgcaggactcggcttgctgaagcgcgcacggcaagaggcgaggggcggcgactggtgagtacgccaaaaattttgactagcggaggctagaaggagagagatgggtgcgagagcgtcagtattaagcgggggagaattagatcgcgatgggaaaaaattcggttaaggccagggggaaagaaaaaatataaattaaaacatatagtatgggcaagcagggagctagaacgattcgcagttaatcctggcctgttagaaacatcagaaggctgtagacaaatactgggacagctacaaccatcccttcagacaggatcagaagaacttagatcattatataatacagtagcaaccctctattgtgtgcatcaaaggatagagataaaagacaccaaggaagctttagacaagatagaggaagagcaaaacaaaagtaagaccaccgcacagcaagcggccgctgatcttcagacctggaggaggagatatgagggacaattggagaagtgaattatataaatataaagtagtaaaaattgaaccattaggagtagcacccaccaaggcaaagagaagagtggtgcagagagaaaaaagagcagtgggaataggagctttgttccttgggttcttgggagcagcaggaagcactatgggcgcagcgtcaatgacgctgacggtacaggccagacaattattgtctggtatagtgcagcagcagaacaatttgctgagggctattgaggcgcaacagcatctgttgcaactcacagtctggggcatcaagcagctccaggcaagaatcctggctgtggaaagatacctaaaggatcaacagctcctggggatttggggttgctctggaaaactcatttgcaccactgctgtgccttggaatgctagttggagtaataaatctctggaacagatttggaatcacacgacctggatggagtgggacagagaaattaacaattacacaagcttaatacactccttaattgaagaatcgcaaaaccagcaagaaaagaatgaacaagaattattggaattagataaatgggcaagtttgtggaattggtttaacataacaaattggctgtggtatataaaattattcataatgatagtaggaggcttggtaggtttaagaatagtttttgctgtactttctatagtgaatagagttaggcagggatattcaccattatcgtttcagacccacctcccaaccccgaggggacccgacaggcccgaaggaatagaagaagaaggtggagagagagacagagacagatccattcgattagtgaacggatctcgacggtatcgctagcttttaaaagaaaaggggggattggggggtacagtgcaggggaaagaatagtagacataatagcaacagacatacaaactaaagaattacaaaaacaaattacaaaaattcaaaattttactagtgattatcggattgataatcgaattccacgtgtttactccctatcagtgatagagaacgtatgaagagtttactccctatcagtgatagagaacgtatgcagactttactccctatcagtgatagagaacgtataaggagtttactccctatcagtgatagagaacgtatgaccagtttactccctatcagtgatagagaacgtatctacagtttactccctatcagtgatagagaacgtatatccagtttactccctatcagtgatagagaacgtataagctttaggcgtgtacggtgggcgcctataaaagcagagctcgtttagtgaaccgtcagatcgcctggagcaattccacaacacttttgtcttataccaactttccgtaccacttcctaccctcgtaaactcgaggccgccaccatggctggccacctggcctctgacttcgccttctctcccccacctggcggcggcggtgacggccccggaggacccgagcctggatgggtggaccctagaacctggctgtcattccagggacctcctggcggacccggcatcggacctggcgtcgggcccggcagcgaggtgtggggcatacctccctgccctcccccctacgagttctgcgggggcatggcctactgtggcccccaggtcggggtcggcctggtgccccagggcggcctcgaaaccagccagcccgagggcgaggctggtgtcggagtggagagcaactccgacggggccagcccagagccatgcaccgtgactcccggcgcagtgaagctggaaaaggagaagctggagcagaatcctgaggagtctcaggacatcaaggcgctccagaaggagctggagcagttcgcgaagctgctgaagcagaagcggatcacgctggggtacacccaggccgacgtcggcctgaccctgggcgtcctgttcggcaaggtgttcagccagaccaccatctgccggttcgaggccctgcagcttagcttcaagaacatgtgcaagctgcgcccacttctgcagaagtgggtggaggaggcggataacaacgagaacctgcaggagatctgcaaggccgagacgctggtgcaggccaggaagcgaaagcggacctccatcgagaaccgcgttcgcgggaacctggagaacctgttcctgcagtgtcccaagcctacactgcagcagatctctcacatagcccagcagctgggcctggagaaggatgtggtgcgagtgtggttctgcaatcggaggcagaagggcaagcgctcttcctccgattacgcccagagggaggacttcgaggcggcggggtcccccttcagcggcggccccgtgtccttccctctggcccccgggccacacttcgggactcccggctacggcagcccacacttcaccgcgctgtacagcagcgtgccattccctgagggggaggccttcccccccgtgagcgtgacgacgctgggcagccccatgcacagcaatggaagcggagccacgaacttctctctgttaaagcaagcaggagatgttgaagaaaaccccgggcctatggccgtgtccgacgccctgctgccctcattcagcaccttcgcctcaggccccgctggcagagaaaagacactgagacaggctggagcccctaacaaccgctggcgcgaggagctgagtcacatgaaacgcctgccccctgtcctgcctgggcggccatacgacctggccgccgccacggtggccaccgacctggagtcaggcggggccggagccgcctgtggcggctccaacctggcgcccctgccccgcagggagactgaggagttcaacgatctgctggatctggacttcatcctcagtaactctctgacccaccccccagagagtgttgctgctaccgtgagcagcagcgccagcgcgagctctagcagcagccctagcagctccgggcctgccagtgcccccagcacctgcagcttcacctaccccatcagggccggtaacgaccctggtgtggcccccggcggcaccgggggcggactcctgtacggccgggagtccgcccccccgcccaccgcccccttcaacctggcggacatcaacgatgtgagcccctccgggggcttcgtcgccgagctgctgcggccagagctcgaccctgtgtacatccccccacagcagccgcagcccccgggcggcggcctgatggggaagttcgtgctcaaggccagcctgagcgcacccggctctgagtacggaagcccctccgtgatcagtgtgagcaagggaagccccgacggctcacaccccgtggttgtggccccctacaacggcgggccgccacggacctgccccaagatcaagcaggaggcagtgagcagctgcacccatctgggtgcggggccaccactgtccaacggccaccgccccgctgcccatgacttccctctgggcaggcagctgcccagcaggaccacccctacgctgggcctggaggaggtcctgtcctccagggactgccacccggccctgcccctgcccccggggttccacccccaccccggacccaactaccccagcttcctgcctgaccagatgcagccgcaggttccgcccctgcattaccaggagctgatgcccccgggcagctgcatgcccgaggagcctaagcctaagcggggccggcgcagctggccccgcaagcggaccgccacccacacttgcgattacgccgggtgcggcaagacctacacaaagagttcgcacctgaaggcccacctgcgaactcacacgggcgagaagccctaccactgcgactgggacgggtgcggctggaagttcgcccggtccgatgagctgacccggcactatcggaagcacaccgggcacaggcccttccagtgccagaagtgtgaccgggccttcagccggtcagaccatctggcactgcacatgaagcgccacttcggaagcggagagggcaggggaagtcttctaacatgcggggacgtggaggaaaatcccggccccatgcccctgaatgtgtccttcaccaaccgcaactatgatctggactatgactctgtgcagccttacttctactgcgatgaggaggagaacttctaccagcagcagcagcagagcgaactgcagccacccgccccatccgaggatatctggaagaagttcgagctgctgccgacccctcctctcagcccctccaggaggagcgggctgtgcagtcccagctacgtggctgtgacccccttctccctgcgcggcgacaacgacggcgggggggggagcttcagcaccgctgaccagctggagatggtcaccgagctgctgggtggcgacatggtcaaccagagcttcatctgcgaccctgatgatgagacattcatcaagaacatcatcatccaggactgcatgtggtccggcttctcggccgctgccaagctggtcagcgagaagctggccagctaccaggccgcccggaaggattccgggtcgcctaaccccgccaggggccacagcgtctgctccacgagcagcctgtacctgcaggatctgagcgccgccgccagcgagtgcatagatccttcagtggtgttcccatacccactgaacgacagcagctctcccaagagctgcgcctcgcaggacagcagcgccttcagcccctcgtccgactcgctgctgtccagcaccgagtcgagcccccagggctctcctgagcccctggtgctgcacgaggagacccctcctaccacctcctcggactccgaggaggagcaggaggatgaggaagagatcgacgtggtcagcgtggagaagcgccaggctcctggcaagcgcagcgagtctggcagcccctccgccgggggccacagcaagcccccgcacagcccgctggtgctgaagcggtgtcacgtgagcacccaccagcataactatgctgcgcctccttccaccaggaaggactaccccgctgccaagcgggtgaagctggatagcgtccgggtgctgaggcagatcagcaataaccgtaagtgcacctcccccaggagcagtgacacagaggagaacgtgaagaggcggactcacaacgttctggagcgccagcgccggaacgagctgaagcggtccttcttcgctctgagggaccagatcccagagctggagaacaatgagaaggcaccgaaggtggtcatcctgaagaaggccaccgcgtatatcctgagcgtgcaggctgaggagcagaagctgatcagcgaggaggacttgctgaggaagcggcgcgagcagctgaaacacaagctggagcagctgcgaaacagctgcgccggaagcggacagtgtactaattatgctctcttgaaattggctggagatgttgagagcaacccaggtcccatgtacaacatgatggagacagagctgaagccccccgggcctcagcagaccagcggcggcggcgggggcaactccaccgccgccgctgctgggggcaaccagaagaacagccccgatagggtgaagcgccctatgaacgccttcatggtgtggtcccgcggccagcgccgtaagatggctcaggagaaccctaagatgcacaactccgagatcagcaagcggctgggcgcggagtggaagctgctgtcggagaccgagaagcggccattcatcgacgaggccaagaggcttcgtgccctgcacatgaaggagcatcctgactacaagtaccggccccgccggaagaccaagacactgatgaagaaggacaagtacaccttgcctgggggcctgctggcccccgggggcaactccatggcttccggcgtgggcgtgggagccggtctaggcgctggcgtgaaccagcgcatggactcctacgctcacatgaacggctggagcaacgggtcctacagcatgatgcaggaccagttgggctacccccagcaccctgggctgaacgcccatggggctgcccagatgcagcccatgcatcggtacgacgtgagtgccctgcagtacaactccatgacatctagccagacctacatgaacgggagtcccacctacagcatgagctatagccagcaggggaccccaggcatggccctggggtccatgggctccgtggtgaagtcggaggccagctcctcacctcccgtggtgacaagctcctcccacagccgggccccctgccaggctggggatctgagggacatgatctccatgtacctcccgggcgccgaggtgcccgagcctgctgctcccagcaggctgcatatgagccagcattaccagtccgggcccgtgcccggcactgccatcaatgggacactgccactgtcccatatgtgaggcgcgccgataatcaacctctggattacaaaatttgtgaaagattgactggtattcttaactatgttgctccttttacgctatgtggatacgctgctttaatgcctttgtatcatgctattgcttcccgtatggctttcattttctcctccttgtataaatcctggttgctgtctctttatgaggagttgtggcccgttgtcaggcaacgtggcgtggtgtgcactgtgtttgctgacgcaacccccactggttggggcattgccaccacctgtcagctcctttccgggactttcgctttccccctccctattgccacggcggaactcatcgccgcctgccttgcccgctgctggacaggggctcggctgttgggcactgacaattccgtggtgttgtcggggaagctgacgtcctttccatggctgctcgcctgtgttgccacctggattctgcgcgggacgtccttctgctacgtcccttcggccctcaatccagcggaccttccttcccgcggcctgctgccggctctgcggcctcttccgcgtcttcgccttcgccctcagacgagtcggatctccctttgggccgcctccccgcatcgggaattcccgcggttcgaacgcgatcgcttggtacctttaagaccaatgacttacaaggcagctgtagatcttagccactttttaaaagaaaaggggggactggaagggctaattcactcccaacgaagacaagatctgctttttgcttgtactgggtctctctggttagaccagatctgagcctgggagctctctggctaactagggaacccactgcttaagcctcaataaagcttgccttgagtgcttcaagtagtgtgtgcccgtctgttgtgtgactctggtaactagagatccctcagacccttttagtcagtgtggaaaatctctagcagtagtagttcatgtcatcttattattcagtatttataacttgcaaagaaatgaatatcagagagtgagaggaacttgtttattgcagcttataatggttacaaataaagcaatagcatcacaaatttcacaaataaagcatttttttcactgcattctagttgtggtttgtccaaactcatcaatgtatcttatcatgtctggctctagctatcccgcccctaactccgcccatcccgcccctaactccgcccagttccgcccattctccgccccatggctgactaattttttttatttatgcagaggccgaggccgcctcggcctctgagctattccagaagtagtgaggaggcttttttggaggcctagggacgtacccaattcgccctatagtgagtcgtattacgcgcgctcactggccgtcgttttacaacgtcgtgactgggaaaaccctggcgttacccaacttaatcgccttgcagcacatccccctttcgccagctggcgtaatagcgaagaggcccgcaccgatcgcccttcccaacagttgcgcagcctgaatggcgaatgggacgcgccctgtagcggcgcattaagcgcggcgggtgtggtggttacgcgcagcgtgaccgctacacttgccagcgccctagcgcccgctcctttcgctttcttcccttcctttctcgccacgttcgccggctttccccgtcaagctctaaatcgggggctccctttagggttccgatttagtgctttacggcacctcgaccccaaaaaacttgattagggtgatggttcacgtagtgggccatcgccctgatagacggtttttcgccctttgacgttggagtccacgttctttaatagtggactcttgttccaaactggaacaacactcaaccctatctcggtctattcttttgatttataagggattttgccgatttcggcctattggttaaaaaatgagctgatttaacaaaaatttaacgcgaattttaacaaaatattaacgcttacaatttaggtggcacttttcggggaaatgtgcgcggaacccctatttgtttatttttctaaatacattcaaatatgtatccgctcatgagacaataaccctgataaatgcttcaataatattgaaaaaggaagagtatgagtattcaacatttccgtgtcgcccttattcccttttttgcggcattttgccttcctgtttttgctcacccagaaacgctggtgaaagtaaaagatgctgaagatcagttgggtgcacgagtgggttacatcgaactggatctcaacagcggtaagatccttgagagttttcgccccgaagaacgttttccaatgatgagcacttttaaagttctgctatgtggcgcggtattatcccgtattgacgccgggcaagagcaactcggtcgccgcatacactattctcagaatgacttggttgagtactcaccagtcacagaaaagcatcttacggatggcatgacagtaagagaattatgcagtgctgccataaccatgagtgataacactgcggccaacttacttctgacaacgatcggaggaccgaaggagctaaccgcttttttgcacaacatgggggatcatgtaactcgccttgatcgttgggaaccggagctgaatgaagccataccaaacgacgagcgtgacaccacgatgcctgtagcaatggcaacaacgttgcgcaaactattaactggcgaactacttactctagcttcccggcaacaattaatagactggatggaggcggataaagttgcaggaccacttctgcgctcggcccttccggctggctggtttattgctgataaatctggagccggtgagcgtgggtctcgcggtatcattgcagcactggggccagatggtaagccctcccgtatcgtagttatctacacgacggggagtcaggcaactatggatgaacgaaatagacagatcgctgagataggtgcctcactgattaagcattggtaactgtcagaccaagtttactcatatatactttagattgatttaaaacttcatttttaatttaaaaggatctaggtgaagatcctttttgataatctcatgaccaaaatcccttaacgtgagttttcgttccactgagcgtcagaccccgtagaaaagatcaaaggatcttcttgagatcctttttttctgcgcgtaatctgctgcttgcaaacaaaaaaaccaccgctaccagcggtggtttgtttgccggatcaagagctaccaactctttttccgaaggtaactggcttcagcagagcgcagataccaaatactgttcttctagtgtagccgtagttaggccaccacttcaagaactctgtagcaccgcctacatacctcgctctgctaatcctgttaccagtggctgctgccagtggcgataagtcgtgtcttaccgggttggactcaagacgatagttaccggataaggcgcagcggtcgggctgaacggggggttcgtgcacacagcccagcttggagcgaacgacctacaccgaactgagatacctacagcgtgagctatgagaaagcgccacgcttcccgaagggagaaaggcggacaggtatccggtaagcggcagggtcggaacaggagagcgcacgagggagcttccagggggaaacgcctggtatctttatagtcctgtcgggtttcgccacctctgacttgagcgtcgatttttgtgatgctcgtcaggggggcggagcctatggaaaaacgccagcaacgcggcctttttacggttcctggccttttgctggccttttgctcacatgttctttcctgcgttatcccctgattctgtggataaccgtattaccgcctttgagtgagctgataccgctcgccgcagccgaacgaccgagcgcagcgagtcagtgagcgaggaagcggaagagcgcccaatacgcaaaccgcctctccccgcgcgttggccgattcattaatgcagctggcacgacaggtttcccgactggaaagcgggcagtgagcgcaacgcaattaatgtgagttagctcactcattaggcaccccaggctttacactttatgcttccggctcgtatgttgtgtggaattgtgagcggataacaatttcacacaggaaacagctatgaccatgattacgccaagcgcgcaattaaccctcactaaagggaacaaaagctggagctgcaagctt

SEQ ID NO: 37 - DNA, 11492 bp, synthetic construct
  source 1..11492: mol_type = other DNA
aatgtagtcttatgcaatactcttgtagtcttgcaacatggtaacgatgagttagcaacatgccttacaaggagagaaaaagcaccgtgcatgccgattggtggaagtaaggtggtacgatcgtgccttattaggaaggcaacagacgggtctgacatggattggacgaaccactgaattgccgcattgcagagatattgtatttaagtgcctagctcgatacataaacgggtctctctggttagaccagatctgagcctgggagctctctggctaactagggaacccactgcttaagcctcaataaagcttgccttgagtgcttcaagtagtgtgtgcccgtctgttgtgtgactctggtaactagagatccctcagacccttttagtcagtgtggaaaatctctagcagtggcgcccgaacagggacttgaaagcgaaagggaaaccagaggagctctctcgacgcaggactcggcttgctgaagcgcgcacggcaagaggcgaggggcggcgactggtgagtacgccaaaaattttgactagcggaggctagaaggagagagatgggtgcgagagcgtcagtattaagcgggggagaattagatcgcgatgggaaaaaattcggttaaggccagggggaaagaaaaaatataaattaaaacatatagtatgggcaagcagggagctagaacgattcgcagttaatcctggcctgttagaaacatcagaaggctgtagacaaatactgggacagctacaaccatcccttcagacaggatcagaagaacttagatcattatataatacagtagcaaccctctattgtgtgcatcaaaggatagagataaaagacaccaaggaagctttagacaagatagaggaagagcaaaacaaaagtaagaccaccgcacagcaagcggccgctgatcttcagacctggaggaggagatatgagggacaattggagaagtgaattatataaatataaagtagtaaaaattgaaccattaggagtagcacccaccaaggcaaagagaagagtggtgcagagagaaaaaagagcagtgggaataggagctttgttccttgggttcttgggagcagcaggaagcactatgggcgcagcgtcaatgacgctgacggtacaggccagacaattattgtctggtatagtgcagcagcagaacaatttgctgagggctattgaggcgcaacagcatctgttgcaactcacagtctggggcatcaagcagctccaggcaagaatcctggctgtggaaagatacctaaaggatcaacagctcctggggatttggggttgctctggaaaactcatttgcaccactgctgtgccttggaatgctagttggagtaataaatctctggaacagatttggaatcacacgacctggatggagtgggacagagaaattaacaattacacaagcttaatacactccttaattgaagaatcgcaaaaccagcaagaaaagaatgaacaagaattattggaattagataaatgggcaagtttgtggaattggtttaacataacaaattggctgtggtatataaaattattcataatgatagtaggaggcttggtaggtttaagaatagtttttgctgtactttctatagtgaatagagttaggcagggatattcaccattatcgtttcagacccacctcccaaccccgaggggacccgacaggcccgaaggaatagaagaagaaggtggagagagagacagagacagatccattcgattagtgaacggatctcgacggtatcgctagcttttaaaagaaaaggggggattggggggtacagtgcaggggaaagaatagtagacataatagcaacagacatacaaactaaagaattacaaaaacaaattacaaaaattcaaaattttactagtgattatcggattgataatcgaattccacgtgtttactccctatcagtgatagagaacgtatgaagagtttactccctatcagtgatagagaacgtatgcagactttactccctatcagtgatagagaacgtataaggagtttactccctatcagtgatagagaacgtatgaccagtttactccctatcagtgatagagaacgtatctacagtttactccctatcagtgatagagaacgtatatccagtttactccctatcagtgatagagaacgtataagctttaggcgtgtacggtgggcgcctataaaagcagagctcgtttagtgaaccgtcagatcgcctggagcaattccacaacacttttgtcttataccaactttccgtaccacttcctaccctcgtaaactcgaggccgccaccatggctggccacctggcctctgccttcgccttctctcccccacctggcggcggcggtgccggccccggaggacccgcccctggatgggtggcccctagaacctggctgtcattccagggacctcctggcggacccggcatcggacctggcgtcgggcccggcagcgccgtgtggggcatacctccctgccctcccccctacgccttctgcgggggcatggcctactgtggcccccaggtcggggtcggcctggtgccccagggcggcctcgccaccagccagcccgccggcgccgctggtgtcggagtggccagcaactccgccggggccagcccagccccatgcaccgtgactcccggcgcagtgaagctggccaaggccaagctggcccagaatcctgccgcctctcaggccatcaaggcgctccagaaggagctggagcagttcgcgaagctgctgaagcagaagcggatcacgctggggtacacccaggccgacgtcggcctgaccctgggcgtcctgttcggcaaggtgttcagccagaccaccatctgccggttcgaggccctgcagcttagcttcaagaacatgtgcaagctgcgcccacttctgcagaagtgggtggaggaggcggataacaacgagaacctgcaggagatctgcaaggccgagacgctggtgcaggccaggaagcgaaagcggacctccatcgagaaccgcgttcgcgggaacctggagaacctgttcctgcagtgtcccaagcctacactgcagcagatctctcacatagcccagcagctgggcctggagaaggatgtggtgcgagtgtggttctgcaatcggaggcagaagggcaagcgctcttcctccgcctacgcccagagggccgccttcgccgcggcggggtcccccttcagcggcggccccgtgtccttccctctggcccccgggccacacttcgggactcccggctacggcagcccacacttcaccgcgctgtacagcagcgtgccattccctgccggggccgccttcccccccgtgagcgtgacgacgctgggcagccccatgcacagcaatggaagcggagccacgaacttctctctgttaaagcaagcaggagatgttgaagaaaaccccgggcctatggccgtgtccgacgccctgctgccctcattcagcaccttcgcctcaggccccgctggcagagaaaagacactgagacaggctggagcccctaacaaccgctggcgcgaggagctgagtcacatgaaacgcctgccccctgtcctgcctgggcggccatacgacctggccgccgccacggtggccaccgacctggagtcaggcggggccggagccgcctgtggcggctccaacctggcgcccctgccccgcagggagactgaggagttcaacgatctgctggatctggacttcatcctcagtaactctctgacccaccccccagagagtgttgctgctaccgtgagcagcagcgccagcgcgagctctagcagcagccctagcagctccgggcctgccagtgcccccagcacctgcagcttcacctaccccatcagggccggtaacgaccctggtgtggcccccggcggcaccgggggcggactcctgtacggccgggagtccgcccccccgcccaccgcccccttcaacctggcggacatcaacgatgtgagcccctccgggggcttcgtcgccgagctgctgcggccagagctcgaccctgtgtacatccccccacagcagccgcagcccccgggcggcggcctgatggggaagttcgtgctcaaggccagcctgagcgcacccggctctgagtacggaagcccctccgtgatcagtgtgagcaagggaagccccgacggctcacaccccgtggttgtggccccctacaacggcgggccgccacggacctgccccaagatcaagcaggaggcagtgagcagctgcacccatctgggtgcggggccaccactgtccaacggccaccgccccgctgcccatgacttccctctgggcaggcagctgcccagcaggaccacccctacgctgggcctggaggaggtcctgtcctccagggactgccacccggccctgcccctgcccccggggttccacccccaccccggacccaactaccccagcttcctgcctgaccagatgcagccgcaggttccgcccctgcattaccaggagctgatgcccccgggcagctgcatgcccgaggagcctaagcctaagcggggccggcgcagctggccccgcaagcggaccgccacccacacttgcgattacgccgggtgcggcaagacctacacaaagagttcgcacctgaaggcccacctgcgaactcacacgggcgagaagccctaccactgcgactgggacgggtgcggctggaagttcgcccggtccgatgagctgacccggcactatcggaagcacaccgggcacaggcccttccagtgccagaagtgtgaccgggccttcagccggtcagaccatctggcactgcacatgaagcgccacttcggaagcggagagggcaggggaagtcttctaacatgcggggacgtggaggaaaatcccggccccatgcccctgaatgtgtccttcaccaaccgcaactatgatctggactatgactctgtgcagccttacttctactgcgatgaggaggagaacttctaccagcagcagcagcagagcgaactgcagccacccgccccatccgaggatatctggaggaggttcgagctgctgccgacccctcctctcagcccctccaggaggagcgggctgtgcagtcccagctacgtggctgtgacccccttctccctgcgcggcgacaacgacggcgggggggggagcttcagcaccgctgaccagctggagatggtcaccgagctgctgggtggcgacatggtcaaccagagcttcatctgcgaccctgatgatgagacattcatcaggaacatcatcatccaggactgcatgtggtccggcttctcggccgctgccaggctggtcagcgagaggctggccagctaccaggccgcccggagggattccgggtcgcctaaccccgccaggggccacagcgtctgctccacgagcagcctgtacctgcaggatctgagcgccgccgccagcgagtgcatagatccttcagtggtgttcccatacccactgaacgacagcagctctcccaggagctgcgcctcgcaggacagcagcgccttcagcccctcgtccgactcgctgctgtccagcaccgagtcgagcccccagggctctcctgagcccctggtgctgcacgaggagacccctcctaccacctcctcggactccgaggaggagcaggaggatgaggaagagatcgacgtggtcagcgtggagaggcgccaggctcctggcaggcgcagcgagtctggcagcccctccgccgggggccacagcaggcccccgcacagcccgctggtgctgaggcggtgtcacgtgagcacccaccagcataactatgctgcgcctccttccaccaggagggactaccccgctgccaggcgggtgaggctggatagcgtccgggtgctgaggcagatcagcaataaccgtaggtgcacctcccccaggagcagtgacacagaggagaacgtgaggaggcggactcacaacgttctggagcgccagcgccggaacgagctgaggcggtccttcttcgctctgagggaccagatcccagagctggagaacaatgagagggcaccgagggtggtcatcctgaggagggccaccgcgtatatcctgagcgtgcaggctgaggagcagaggctgatcagcgaggaggacttgctgaggaggcggcgcgagcagctgaggcacaggctggagcagctgcgaaacagctgcgccggaagcggacagtgtactaattatgctctcttgaaattggctggagatgttgagagcaacccaggtcccatgtacaacatgatggagacagagctgaagccccccgggcctcagcagaccagcggcggcggcgggggcaactccaccgccgccgctgctgggggcaaccagaagaacagccccgatagggtgaagcgccctatgaacgccttcatggtgtggtcccgcggccagcgccgtaagatggctcaggagaaccctaagatgcacaactccgagatcagcaagcggctgggcgcggagtggaagctgctgtcggagaccgagaagcggccattcatcgacgaggccaagaggcttcgtgccctgcacatgaaggagcatcctgactacaagtaccggccccgccggaagaccaagacactgatgaagaaggacaagtacaccttgcctgggggcctgctggcccccgggggcaactccatggcttccggcgtgggcgtgggagccggtctaggcgctggcgtgaaccagcgcatggactcctacgctcacatgaacggctggagcaacgggtcctacagcatgatgcaggaccagttgggctacccccagcaccctgggctgaacgcccatggggctgcccagatgcagcccatgcatcggtacgacgtgagtgccctgcagtacaactccatgacatctagccagacctacatgaacgggagtcccacctacagcatgagctatagccagcaggggaccccaggcatggccctggggtccatgggctccgtggtgaagtcggaggccagctcctcacctcccgtggtgacaagctcctcccacagccgggccccctgccaggctggggatctgagggacatgatctccatgtacctcccgggcgccgaggtgcccgagcctgctgctcccagcaggctgcatatgagccagcattaccagtccgggcccgtgcccggcactgccatcaatgggacactgccactgtcccatatgtgaggcgcgccgataatcaacctctggattacaaaatttgtgaaagattgactggtattcttaactatgttgctccttttacgctatgtggatacgctgctttaatgcctttgtatcatgctattgcttcccgtatggctttcattttctcctccttgtataaatcctggttgctgtctctttatgaggagttgtggcccgttgtcaggcaacgtggcgtggtgtgcactgtgtttgctgacgcaacccccactggttggggcattgccaccacctgtcagctcctttccgggactttcgctttccccctccctattgccacggcggaactcatcgccgcctgccttgcccgctgctggacaggggctcggctgttgggcactgacaattccgtggtgttgtcggggaagctgacgtcctttccatggctgctcgcctgtgttgccacctggattctgcgcgggacgtccttctgctacgtcccttcggccctcaatccagcggaccttccttcccgcggcctgctgccggctctgcggcctcttccgcgtcttcgccttcgccctcagacgagtcggatctccctttgggccgcctccccgcatcgggaattcccgcggttcgaacgcgatcgcttggtacctttaagaccaatgacttacaaggcagctgtagatcttagccactttttaaaagaaaaggggggactggaagggctaattcactcccaacgaagacaagatctgctttttgcttgtactgggtctctctggttagaccagatctgagcctgggagctctctggctaactagggaacccactgcttaagcctcaataaagcttgccttgagtgcttcaagtagtgtgtgcccgtctgttgtgtgactctggtaactagagatccctcagacccttttagtcagtgtggaaaatctctagcagtagtagttcatgtcatcttattattcagtatttataacttgcaaagaaatgaatatcagagagtgagaggaacttgtttattgcagcttataatggttacaaataaagcaatagcatcacaaatttcacaaataaagcatttttttcactgcattctagttgtggtttgtccaaactcatcaatgtatcttatcatgtctggctctagctatcccgcccctaactccgcccatcccgcccctaactccgcccagttccgcccattctccgccccatggctgactaattttttttatttatgcagaggccgaggccgcctcggcctctgagctattccagaagtagtgaggaggcttttttggaggcctagggacgtacccaattcgccctatagtgagtcgtattacgcgcgctcactggccgtcgttttacaacgtcgtgactgggaaaaccctggcgttacccaacttaatcgccttgcagcacatccccctttcgccagctggcgtaatagcgaagaggcccgcaccgatcgcccttcccaacagttgcgcagcctgaatggcgaatgggacgcgccctgtagcggcgcattaagcgcggcgggtgtggtggttacgcgcagcgtgaccgctacacttgccagcgccctagcgcccgctcctttcgctttcttcccttcctttctcgccacgttcgccggctttccccgtcaagctctaaatcgggggctccctttagggttccgatttagtgctttacggcacctcgaccccaaaaaacttgattagggtgatggttcacgtagtgggccatcgccctgatagacggtttttcgccctttgacgttggagtccacgttctttaatagtggactcttgttccaaactggaacaacactcaaccctatctcggtctattcttttgatttataagggattttgccgatttcggcctattggttaaaaaatgagctgatttaacaaaaatttaacgcgaattttaacaaaatattaacgcttacaatttaggtggcacttttcggggaaatgtgcgcggaacccctatttgtttatttttctaaatacattcaaatatgtatccgctcatgagacaataaccctgataaatgcttcaataatattgaaaaaggaagagtatgagtattcaacatttccgtgtcgcccttattcccttttttgcggcattttgccttcctgtttttgctcacccagaaacgctggtgaaagtaaaagatgctgaagatcagttgggtgcacgagtgggttacatcgaactggatctcaacagcggtaagatccttgagagttttcgccccgaagaacgttttccaatgatgagcacttttaaagttctgctatgtggcgcggtattatcccgtattgacgccgggcaagagcaactcggtcgccgcatacactattctcagaatgacttggttgagtactcaccagtcacagaaaagcatcttacggatggcatgacagtaagagaattatgcagtgctgccataaccatgagtgataacactgcggccaacttacttctgacaacgatcggaggaccgaaggagctaaccgcttttttgcacaacatgggggatcatgtaactcgccttgatcgttgggaaccggagctgaatgaagccataccaaacgacgagcgtgacaccacgatgcctgtagcaatggcaacaacgttgcgcaaactattaactggcgaactacttactctagcttcccggcaacaattaatagactggatggaggcggataaagttgcaggaccacttctgcgctcggcccttccggctggctggtttattgctgataaatctggagccggtgagcgtgggtctcgcggtatcattgcagcactggggccagatggtaagccctcccgtatcgtagttatctacacgacggggagtcaggcaactatggatgaacgaaatagacagatcgctgagataggtgcctcactgattaagcattggtaactgtcagaccaagtttactcatatatactttagattgatttaaaacttcatttttaatttaaaaggatctaggtgaagatcctttttgataatctcatgaccaaaatcccttaacgtgagttttcgttccactgagcgtcagaccccgtagaaaagatcaaaggatcttcttgagatcctttttttctgcgcgtaatctgctgcttgcaaacaaaaaaaccaccgctaccagcggtggtttgtttgccggatcaagagctaccaactctttttccgaaggtaactggcttcagcagagcgcagataccaaatactgttcttctagtgtagccgtagttaggccaccacttcaagaactctgtagcaccgcctacatacctcgctctgctaatcctgttaccagtggctgctgccagtggcgataagtcgtgtcttaccgggttggactcaagacgatagttaccggataaggcgcagcggtcgggctgaacggggggttcgtgcacacagcccagcttggagcgaacgacctacaccgaactgagatacctacagcgtgagctatgagaaagcgccacgcttcccgaagggagaaaggcggacaggtatccggtaagcggcagggtcggaacaggagagcgcacgagggagcttccagggggaaacgcctggtatctttatagtcctgtcgggtttcgccacctctgacttgagcgtcgatttttgtgatgctcgtcaggggggcggagcctatggaaaaacgccagcaacgcggcctttttacggttcctggccttttgctggccttttgctcacatgttctttcctgcgttatcccctgattctgtggataaccgtattaccgcctttgagtgagctgataccgctcgccgcagccgaacgaccgagcgcagcgagtcagtgagcgaggaagcggaagagcgcccaatacgcaaaccgcctctccccgcgcgttggccgattcattaatgcagctggcacgacaggtttcccgactggaaagcgggcagtgagcgcaacgcaattaatgtgagttagctcactcattaggcaccccaggctttacactttatgcttccggctcgtatgttgtgtggaattgtgagcggataacaatttcacacaggaaacagctatgaccatgattacgccaagcgcgcaattaaccctcactaaagggaacaaaagctggagctgcaagctt

SEQ ID NO: 38 - DNA, 7920 bp, synthetic construct
  source 1..7920: mol_type = other DNA
agcgcccaatacgcaaaccgcctctccccgcgcgttggccgattcattaatgcagctggcacgacaggtttcccgactggaaagcgggcagtgagcgcaacgcaattaatgtgagttagctcactcattaggcaccccaggctttacactttatgcttccggctcgtatgttgtgtggaattgtgagcggataacaatttcacacaggaaacagctatgaccatgattacgaattgcctgcaggcagctgcgcgctcgctcgctcactgaggccgcccgggcaaagcccgggcgtcgggcgacctttggtcgcccggcctcagtgagcgagcgagcgcgcagagagggagtggccaactccatcactaggggttcctatcgatatcaagcttactagtgattatcggattgataatcgaattccacgtgtttactccctatcagtgatagagaacgtatgaagagtttactccctatcagtgatagagaacgtatgcagactttactccctatcagtgatagagaacgtataaggagtttactccctatcagtgatagagaacgtatgaccagtttactccctatcagtgatagagaacgtatctacagtttactccctatcagtgatagagaacgtatatccagtttactccctatcagtgatagagaacgtataagctttaggcgtgtacggtgggcgcctataaaagcagagctcgtttagtgaaccgtcagatcgcctggagcaattccacaacacttttgtcttataccaactttccgtaccacttcctaccctcgtaaagaattcacctcgaggccgccaccatggctggccacctggcctctgacttcgccttctctcccccacctggcggcggcggtgacggccccggaggacccgagcctggatgggtggaccctagaacctggctgtcattccagggacctcctggcggacccggcatcggacctggcgtcgggcccggcagcgaggtgtggggcatacctccctgccctcccccctacgagttctgcgggggcatggcctactgtggcccccaggtcggggtcggcctggtgccccagggcggcctcgaaaccagccagcccgagggcgaggctggtgtcggagtggagagcaactccgacggggccagcccagagccatgcaccgtgactcccggcgcagtgaagctggaaaaggagaagctggagcagaatcctgaggagtctcaggacatcaaggcgctccagaaggagctggagcagttcgcgaagctgctgaagcagaagcggatcacgctggggtacacccaggccgacgtcggcctgaccctgggcgtcctgttcggcaaggtgttcagccagaccaccatctgccggttcgaggccctgcagcttagcttcaagaacatgtgcaagctgcgcccacttctgcagaagtgggtggaggaggcggataacaacgagaacctgcaggagatctgcaaggccgagacgctggtgcaggccaggaagcgaaagcggacctccatcgagaaccgcgttcgcgggaacctggagaacctgttcctgcagtgtcccaagcctacactgcagcagatctctcacatagcccagcagctgggcctggagaaggatgtggtgcgagtgtggttctgcaatcggaggcagaagggcaagcgctcttcctccgattacgcccagagggaggacttcgaggcggcggggtcccccttcagcggcggccccgtgtccttccctctggcccccgggccacacttcgggactcccggctacggcagcccacacttcaccgcgctgtacagcagcgtgccattccctgagggggaggccttcccccccgtgagcgtgacgacgctgggcagccccatgcacagcaatggaagcggagccacgaacttctctctgttaaagcaagcaggagatgttgaagaaaaccccgggcctatggccgtgtccgacgccctgctgccctcattcagcaccttcgcctcaggccccgctggcagagaaaagacactgagacaggctggagcccctaacaaccgctggcgcgaggagctgagtcacatgaaacgcctgccccctgtcctgcctgggcggccatacgacctggccgccgccacggtggccaccgacctggagtcaggcggggccggagccgcctgtggcggctccaacctggcgcccctgccccgcagggagactgaggagttcaacgatctgctggatctggacttcatcctcagtaactctctgacccaccccccagagagtgttgctgctaccgtgagcagcagcgccagcgcgagctctagcagcagccctagcagctccgggcctgccagtgcccccagcacctgcagcttcacctaccccatcagggccggtaacgaccctggtgtggcccccggcggcaccgggggcggactcctgtacggccgggagtccgcccccccgcccaccgcccccttcaacctggcggacatcaacgatgtgagcccctccgggggcttcgtcgccgagctgctgcggccagagctcgaccctgtgtacatccccccacagcagccgcagcccccgggcggcggcctgatggggaagttcgtgctcaaggccagcctgagcgcacccggctctgagtacggaagcccctccgtgatcagtgtgagcaagggaagccccgacggctcacaccccgtggttgtggccccctacaacggcgggccgccacggacctgccccaagatcaagcaggaggcagtgagcagctgcacccatctgggtgcggggccaccactgtccaacggccaccgccccgctgcccatgacttccctctgggcaggcagctgcccagcaggaccacccctacgctgggcctggaggaggtcctgtcctccagggactgccacccggccctgcccctgcccccggggttccacccccaccccggacccaactaccccagcttcctgcctgaccagatgcagccgcaggttccgcccctgcattaccaggagctgatgcccccgggcagctgcatgcccgaggagcctaagcctaagcggggccggcgcagctggccccgcaagcggaccgccacccacacttgcgattacgccgggtgcggcaagacctacacaaagagttcgcacctgaaggcccacctgcgaactcacacgggcgagaagccctaccactgcgactgggacgggtgcggctggaagttcgcccggtccgatgagctgacccggcactatcggaagcacaccgggcacaggcccttccagtgccagaagtgtgaccgggccttcagccggtcagaccatctggcactgcacatgaagcgccacttcggaagcggagagggcaggggaagtcttctaacatgcggggacgtggaggaaaatcccggccccatgtacaacatgatggagacagagctgaagccccccgggcctcagcagaccagcggcggcggcgggggcaactccaccgccgccgctgctgggggcaaccagaagaacagccccgatagggtgaagcgccctatgaacgccttcatggtgtggtcccgcggccagcgccgtaagatggctcaggagaaccctaagatgcacaactccgagatcagcaagcggctgggcgcggagtggaagctgctgtcggagaccgagaagcggccattcatcgacgaggccaagaggcttcgtgccctgcacatgaaggagcatcctgactacaagtaccggccccgccggaagaccaagacactgatgaagaaggacaagtacaccttgcctgggggcctgctggcccccgggggcaactccatggcttccggcgtgggcgtgggagccggtctaggcgctggcgtgaaccagcgcatggactcctacgctcacatgaacggctggagcaacgggtcctacagcatgatgcaggaccagttgggctacccccagcaccctgggctgaacgcccatggggctgcccagatgcagcccatgcatcggtacgacgtgagtgccctgcagtacaactccatgacatctagccagacctacatgaacgggagtcccacctacagcatgagctatagccagcaggggaccccaggcatggccctggggtccatgggctccgtggtgaagtcggaggccagctcctcacctcccgtggtgacaagctcctcccacagccgggccccctgccaggctggggatctgagggacatgatctccatgtacctcccgggcgccgaggtgcccgagcctgctgctcccagcaggctgcatatgagccagcattaccagtccgggcccgtgcccggcactgccatcaatgggacactgccactgtcccatatgtgaggatccacgggtggcatccctgtgacccctccccagtgcctctcctggccctggaagttgccactccagtgcccaccagccttgtcctaataaaattaagttgcatcattttgtctgactaggtgtccttctataatattatggggtggaggggggtggtatggagcaaggggcaagttgggaagacaacctgtagggcctgcggggtctattgggaaccaagctggagtgcagtggcacaatcttggctcactgcaatctccgcctcctgggttcaagcgattctcctgcctcagcctcccgagttgttgggattccaggcatgcatgaccaggctcagctaatttttgtttttttggtagagacggggtttcaccatattggccaggctggtctccaactcctaatctcaggtgatctacccaccttggcctcccaaattgctgggattacaggcgtgaaccactgctcccttccctgtccttatcgatagatctaggaacccctagtgatggagttggccactccctctctgcgcgctcgctcgctcactgaggccgggcgaccaaaggtcgcccgacgcccgggctttgcccgggcggcctcagtgagcgagcgagcgcgcagctgcctgcaggcagcttggcactggccgtcgttttacaacgtcgtgactgggaaaaccctggcgttacccaacttaatcgccttgcagcacatccccctttcgccagctggcgtaatagcgaagaggcccgcaccgatcgcccttcccaacagttgcgcagcctgaatggcgaatggcgcctgatgcggtattttctccttacgcatctgtgcggtatttcacaccgcatacgtcaaagcaaccatagtacgcgccctgtagcggcgcattaagcgcggcgggtgtggtggttacgcgcagcgtgaccgctacacttgccagcgccctagcgcccgctcctttcgctttcttcccttcctttctcgccacgttcgccggctttccccgtcaagctctaaatcgggggctccctttagggttccgatttagtgctttacggcacctcgaccccaaaaaacttgatttgggtgatggttcacgtagtgggccatcgccctgatagacggtttttcgccctttgacgttggagtccacgttctttaatagtggactcttgttccaaactggaacaacactcaaccctatctcgggctattcttttgatttataagggattttgccgatttcggcctattggttaaaaaatgagctgatttaacaaaaatttaacgcgaattttaacaaaatattaacgtttacaattttatggtgcactctcagtacaatctgctctgatgccgcatagttaagccagccccgacacccgccaacacccgctgacgcgccctgacgggcttgtctgctcccggcatccgcttacagacaagctgtgaccgtctccgggagctgcatgtgtcagaggttttcaccgtcatcaccgaaacgcgcgagacgaaagggcctcgtgatacgcctatttttataggttaatgtcatgataataatggtttcttagacgtcaggtggcacttttcggggaaatgtgcgcggaacccctatttgtttatttttctaaatacattcaaatatgtatccgctcatgagacaataaccctgataaatgcttcaataatattgaaaaaggaagagtatgagtattcaacatttccgtgtcgcccttattcccttttttgcggcattttgccttcctgtttttgctcacccagaaacgctggtgaaagtaaaagatgctgaagatcagttgggtgcacgagtgggttacatcgaactggatctcaacagcggtaagatccttgagagttttcgccccgaagaacgttttccaatgatgagcacttttaaagttctgctatgtggcgcggtattatcccgtattgacgccgggcaagagcaactcggtcgccgcatacactattctcagaatgacttggttgagtactcaccagtcacagaaaagcatcttacggatggcatgacagtaagagaattatgcagtgctgccataaccatgagtgataacactgcggccaacttacttctgacaacgatcggaggaccgaaggagctaaccgcttttttgcacaacatgggggatcatgtaactcgccttgatcgttgggaaccggagctgaatgaagccataccaaacgacgagcgtgacaccacgatgcctgtagcaatggcaacaacgttgcgcaaactattaactggcgaactacttactctagcttcccggcaacaattaatagactggatggaggcggataaagttgcaggaccacttctgcgctcggcccttccggctggctggtttattgctgataaatctggagccggtgagcgtgggtctcgcggtatcattgcagcactggggccagatggtaagccctcccgtatcgtagttatctacacgacggggagtcaggcaactatggatgaacgaaatagacagatcgctgagataggtgcctcactgattaagcattggtaactgtcagaccaagtttactcatatatactttagattgatttaaaacttcatttttaatttaaaaggatctaggtgaagatcctttttgataatctcatgaccaaaatcccttaacgtgagttttcgttccactgagcgtcagaccccgtagaaaagatcaaaggatcttcttgagatcctttttttctgcgcgtaatctgctgcttgcaaacaaaaaaaccaccgctaccagcggtggtttgtttgccggatcaagagctaccaactctttttccgaaggtaactggcttcagcagagcgcagataccaaatactgttcttctagtgtagccgtagttaggccaccacttcaagaactctgtagcaccgcctacatacctcgctctgctaatcctgttaccagtggctgctgccagtggcgataagtcgtgtcttaccgggttggactcaagacgatagttaccggataaggcgcagcggtcgggctgaacggggggttcgtgcacacagcccagcttggagcgaacgacctacaccgaactgagatacctacagcgtgagctatgagaaagcgccacgcttcccgaagggagaaaggcggacaggtatccggtaagcggcagggtcggaacaggagagcgcacgagggagcttccagggggaaacgcctggtatctttatagtcctgtcgggtttcgccacctctgacttgagcgtcgatttttgtgatgctcgtcaggggggcggagcctatggaaaaacgccagcaacgcggcctttttacggttcctggccttttgctggccttttgctcacatgttctttcctgcgttatcccctgattctgtggataaccgtattaccgcctttgagtgagctgataccgctcgccgcagccgaacgaccgagcgcagcgagtcagtgagcgaggaagcggaag

SEQ ID NO: 39 - DNA, 7920 bp, synthetic construct
  source 1..7920: mol_type = other DNA
agcgcccaatacgcaaaccgcctctccccgcgcgttggccgattcattaatgcagctggcacgacaggtttcccgactggaaagcgggcagtgagcgcaacgcaattaatgtgagttagctcactcattaggcaccccaggctttacactttatgcttccggctcgtatgttgtgtggaattgtgagcggataacaatttcacacaggaaacagctatgaccatgattacgaattgcctgcaggcagctgcgcgctcgctcgctcactgaggccgcccgggcaaagcccgggcgtcgggcgacctttggtcgcccggcctcagtgagcgagcgagcgcgcagagagggagtggccaactccatcactaggggttcctatcgatatcaagcttactagtgattatcggattgataatcgaattccacgtgtttactccctatcagtgatagagaacgtatgaagagtttactccctatcagtgatagagaacgtatgcagactttactccctatcagtgatagagaacgtataaggagtttactccctatcagtgatagagaacgtatgaccagtttactccctatcagtgatagagaacgtatctacagtttactccctatcagtgatagagaacgtatatccagtttactccctatcagtgatagagaacgtataagctttaggcgtgtacggtgggcgcctataaaagcagagctcgtttagtgaaccgtcagatcgcctggagcaattccacaacacttttgtcttataccaactttccgtaccacttcctaccctcgtaaagaattcacctcgaggccgccaccatggctggccacctggcctctgccttcgccttctctcccccacctggcggcggcggtgccggccccggaggacccgcccctggatgggtggcccctagaacctggctgtcattccagggacctcctggcggacccggcatcggacctggcgtcgggcccggcagcgccgtgtggggcatacctccctgccctcccccctacgccttctgcgggggcatggcctactgtggcccccaggtcggggtcggcctggtgccccagggcggcctcgccaccagccagcccgccggcgccgctggtgtcggagtggccagcaactccgccggggccagcccagccccatgcaccgtgactcccggcgcagtgaagctggccaaggccaagctggcccagaatcctgccgcctctcaggccatcaaggcgctccagaaggagctggagcagttcgcgaagctgctgaagcagaagcggatcacgctggggtacacccaggccgacgtcggcctgaccctgggcgtcctgttcggcaaggtgttcagccagaccaccatctgccggttcgaggccctgcagcttagcttcaagaacatgtgcaagctgcgcccacttctgcagaagtgggtggaggaggcggataacaacgagaacctgcaggagatctgcaaggccgagacgctggtgcaggccaggaagcgaaagcggacctccatcgagaaccgcgttcgcgggaacctggagaacctgttcctgcagtgtcccaagcctacactgcagcagatctctcacatagcccagcagctgggcctggagaaggatgtggtgcgagtgtggttctgcaatcggaggcagaagggcaagcgctcttcctccgcctacgcccagagggccgccttcgccgcggcggggtcccccttcagcggcggccccgtgtccttccctctggcccccgggccacacttcgggactcccggctacggcagcccacacttcaccgcgctgtacagcagcgtgccattccctgccggggccgccttcccccccgtgagcgtgacgacgctgggcagccccatgcacagcaatggaagcggagccacgaacttctctctgttaaagcaagcaggagatgttgaagaaaaccccgggcctatggccgtgtccgacgccctgctgccctcattcagcaccttcgcctcaggccccgctggcagagaaaagacactgagacaggctggagcccctaacaaccgctggcgcgaggagctgagtcacatgaaacgcctgccccctgtcctgcctgggcggccatacgacctggccgccgccacggtggccaccgacctggagtcaggcggggccggagccgcctgtggcggctccaacctggcgcccctgccccgcagggagactgaggagttcaacgatctgctggatctggacttcatcctcagtaactctctgacccaccccccagagagtgttgctgctaccgtgagcagcagcgccagcgcgagctctagcagcagccctagcagctccgggcctgccagtgcccccagcacctgcagcttcacctaccccatcagggccggtaacgaccctggtgtggcccccggcggcaccgggggcggactcctgtacggccgggagtccgcccccccgcccaccgcccccttcaacctggcggacatcaacgatgtgagcccctccgggggcttcgtcgccgagctgctgcggccagagctcgaccctgtgtacatccccccacagcagccgcagcccccgggcggcggcctgatggggaagttcgtgctcaaggccagcctgagcgcacccggctctgagtacggaagcccctccgtgatcagtgtgagcaagggaagccccgacggctcacaccccgtggttgtggccccctacaacggcgggccgccacggacctgccccaagatcaagcaggaggcagtgagcagctgcacccatctgggtgcggggccaccactgtccaacggccaccgccccgctgcccatgacttccctctgggcaggcagctgcccagcaggaccacccctacgctgggcctggaggaggtcctgtcctccagggactgccacccggccctgcccctgcccccggggttccacccccaccccggacccaactaccccagcttcctgcctgaccagatgcagccgcaggttccgcccctgcattaccaggagctgatgcccccgggcagctgcatgcccgaggagcctaagcctaagcggggccggcgcagctggccccgcaagcggaccgccacccacacttgcgattacgccgggtgcggcaagacctacacaaagagttcgcacctgaaggcccacctgcgaactcacacgggcgagaagccctaccactgcgactgggacgggtgcggctggaagttcgcccggtccgatgagctgacccggcactatcggaagcacaccgggcacaggcccttccagtgccagaagtgtgaccgggccttcagccggtcagaccatctggcactgcacatgaagcgccacttcggaagcggagagggcaggggaagtcttctaacatgcggggacgtggaggaaaatcccggccccatgtacaacatgatggagacagagctgaagccccccgggcctcagcagaccagcggcggcggcgggggcaactccaccgccgccgctgctgggggcaaccagaagaacagccccgatagggtgaagcgccctatgaacgccttcatggtgtggtcccgcggccagcgccgtaagatggctcaggagaaccctaagatgcacaactccgagatcagcaagcggctgggcgcggagtggaagctgctgtcggagaccgagaagcggccattcatcgacgaggccaagaggcttcgtgccctgcacatgaaggagcatcctgactacaagtaccggccccgccggaagaccaagacactgatgaagaaggacaagtacaccttgcctgggggcctgctggcccccgggggcaactccatggcttccggcgtgggcgtgggagccggtctaggcgctggcgtgaaccagcgcatggactcctacgctcacatgaacggctggagcaacgggtcctacagcatgatgcaggaccagttgggctacccccagcaccctgggctgaacgcccatggggctgcccagatgcagcccatgcatcggtacgacgtgagtgccctgcagtacaactccatgacatctagccagacctacatgaacgggagtcccacctacagcatgagctatagccagcaggggaccccaggcatggccctggggtccatgggctccgtggtgaagtcggaggccagctcctcacctcccgtggtgacaagctcctcccacagccgggccccctgccaggctggggatctgagggacatgatctccatgtacctcccgggcgccgaggtgcccgagcctgctgctcccagcaggctgcatatgagccagcattaccagtccgggcccgtgcccggcactgccatcaatgggacactgccactgtcccatatgtgaggatccacgggtggcatccctgtgacccctccccagtgcctctcctggccctggaagttgccactccagtgcccaccagccttgtcctaataaaattaagttgcatcattttgtctgactaggtgtccttctataatattatggggtggaggggggtggtatggagcaaggggcaagttgggaagacaacctgtagggcctgcggggtctattgggaaccaagctggagtgcagtggcacaatcttggctcactgcaatctccgcctcctgggttcaagcgattctcctgcctcagcctcccgagttgttgggattccaggcatgcatgaccaggctcagctaatttttgtttttttggtagagacggggtttcaccatattggccaggctggtctccaactcctaatctcaggtgatctacccaccttggcctcccaaattgctgggattacaggcgtgaaccactgctcccttccctgtccttatcgatagatctaggaacccctagtgatggagttggccactccctctctgcgcgctcgctcgctcactgaggccgggcgaccaaaggtcgcccgacgcccgggctttgcccgggcggcctcagtgagcgagcgagcgcgcagctgcctgcaggcagcttggcactggccgtcgttttacaacgtcgtgactgggaaaaccctggcgttacccaacttaatcgccttgcagcacatccccctttcgccagctggcgtaatagcgaagaggcccgcaccgatcgcccttcccaacagttgcgcagcctgaatggcgaatggcgcctgatgcggtattttctccttacgcatctgtgcggtatttcacaccgcatacgtcaaagcaaccatagtacgcgccctgtagcggcgcattaagcgcggcgggtgtggtggttacgcgcagcgtgaccgctacacttgccagcgccctagcgcccgctcctttcgctttcttcccttcctttctcgccacgttcgccggctttccccgtcaagctctaaatcgggggctccctttagggttccgatttagtgctttacggcacctcgaccccaaaaaacttgatttgggtgatggttcacgtagtgggccatcgccctgatagacggtttttcgccctttgacgttggagtccacgttctttaatagtggactcttgttccaaactggaacaacactcaaccctatctcgggctattcttttgatttataagggattttgccgatttcggcctattggttaaaaaatgagctgatttaacaaaaatttaacgcgaattttaacaaaatattaacgtttacaattttatggtgcactctcagtacaatctgctctgatgccgcatagttaagccagccccgacacccgccaacacccgctgacgcgccctgacgggcttgtctgctcccggcatccgcttacagacaagctgtgaccgtctccgggagctgcatgtgtcagaggttttcaccgtcatcaccgaaacgcgcgagacgaaagggcctcgtgatacgcctatttttataggttaatgtcatgataataatggtttcttagacgtcaggtggcacttttcggggaaatgtgcgcggaacccctatttgtttatttttctaaatacattcaaatatgtatccgctcatgagacaataaccctgataaatgcttcaataatattgaaaaaggaagagtatgagtattcaacatttccgtgtcgcccttattcccttttttgcggcattttgccttcctgtttttgctcacccagaaacgctggtgaaagtaaaagatgctgaagatcagttgggtgcacgagtgggttacatcgaactggatctcaacagcggtaagatccttgagagttttcgccccgaagaacgttttccaatgatgagcacttttaaagttctgctatgtggcgcggtattatcccgtattgacgccgggcaagagcaactcggtcgccgcatacactattctcagaatgacttggttgagtactcaccagtcacagaaaagcatcttacggatggcatgacagtaagagaattatgcagtgctgccataaccatgagtgataacactgcggccaacttacttctgacaacgatcggaggaccgaaggagctaaccgcttttttgcacaacatgggggatcatgtaactcgccttgatcgttgggaaccggagctgaatgaagccataccaaacgacgagcgtgacaccacgatgcctgtagcaatggcaacaacgttgcgcaaactattaactggcgaactacttactctagcttcccggcaacaattaatagactggatggaggcggataaagttgcaggaccacttctgcgctcggcccttccggctggctggtttattgctgataaatctggagccggtgagcgtgggtctcgcggtatcattgcagcactggggccagatggtaagccctcccgtatcgtagttatctacacgacggggagtcaggcaactatggatgaacgaaatagacagatcgctgagataggtgcctcactgattaagcattggtaactgtcagaccaagtttactcatatatactttagattgatttaaaacttcatttttaatttaaaaggatctaggtgaagatcctttttgataatctcatgaccaaaatcccttaacgtgagttttcgttccactgagcgtcagaccccgtagaaaagatcaaaggatcttcttgagatcctttttttctgcgcgtaatctgctgcttgcaaacaaaaaaaccaccgctaccagcggtggtttgtttgccggatcaagagctaccaactctttttccgaaggtaactggcttcagcagagcgcagataccaaatactgttcttctagtgtagccgtagttaggccaccacttcaagaactctgtagcaccgcctacatacctcgctctgctaatcctgttaccagtggctgctgccagtggcgataagtcgtgtcttaccgggttggactcaagacgatagttaccggataaggcgcagcggtcgggctgaacggggggttcgtgcacacagcccagcttggagcgaacgacctacaccgaactgagatacctacagcgtgagctatgagaaagcgccacgcttcccgaagggagaaaggcggacaggtatccggtaagcggcagggtcggaacaggagagcgcacgagggagcttccagggggaaacgcctggtatctttatagtcctgtcgggtttcgccacctctgacttgagcgtcgatttttgtgatgctcgtcaggggggcggagcctatggaaaaacgccagcaacgcggcctttttacggttcctggccttttgctggccttttgctcacatgttctttcctgcgttatcccctgattctgtggataaccgtattaccgcctttgagtgagctgataccgctcgccgcagccgaacgaccgagcgcagcgagtcagtgagcgaggaagcggaag

SEQ ID NO: 40 - protein, 97 aa, synthetic construct
MGRRSWPRKRTATHTCDYAGCGKTYTKSSHLKAHLRTHTGEKPYHCDWDGCGWKFARSDELTRHYRKHTGHRPFQCQKCDRAFSRSDHLALHMKRHF

SEQ ID NO: 41 - protein, 161 aa, synthetic construct
MVKRPMNAFMVWSRGQRRKMAQENPKMHNSEISKRLGAEWKLLSETEKRPFIDEAKRLRALHMKEHPDYKYRPRRKTKTLMKKDKYTLPGGLLAPGGNSMASGVGVGAGLGAGVNQRMDSYAHMNGWSNGSYSMMQDQLGYPQHPGLNAHGAAQMQPMHRY

SEQ ID NO: 42 - protein, 200 aa, synthetic construct
MYNMMETELKPPGPQQTSGGGGGNSTAAAAGGNQKNSPDRVKRPMNAFMVWSRGQRRKMAQENPKMHNSEISKRLGAEWKLLSETEKRPFIDEAKRLRALHMKEHPDYKYRPRRKTKTLMKKDKYTLPGGLLAPGGNSMASGVGVGAGLGAGVNQRMDSYAHMNGWSNGSYSMMQDQLGYPQHPGLNAHGAAQMQPMHRY

SEQ ID NO: 43 - protein, 278 aa, synthetic construct
MVKRPMNAFMVWSRGQRRKMAQENPKMHNSEISKRLGAEWKLLSETEKRPFIDEAKRLRALHMKEHPDYKYRPRRKTKTLMKKDKYTLPGGLLAPGGNSMASGVGVGAGLGAGVNQRMDSYAHMNGWSNGSYSMMQDQLGYPQHPGLNAHGAAQMQPMHRYDVSALQYNSMTSSQTYMNGSPTYSMSYSQQGTPGMALGSMGSVVKSEASSSPPVVTSSSHSRAPCQAGDLRDMISMYLPGAEVPEPAAPSRLHMSQHYQSGPVPGTAINGTLPLSHM

SEQ ID NO: 44 - protein, 161 aa, synthetic construct
MALQKELEQFAKLLKQKRITLGYTQADVGLTLGVLFGKVFSQTTICRFEALQLSFKNMCKLRPLLQKWVEEADNNENLQEICKAETLVQARKRKRTSIENRVRGNLENLFLQCPKPTLQQISHIAQQLGLEKDVVRVWFCNRRQKGKRSSSDYAQREDFEA

SEQ ID NO: 45 - protein, 300 aa, synthetic construct
MAGHLASDFAFSPPPGGGGDGPGGPEPGWVDPRTWLSFQGPPGGPGIGPGVGPGSEVWGIPPCPPPYEFCGGMAYCGPQVGVGLVPQGGLETSQPEGEAGVGVESNSDGASPEPCTVTPGAVKLEKEKLEQNPEESQDIKALQKELEQFAKLLKQKRITLGYTQADVGLTLGVLFGKVFSQTTICRFEALQLSFKNMCKLRPLLQKWVEEADNNENLQEICKAETLVQARKRKRTSIENRVRGNLENLFLQCPKPTLQQISHIAQQLGLEKDVVRVWFCNRRQKGKRSSSDYAQREDFEA

SEQ ID NO: 46 - protein, 234 aa, synthetic construct
MALQKELEQFAKLLKQKRITLGYTQADVGLTLGVLFGKVFSQTTICRFEALQLSFKNMCKLRPLLQKWVEEADNNENLQEICKAETLVQARKRKRTSIENRVRGNLENLFLQCPKPTLQQISHIAQQLGLEKDVVRVWFCNRRQKGKRSSSDYAQREDFEASSSDYAQREDFEAAGSPFSGGPVSFPLAPGPHFGTPGYGSPHFTALYSSVPFPEGEAFPPVSVTTLGSPMHSN

SEQ ID NO: 47 - protein, 80 aa, synthetic construct
MVLERQRRNELKRSFFALRDQIPELENNEKAPKVVILKKATAYILSVQAEEQKLISEEDLLRKRREQLKHKLEQLRNSCA

SEQ ID NO: 48 - protein, 300 aa, synthetic construct
MAAKLVSEKLASYQAARKDSGSPNPARGHSVCSTSSLYLQDLSAAASECIDPSVVFPYPLNDSSSPKSCASQDSSAFSPSSDSLLSSTESSPQGSPEPLVLHEETPPTTSSDSEEEQEDEEEIDVVSVEKRQAPGKRSESGSPSAGGHSKPPHSPLVLKRCHVSTHQHNYAAPPSTRKDYPAAKRVKLDSVRVLRQISNNRKCTSPRSSDTEENVKRRTHNVLERQRRNELKRSFFALRDQIPELENNEKAPKVVILKKATAYILSVQAEEQKLISEEDLLRKRREQLKHKLEQLRNSCA

SEQ ID NO: 49 - DNA, 283 bp, synthetic construct
  source 1..283: mol_type = other DNA
gagaccctcgaccgtcgattgtccactggtcaacaatagatgacttacaactaatcggaaggtgcagagactcgacgggagctaccctaacgtcaagacgagggtaaagagagagtccaattctcaaagccaataggcagtagcgaaagctgcaagagaatgaaaatccgttgaccttaaacggtcgtgtgggttcaagtccctccacccccacgccggaaacgcaatagccgaaaaacaaaaaacaaaaaaaacaaaaaaaaaaccaaaaaaacaaaacaca

SEQ ID NO: 50 - DNA, 206 bp, synthetic construct
  source 1..206: mol_type = other DNA
aaaaaacaaaaaacaaaacggctattatgcgttaccggcgagacgctacggacttaaataattgagccttaaagaagaaattctttaagtggatgctctcaaactcagggaaacctaaatctagttatagacaaggcaatcctgagccaagccgaagtagtaattagtaagaccagtggacaatcgacggataacagcatatctag

SEQ ID NO: 51 - DNA, 199 bp, synthetic construct
  source 1..199: mol_type = other DNA
gggagaccctcgaatggaatttgcgccgatgaaggtgtagagactagacggcacccacctaaggcaaacgctatggtgaaggcatagtccagggagtggcgaaagtcacacaaaccggaatattggactcgccggaaacgcaatagccgaaaaacaaaaaacaaaaaaaacaaaaaaaaaaccaaaaaaacaaaacaca

SEQ ID NO: 52 - DNA, 188 bp, synthetic construct
  source 1..188: mol_type = other DNA
aaaaaacaaaaaacaaaacggctattatgcgttaccggcgatgctcaatgtacctatttctatgggccttgcgccgggaaaccacgcaagggatggtgtcaaattcggcgaaacctaagcgcccgcccgggcgtatggcaacgccgagccaagcttcggcgccaattccatttatcagatttctagag

SEQ ID NO: 53 - DNA, 2559 bp, synthetic construct
  source 1..2559: mol_type = other DNA
gagaccctcgaccgtcgattgtccactggtcaacaatagatgacttacaactaatcggaaggtgcagagactcgacgggagctaccctaacgtcaagacgagggtaaagagagagtccaattctcaaagccaataggcagtagcgaaagctgcaagagaatgaaaatccgttgaccttaaacggtcgtgtgggttcaagtccctccacccccacgccggaaacgcaatagccgaaaaacaaaaaacaaaaaaaacaaaaaaaaaaccaaaaaaacaaaacacattaaaacagcctgtgggttgatcccacccacaggcccattgggcgctagcactctggtatcacggtacctttgtgcgcctgttttataccccctcccccaactgtaacttagaagtaacacacaccgatcaacagtcagcgtggcacaccagccacgttttgatcaagcacttctgttaccccggactgagtatcaatagactgctcacgcggttgaaggagaaagcgttcgttatccggccaactacttcgaaaaacctagtaacaccgtggaagttgcagagtgtttcgctcagcactaccccagtgtagatcaggtcgatgagtcaccgcattccccacgggcgaccgtggcggtggctgcgttggcggcctgcccatggggaaacccatgggacgctctaatacagacatggtgcgaagagtctattgagctagttggtagtcctccggcccctgaatgcggctaatcctaactgcggagcacacaccctcaagccagagggcagtgtgtcgtaacgggcaactctgcagcggaaccgactactttgggtgtccgtgtttcattttattcctatactggctgcttatggtgacaattgagagatcgttaccatatagctattggattggccatccggtgactaatagagctattatatatccctttgttgggtttataccacttagcttgaaagaggttaaaacattacaattcattgttaagttgaatacagcaaaatgcccctgaatgtgtccttcaccaaccgcaactatgatctggactatgactctgtgcagccttacttctactgcgatgaggaggagaacttctaccagcagcagcagcagagcgaactgcagccacccgccccatccgaggatatctggaagaagttcgagctgctgccggctcctcctctcagcccctccaggaggagcgggctgtgcagtcccagctacgtggctgtgacccccttctccctgcgcggcgacaacgacggcgggggggggagcttcagcaccgctgaccagctggagatggtcaccgagctgctgggtggcgacatggtcaaccagagcttcatctgcgaccctgatgatgagacattcatcaagaacatcatcatccaggactgcatgtggtccggcttctcggccgctgccaagctggtcagcgagaagctggccagctaccaggccgcccggaaggattccgggtcgcctaaccccgccaggggccacagcgtctgctccacgagcagcctgtacctgcaggatctgagcgccgccgccagcgagtgcatagatccttcagtggtgttcccatacccactgaacgacagcagctctcccaagagctgcgcctcgcaggacagcagcgccttcagcccctcgtccgactcgctgctgtccagcaccgagtcgagcccccagggctctcctgagcccctggtgctgcacgaggagacccctcctaccacctcctcggactccgaggaggagcaggaggatgaggaagagatcgacgtggtcagcgtggagaagcgccaggctcctggcaagcgcagcgagtctggcagcccctccgccgggggccacagcaagcccccgcacagcccgctggtgctgaagcggtgtcacgtgagcacccaccagcataactatgctgcgcctccttccaccaggaaggactaccccgctgccaagcgggtgaagctggatagcgtccgggtgctgaggcagatcagcaataaccgtaagtgcacctcccccaggagcagtgacacagaggagaacgtgaagaggcggactcacaacgttctggagcgccagcgccggaacgagctgaagcggtccttcttcgctctgagggaccagatcccagagctggagaacaatgagaaggcaccgaaggtggtcatcctgaagaaggccaccgcgtatatcctgagcgtgcaggctgaggagcagaagctgatcagcgaggaggacttgctgaggaagcggcgcgagcagctgaaacacaagctggagcagctgcgaaacagctgcgcctagtgataatgaaaaaaacaaaaaacaaaacggctattatgcgttaccggcgagacgctacggacttaaataattgagccttaaagaagaaattctttaagtggatgctctcaaactcagggaaacctaaatctagttatagacaaggcaatcctgagccaagccgaagtagtaattagtaagaccagtggacaatcgacggataacagcatatctag

SEQ ID NO: 54 - DNA, 2652 bp, synthetic construct
  source 1..2652: mol_type = other DNA
gagaccctcgaccgtcgattgtccactggtcaacaatagatgacttacaactaatcggaaggtgcagagactcgacgggagctaccctaacgtcaagacgagggtaaagagagagtccaattctcaaagccaataggcagtagcgaaagctgcaagagaatgaaaatccgttgaccttaaacggtcgtgtgggttcaagtccctccacccccacgccggaaacgcaatagccgaaaaacaaaaaacaaaaaaaacaaaaaaaaaaccaaaaaaacaaaacacattaaaacagcctgtgggttgatcccacccacaggcccattgggcgctagcactctggtatcacggtacctttgtgcgcctgttttataccccctcccccaactgtaacttagaagtaacacacaccgatcaacagtcagcgtggcacaccagccacgttttgatcaagcacttctgttaccccggactgagtatcaatagactgctcacgcggttgaaggagaaagcgttcgttatccggccaactacttcgaaaaacctagtaacaccgtggaagttgcagagtgtttcgctcagcactaccccagtgtagatcaggtcgatgagtcaccgcattccccacgggcgaccgtggcggtggctgcgttggcggcctgcccatggggaaacccatgggacgctctaatacagacatggtgcgaagagtctattgagctagttggtagtcctccggcccctgaatgcggctaatcctaactgcggagcacacaccctcaagccagagggcagtgtgtcgtaacgggcaactctgcagcggaaccgactactttgggtgtccgtgtttcattttattcctatactggctgcttatggtgacaattgagagatcgttaccatatagctattggattggccatccggtgactaatagagctattatatatccctttgttgggtttataccacttagcttgaaagaggttaaaacattacaattcattgttaagttgaatacagcaaaatggccgtgtccgacgccctgctgccctcattcagcaccttcgcctcaggccccgctggcagagaaaagacactgagacaggctggagcccctaacaaccgctggcgcgaggagctgagtcacatgaaacgcctgccccctgtcctgcctgggcggccatacgacctggccgccgccacggtggccaccgacctggagtcaggcggggccggagccgcctgtggcggctccaacctggcgcccctgccccgcagggagactgaggagttcaacgatctgctggatctggacttcatcctcagtaactctctgacccaccccccagagagtgttgctgctaccgtgagcagcagcgccagcgcgagctctagcagcagccctagcagctccgggcctgccagtgcccccagcacctgcagcttcacctaccccatcagggccggtaacgaccctggtgtggcccccggcggcaccgggggcggactcctgtacggccgggagtccgcccccccgcccaccgcccccttcaacctggcggacatcaacgatgtgagcccctccgggggcttcgtcgccgagctgctgcggccagagctcgaccctgtgtacatccccccacagcagccgcagcccccgggcggcggcctgatggggaagttcgtgctcaaggccagcctgagcgcacccggctctgagtacggaagcccctccgtgatcagtgtgagcaagggaagccccgacggctcacaccccgtggttgtggccccctacaacggcgggccgccacggacctgccccaagatcaagcaggaggcagtgagcagctgcacccatctgggtgcggggccaccactgtccaacggccaccgccccgctgcccatgacttccctctgggcaggcagctgcccagcaggaccacccctacgctgggcctggaggaggtcctgtcctccagggactgccacccggccctgcccctgcccccggggttccacccccaccccggacccaactaccccagcttcctgcctgaccagatgcagccgcaggttccgcccctgcattaccaggagctgatgcccccgggcagctgcatgcccgaggagcctaagcctaagcggggccggcgcagctggccccgcaagcggaccgccacccacacttgcgattacgccgggtgcggcaagacctacacaaagagttcgcacctgaaggcccacctgcgaactcacacgggcgagaagccctaccactgcgactgggacgggtgcggctggaagttcgcccggtccgatgagctgacccggcactatcggaagcacaccgggcacaggcccttccagtgccagaagtgtgaccgggccttcagccggtcagaccatctggcactgcacatgaagcgccacttctgatgataatgaaaaaaacaaaaaacaaaacggctattatgcgttaccggcgagacgctacggacttaaataattgagccttaaagaagaaattctttaagtggatgctctcaaactcagggaaacctaaatctagttatagacaaggcaatcctgagccaagccgaagtagtaattagtaagaccagtggacaatcgacggataacagcatatctag

SEQ ID NO: 55 - DNA, 2850 bp, synthetic construct
  source 1..2850: mol_type = other DNA
gagaccctcgaccgtcgattgtccactggtcaacaatagatgacttacaactaatcggaaggtgcagagactcgacgggagctaccctaacgtcaagacgagggtaaagagagagtccaattctcaaagccaataggcagtagcgaaagctgcaagagaatgaaaatccgttgaccttaaacggtcgtgtgggttcaagtccctccacccccacgccggaaacgcaatagccgaaaaacaaaaaacaaaaaaaacaaaaaaaaaaccaaaaaaacaaaacacattaaaacagcctgtgggttgatcccacccacaggcccattgggcgctagcactctggtatcacggtacctttgtgcgcctgttttataccccctcccccaactgtaacttagaagtaacacacaccgatcaacagtcagcgtggcacaccagccacgttttgatcaagcacttctgttaccccggactgagtatcaatagactgctcacgcggttgaaggagaaagcgttcgttatccggccaactacttcgaaaaacctagtaacaccgtggaagttgcagagtgtttcgctcagcactaccccagtgtagatcaggtcgatgagtcaccgcattccccacgggcgaccgtggcggtggctgcgttggcggcctgcccatggggaaacccatgggacgctctaatacagacatggtgcgaagagtctattgagctagttggtagtcctccggcccctgaatgcggctaatcctaactgcggagcacacaccctcaagccagagggcagtgtgtcgtaacgggcaactctgcagcggaaccgactactttgggtgtccgtgtttcattttattcctatactggctgcttatggtgacaattgagagatcgttaccatatagctattggattggccatccggtgactaatagagctattatatatccctttgttgggtttataccacttagcttgaaagaggttaaaacattacaattcattgttaagttgaatacagcaaaatgggaagcgtgagcaaccagcagttcgccggaggatgtgccaaggccgcagaggaggctcccgaagaggccccagaggatgccgctagagccgcagacgagccccagctgctccacggagccggaatctgcaagtggttcaatgtgaggatggggttcggcttcctgagcatgaccgcacgggccggggtcgccctggacccccccgtggacgtgttcgtgcaccagagcaagttgcacatggagggcttccgctctctgaaggagggtgaggctgtggagttcaccttcaagaagtcggccaaaggcctggagagcatccgggtcaccggacccggcggagtgttctgcatcgggtccgagcgtaggcccaagggcaagtctatgcagaagcgccggtctaagggcgaccggtgctacaactgtggtggcctggaccaccacgccaaggagtgcaaactgcctcctcagcccaagaagtgccacttctgtcagagcatctctcacatggtggccagctgccctctgaaggcgcagcaggggccctcggcccagggcaagcccacctacttccgggaggaggaggaggagattcactcccccactctgctgcccgaggctcagaatgggagcggggccaccaacttctccctgctcaagcaggccggggatgtggaggagaaccccggcccgatgtccgtggaccccgcctgtccacagtcgctgccttgcttcgaggccagcgactgtaaggagagctctcctatgcccgtgatctgcgggcctgaggagaactatcccagcctgcagatgtcgagcgccgagatgcctcacaccgagaccgtgtccccgctgcctagcagcatggacctgctgattcaggactcccctgacagcagtacgagcccaaagggcaagcagcccacctcggccgagaagtcggtggccaagaaggaggacaaggtccctgtgaagaagcagaagacccgtactgtgttcagcagcacacagctgtgtgtgctgaacgaccgcttccagcggcagaagtacctgagcctgcagcagatgcaggagctcagtaacattctgaacctgtcctacaagcaggtaaagacctggttccagaaccagcgtatgaaaagcaagcgctggcagaagaacaactggccgaagaacagcaacggggtgacccagaaggcttcggctcccacctaccctagcctgtacagctcgtatcaccagggctgcctggtgaacccgacgggcaacctgcccatgtggtctaaccagacgtggaacaactccacctggtccaaccagacccagaacatccagtcctggtctaaccatagctggaatacccagacctggtgtacccagtcctggaacaaccaggcctggaacagtccgttctacaactgcggcgaggagtcgctgcagagctgtatgcagttccagcctaacagcccggcctccgacctggaggccgccctcgaggcggctggagagggcctgaacgtcatccagcagaccaccaggtacttctctacccctcagaccatggacctgttcctgaactattccatgaatatgcaacctgaggatgtctgatgataatgaaaaaaacaaaaaacaaaacggctattatgcgttaccggcgagacgctacggacttaaataattgagccttaaagaagaaattctttaagtggatgctctcaaactcagggaaacctaaatctagttatagacaaggcaatcctgagccaagccgaagtagtaattagtaagaccagtggacaatcgacggataacagcatatctag

SEQ ID NO: 56 - DNA, 3339 bp, synthetic construct
  source 1..3339: mol_type = other DNA
gagaccctcgaccgtcgattgtccactggtcaacaatagatgacttacaactaatcggaaggtgcagagactcgacgggagctaccctaacgtcaagacgagggtaaagagagagtccaattctcaaagccaataggcagtagcgaaagctgcaagagaatgaaaatccgttgaccttaaacggtcgtgtgggttcaagtccctccacccccacgccggaaacgcaatagccgaaaaacaaaaaacaaaaaaaacaaaaaaaaaaccaaaaaaacaaaacacattaaaacagcctgtgggttgatcccacccacaggcccattgggcgctagcactctggtatcacggtacctttgtgcgcctgttttataccccctcccccaactgtaacttagaagtaacacacaccgatcaacagtcagcgtggcacaccagccacgttttgatcaagcacttctgttaccccggactgagtatcaatagactgctcacgcggttgaaggagaaagcgttcgttatccggccaactacttcgaaaaacctagtaacaccgtggaagttgcagagtgtttcgctcagcactaccccagtgtagatcaggtcgatgagtcaccgcattccccacgggcgaccgtggcggtggctgcgttggcggcctgcccatggggaaacccatgggacgctctaatacagacatggtgcgaagagtctattgagctagttggtagtcctccggcccctgaatgcggctaatcctaactgcggagcacacaccctcaagccagagggcagtgtgtcgtaacgggcaactctgcagcggaaccgactactttgggtgtccgtgtttcattttattcctatactggctgcttatggtgacaattgagagatcgttaccatatagctattggattggccatccggtgactaatagagctattatatatccctttgttgggtttataccacttagcttgaaagaggttaaaacattacaattcattgttaagttgaatacagcaaaatggctggccacctggcctctgacttcgccttctctcccccacctggcggcggcggtgacggccccggaggacccgagcctggatgggtggaccctagaacctggctgtcattccagggacctcctggcggacccggcatcggacctggcgtcgggcccggcagcgaggtgtggggcatacctccctgccctcccccctacgagttctgcgggggcatggcctactgtggcccccaggtcggggtcggcctggtgccccagggcggcctcgaaaccagccagcccgagggcgaggctggtgtcggagtggagagcaactccgacggggccagcccagagccatgcaccgtgactcccggcgcagtgaagctggaaaaggagaagctggagcagaatcctgaggagtctcaggacatcaaggcgctccagaaggagctggagcagttcgcgaagctgctgaagcagaagcggatcacgctggggtacacccaggccgacgtcggcctgaccctgggcgtcctgttcggcaaggtgttcagccagaccaccatctgccggttcgaggccctgcagcttagcttcaagaacatgtgcaagctgcgcccacttctgcagaagtgggtggaggaggcggataacaacgagaacctgcaggagatctgcaaggccgagacgctggtgcaggccaggaagcgaaagcggacctccatcgagaaccgcgttcgcgggaacctggagaacctgttcctgcagtgtcccaagcctacactgcagcagatctctcacatagcccagcagctgggcctggagaaggatgtggtgcgagtgtggttctgcaatcggaggcagaagggcaagcgctcttcctccgattacgcccagagggaggacttcgaggcggcggggtcccccttcagcggcggccccgtgtccttccctctggcccccgggccacacttcgggactcccggctacggcagcccacacttcaccgcgctgtacagcagcgtgccattccctgagggggaggccttcccccccgtgagcgtgacgacgctgggcagccccatgcacagcaatgggagcggggccaccaacttctccctgctcaagcaggctggggacgtggaggagaaccccggtcccatgtacaacatgatggagacagagctgaagccccccgggcctcagcagaccagcggcggcggcgggggcaactccaccgccgccgctgctgggggcaaccagaagaacagccccgatagggtgaagcgccctatgaacgccttcatggtgtggtcccgcggccagcgccgtaagatggctcaggagaaccctaagatgcacaactccgagatcagcaagcggctgggcgcggagtggaagctgctgtcggagaccgagaagcggccattcatcgacgaggccaagaggcttcgtgccctgcacatgaaggagcatcctgactacaagtaccggccccgccggaagaccaagacactgatgaagaaggacaagtacaccttgcctgggggcctgctggcccccgggggcaactccatggcttccggcgtgggcgtgggagccggtctaggcgctggcgtgaaccagcgcatggactcctacgctcacatgaacggctggagcaacgggtcctacagcatgatgcaggaccagttgggctacccccagcaccctgggctgaacgcccatggggctgcccagatgcagcccatgcatcggtacgacgtgagtgccctgcagtacaactccatgacatctagccagacctacatgaacgggagtcccacctacagcatgagctatagccagcaggggaccccaggcatggccctggggtccatgggctccgtggtgaagtcggaggccagctcctcacctcccgtggtgacaagctcctcccacagccgggccccctgccaggctggggatctgagggacatgatctccatgtacctcccgggcgccgaggtgcccgagcctgctgctcccagcaggctgcatatgagccagcattaccagtccgggcccgtgcccggcactgccatcaatgggacactgccactgtcccatatgtgatgataatgaaaaaaacaaaaaacaaaacggctattatgcgttaccggcgagacgctacggacttaaataattgagccttaaagaagaaattctttaagtggatgctctcaaactcagggaaacctaaatctagttatagacaaggcaatcctgagccaagccgaagtagtaattagtaagaccagtggacaatcgacggataacagcatatctag

SEQ ID NO: 57 - DNA, 4707 bp, synthetic construct
  source 1..4707: mol_type = other DNA
gggagaccctcgaatggaatttgcgccgatgaaggtgtagagactagacggcacccacctaaggcaaacgctatggtgaaggcatagtccagggagtggcgaaagtcacacaaaccggaatattggactcgccggaaacgcaatagccgaaaaacaaaaaacaaaaaaaacaaaaaaaaaaccaaaaaaacaaaacacattaaaacagcctgtgggttgatcccacccacaggcccattgggcgctagcactctggtatcacggtacctttgtgcgcctgttttataccccctcccccaactgtaacttagaagtaacacacaccgatcaacagtcagcgtggcacaccagccacgttttgatcaagcacttctgttaccccggactgagtatcaatagactgctcacgcggttgaaggagaaagcgttcgttatccggccaactacttcgaaaaacctagtaacaccgtggaagttgcagagtgtttcgctcagcactaccccagtgtagatcaggtcgatgagtcaccgcattccccacgggcgaccgtggcggtggctgcgttggcggcctgcccatggggaaacccatgggacgctctaatacagacatggtgcgaagagtctattgagctagttggtagtcctccggcccctgaatgcggctaatcctaactgcggagcacacaccctcaagccagagggcagtgtgtcgtaacgggcaactctgcagcggaaccgactactttgggtgtccgtgtttcattttattcctatactggctgcttatggtgacaattgagagatcgttaccatatagctattggattggccatccggtgactaatagagctattatatatccctttgttgggtttataccacttagcttgaaagaggttaaaacattacaattcattgttaagttgaatacagcaaaatggctggccacctggcctctgccttcgccttctctcccccacctggcggcggcggtgccggccccggaggacccgcccctggatgggtggcccctagaacctggctgtcattccagggacctcctggcggacccggcatcggacctggcgtcgggcccggcagcgccgtgtggggcatacctccctgccctcccccctacgccttctgcgggggcatggcctactgtggcccccaggtcggggtcggcctggtgccccagggcggcctcgccaccagccagcccgccggcgccgctggtgtcggagtggccagcaactccgccggggccagcccagccccatgcaccgtgactcccggcgcagtgaagctggccaaggccaagctggcccagaatcctgccgcctctcaggccatcaaggcgctccagaaggagctggagcagttcgcgaagctgctgaagcagaagcggatcacgctggggtacacccaggccgacgtcggcctgaccctgggcgtcctgttcggcaaggtgttcagccagaccaccatctgccggttcgaggccctgcagcttagcttcaagaacatgtgcaagctgcgcccacttctgcagaagtgggtggaggaggcggataacaacgagaacctgcaggagatctgcaaggccgagacgctggtgcaggccaggaagcgaaagcggacctccatcgagaaccgcgttcgcgggaacctggagaacctgttcctgcagtgtcccaagcctacactgcagcagatctctcacatagcccagcagctgggcctggagaaggatgtggtgcgagtgtggttctgcaatcggaggcagaagggcaagcgctcttcctccgcctacgcccagagggccgccttcgccgcggcggggtcccccttcagcggcggccccgtgtccttccctctggcccccgggccacacttcgggactcccggctacggcagcccacacttcaccgcgctgtacagcagcgtgccattccctgccggggccgccttcccccccgtgagcgtgacgacgctgggcagccccatgcacagcaatggaagcggagccacgaacttctctctgttaaagcaagcaggagatgttgaagaaaaccccgggcctatgtacaacatgatggagacagagctgaagccccccgggcctcagcagaccagcggcggcggcgggggcaactccaccgccgccgctgctgggggcaaccagaagaacagccccgatagggtgaagcgccctatgaacgccttcatggtgtggtcccgcggccagcgccgtaagatggctcaggagaaccctaagatgcacaactccgagatcagcaagcggctgggcgcggagtggaagctgctgtcggagaccgagaagcggccattcatcgacgaggccaagaggcttcgtgccctgcacatgaaggagcatcctgactacaagtaccggccccgccggaagaccaagacactgatgaagaaggacaagtacaccttgcctgggggcctgctggcccccgggggcaactccatggcttccggcgtgggcgtgggagccggtctaggcgctggcgtgaaccagcgcatggactcctacgctcacatgaacggctggagcaacgggtcctacagcatgatgcaggaccagttgggctacccccagcaccctgggctgaacgcccatggggctgcccagatgcagcccatgcatcggtacgacgtgagtgccctgcagtacaactccatgacatctagccagacctacatgaacgggagtcccacctacagcatgagctatagccagcaggggaccccaggcatggccctggggtccatgggctccgtggtgaagtcggaggccagctcctcacctcccgtggtgacaagctcctcccacagccgggccccctgccaggctggggatctgagggacatgatctccatgtacctcccgggcgccgaggtgcccgagcctgctgctcccagcaggctgcatatgagccagcattaccagtccgggcccgtgcccggcactgccatcaatgggacactgccactgtcccatatgggaagcggagagggcaggggaagtcttctaacatgcggggacgtggaggaaaatcccggccccatggccgtgtccgacgccctgctgccctcattcagcaccttcgcctcaggccccgctggcagagaaaagacactgagacaggctggagcccctaacaaccgctggcgcgaggagctgagtcacatgaaacgcctgccccctgtcctgcctgggcggccatacgacctggccgccgccacggtggccaccgacctggagtcaggcggggccggagccgcctgtggcggctccaacctggcgcccctgccccgcagggagactgaggagttcaacgatctgctggatctggacttcatcctcagtaactctctgacccaccccccagagagtgttgctgctaccgtgagcagcagcgccagcgcgagctctagcagcagccctagcagctccgggcctgccagtgcccccagcacctgcagcttcacctaccccatcagggccggtaacgaccctggtgtggcccccggcggcaccgggggcggactcctgtacggccgggagtccgcccccccgcccaccgcccccttcaacctggcggacatcaacgatgtgagcccctccgggggcttcgtcgccgagctgctgcggccagagctcgaccctgtgtacatccccccacagcagccgcagcccccgggcggcggcctgatggggaagttcgtgctcaaggccagcctgagcgcacccggctctgagtacggaagcccctccgtgatcagtgtgagcaagggaagccccgacggctcacaccccgtggttgtggccccctacaacggcgggccgccacggacctgccccaagatcaagcaggaggcagtgagcagctgcacccatctgggtgcggggccaccactgtccaacggccaccgccccgctgcccatgacttccctctgggcaggcagctgcccagcaggaccacccctacgctgggcctggaggaggtcctgtcctccagggactgccacccggccctgcccctgcccccggggttccacccccaccccggacccaactaccccagcttcctgcctgaccagatgcagccgcaggttccgcccctgcattaccaggagctgatgcccccgggcagctgcatgcccgaggagcctaagcctaagcggggccggcgcagctggccccgcaagcggaccgccacccacacttgcgattacgccgggtgcggcaagacctacacaaagagttcgcacctgaaggcccacctgcgaactcacacgggcgagaagccctaccactgcgactgggacgggtgcggctggaagttcgcccggtccgatgagctgacccggcactatcggaagcacaccgggcacaggcccttccagtgccagaagtgtgaccgggccttcagccggtcagaccatctggcactgcacatgaagcgccacttctgatgataaaaaaaacaaaaaacaaaacggctattatgcgttaccggcgatgctcaatgtacctatttctatgggccttgcgccgggaaaccacgcaagggatggtgtcaaattcggcgaaacctaagcgcccgcccgggcgtatggcaacgccgagccaagcttcggcgccaattccatttatcagatttctagag

SEQ ID NO: 58 - DNA, 4707 bp, synthetic construct
  source 1..4707: mol_type = other DNA
gggagaccctcgaatggaatttgcgccgatgaaggtgtagagactagacggcacccacctaaggcaaacgctatggtgaaggcatagtccagggagtggcgaaagtcacacaaaccggaatattggactcgccggaaacgcaatagccgaaaaacaaaaaacaaaaaaaacaaaaaaaaaaccaaaaaaacaaaacacattaaaacagcctgtgggttgatcccacccacaggcccattgggcgctagcactctggtatcacggtacctttgtgcgcctgttttataccccctcccccaactgtaacttagaagtaacacacaccgatcaacagtcagcgtggcacaccagccacgttttgatcaagcacttctgttaccccggactgagtatcaatagactgctcacgcggttgaaggagaaagcgttcgttatccggccaactacttcgaaaaacctagtaacaccgtggaagttgcagagtgtttcgctcagcactaccccagtgtagatcaggtcgatgagtcaccgcattccccacgggcgaccgtggcggtggctgcgttggcggcctgcccatggggaaacccatgggacgctctaatacagacatggtgcgaagagtctattgagctagttggtagtcctccggcccctgaatgcggctaatcctaactgcggagcacacaccctcaagccagagggcagtgtgtcgtaacgggcaactctgcagcggaaccgactactttgggtgtccgtgtttcattttattcctatactggctgcttatggtgacaattgagagatcgttaccatatagctattggattggccatccggtgactaatagagctattatatatccctttgttgggtttataccacttagcttgaaagaggttaaaacattacaattcattgttaagttgaatacagcaaaatggctggccacctggcctctgacttcgccttctctcccccacctggcggcggcggtgacggccccggaggacccgagcctggatgggtggaccctagaacctggctgtcattccagggacctcctggcggacccggcatcggacctggcgtcgggcccggcagcgaggtgtggggcatacctccctgccctcccccctacgagttctgcgggggcatggcctactgtggcccccaggtcggggtcggcctggtgccccagggcggcctcgaaaccagccagcccgagggcgaggctggtgtcggagtggagagcaactccgacggggccagcccagagccatgcaccgtgactcccggcgcagtgaagctggaaaaggagaagctggagcagaatcctgaggagtctcaggacatcaaggcgctccagaaggagctggagcagttcgcgaagctgctgaagcagaagcggatcacgctggggtacacccaggccgacgtcggcctgaccctgggcgtcctgttcggcaaggtgttcagccagaccaccatctgccggttcgaggccctgcagcttagcttcaagaacatgtgcaagctgcgcccacttctgcagaagtgggtggaggaggcggataacaacgagaacctgcaggagatctgcaaggccgagacgctggtgcaggccaggaagcgaaagcggacctccatcgagaaccgcgttcgcgggaacctggagaacctgttcctgcagtgtcccaagcctacactgcagcagatctctcacatagcccagcagctgggcctggagaaggatgtggtgcgagtgtggttctgcaatcggaggcagaagggcaagcgctcttcctccgattacgcccagagggaggacttcgaggcggcggggtcccccttcagcggcggccccgtgtccttccctctggcccccgggccacacttcgggactcccggctacggcagcccacacttcaccgcgctgtacagcagcgtgccattccctgagggggaggccttcccccccgtgagcgtgacgacgctgggcagccccatgcacagcaatggaagcggagccacgaacttctctctgttaaagcaagcaggagatgttgaagaaaaccccgggcctatgtacaacatgatggagacagagctgaagccccccgggcctcagcagaccagcggcggcggcgggggcaactccaccgccgccgctgctgggggcaaccagaagaacagccccgatagggtgaagcgccctatgaacgccttcatggtgtggtcccgcggccagcgccgtaagatggctcaggagaaccctaagatgcacaactccgagatcagcaagcggctgggcgcggagtggaagctgctgtcggagaccgagaagcggccattcatcgacgaggccaagaggcttcgtgccctgcacatgaaggagcatcctgactacaagtaccggccccgccggaagaccaagacactgatgaagaaggacaagtacaccttgcctgggggcctgctggcccccgggggcaactccatggcttccggcgtgggcgtgggagccggtctaggcgctggcgtgaaccagcgcatggactcctacgctcacatgaacggctggagcaacgggtcctacagcatgatgcaggaccagttgggctacccccagcaccctgggctgaacgcccatggggctgcccagatgcagcccatgcatcggtacgacgtgagtgccctgcagtacaactccatgacatctagccagacctacatgaacgggagtcccacctacagcatgagctatagccagcaggggaccccaggcatggccctggggtccatgggctccgtggtgaagtcggaggccagctcctcacctcccgtggtgacaagctcctcccacagccgggccccctgccaggctggggatctgagggacatgatctccatgtacctcccgggcgccgaggtgcccgagcctgctgctcccagcaggctgcatatgagccagcattaccagtccgggcccgtgcccggcactgccatcaatgggacactgccactgtcccatatgggaagcggagagggcaggggaagtcttctaacatgcggggacgtggaggaaaatcccggccccatggccgtgtccgacgccctgctgccctcattcagcaccttcgcctcaggccccgctggcagagaaaagacactgagacaggctggagcccctaacaaccgctggcgcgaggagctgagtcacatgaaacgcctgccccctgtcctgcctgggcggccatacgacctggccgccgccacggtggccaccgacctggagtcaggcggggccggagccgcctgtggcggctccaacctggcgcccctgccccgcagggagactgaggagttcaacgatctgctggatctggacttcatcctcagtaactctctgacccaccccccagagagtgttgctgctaccgtgagcagcagcgccagcgcgagctctagcagcagccctagcagctccgggcctgccagtgcccccagcacctgcagcttcacctaccccatcagggccggtaacgaccctggtgtggcccccggcggcaccgggggcggactcctgtacggccgggagtccgcccccccgcccaccgcccccttcaacctggcggacatcaacgatgtgagcccctccgggggcttcgtcgccgagctgctgcggccagagctcgaccctgtgtacatccccccacagcagccgcagcccccgggcggcggcctgatggggaagttcgtgctcaaggccagcctgagcgcacccggctctgagtacggaagcccctccgtgatcagtgtgagcaagggaagccccgacggctcacaccccgtggttgtggccccctacaacggcgggccgccacggacctgccccaagatcaagcaggaggcagtgagcagctgcacccatctgggtgcggggccaccactgtccaacggccaccgccccgctgcccatgacttccctctgggcaggcagctgcccagcaggaccacccctacgctgggcctggaggaggtcctgtcctccagggactgccacccggccctgcccctgcccccggggttccacccccaccccggacccaactaccccagcttcctgcctgaccagatgcagccgcaggttccgcccctgcattaccaggagctgatgcccccgggcagctgcatgcccgaggagcctaagcctaagcggggccggcgcagctggccccgcaagcggaccgccacccacacttgcgattacgccgggtgcggcaagacctacacaaagagttcgcacctgaaggcccacctgcgaactcacacgggcgagaagccctaccactgcgactgggacgggtgcggctggaagttcgcccggtccgatgagctgacccggcactatcggaagcacaccgggcacaggcccttccagtgccagaagtgtgaccgggccttcagccggtcagaccatctggcactgcacatgaagcgccacttctgatgataaaaaaaacaaaaaacaaaacggctattatgcgttaccggcgatgctcaatgtacctatttctatgggccttgcgccgggaaaccacgcaagggatggtgtcaaattcggcgaaacctaagcgcccgcccgggcgtatggcaacgccgagccaagcttcggcgccaattccatttatcagatttctagag

SEQ ID NO: 59 - DNA, 5073 bp, synthetic construct
  source 1..5073: mol_type = other DNA
gggagaccctcgaatggaatttgcgccgatgaaggtgtagagactagacggcacccacctaaggcaaacgctatggtgaaggcatagtccagggagtggcgaaagtcacacaaaccggaatattggactcgccggaaacgcaatagccgaaaaacaaaaaacaaaaaaaacaaaaaaaaaaccaaaaaaacaaaacacattaaaacagcctgtgggttgatcccacccacaggcccattgggcgctagcactctggtatcacggtacctttgtgcgcctgttttataccccctcccccaactgtaacttagaagtaacacacaccgatcaacagtcagcgtggcacaccagccacgttttgatcaagcacttctgttaccccggactgagtatcaatagactgctcacgcggttgaaggagaaagcgttcgttatccggccaactacttcgaaaaacctagtaacaccgtggaagttgcagagtgtttcgctcagcactaccccagtgtagatcaggtcgatgagtcaccgcattccccacgggcgaccgtggcggtggctgcgttggcggcctgcccatggggaaacccatgggacgctctaatacagacatggtgcgaagagtctattgagctagttggtagtcctccggcccctgaatgcggctaatcctaactgcggagcacacaccctcaagccagagggcagtgtgtcgtaacgggcaactctgcagcggaaccgactactttgggtgtccgtgtttcattttattcctatactggctgcttatggtgacaattgagagatcgttaccatatagctattggattggccatccggtgactaatagagctattatatatccctttgttgggtttataccacttagcttgaaagaggttaaaacattacaattcattgttaagttgaatacagcaaaatggctggccacctggcctctgccttcgccttctctcccccacctggcggcggcggtgccggccccggaggacccgcccctggatgggtggcccctagaacctggctgtcattccagggacctcctggcggacccggcatcggacctggcgtcgggcccggcagcgccgtgtggggcatacctccctgccctcccccctacgccttctgcgggggcatggcctactgtggcccccaggtcggggtcggcctggtgccccagggcggcctcgccaccagccagcccgccggcgccgctggtgtcggagtggccagcaactccgccggggccagcccagccccatgcaccgtgactcccggcgcagtgaagctggccaaggccaagctggcccagaatcctgccgcctctcaggccatcaaggcgctccagaaggagctggagcagttcgcgaagctgctgaagcagaagcggatcacgctggggtacacccaggccgacgtcggcctgaccctgggcgtcctgttcggcaaggtgttcagccagaccaccatctgccggttcgaggccctgcagcttagcttcaagaacatgtgcaagctgcgcccacttctgcagaagtgggtggaggaggcggataacaacgagaacctgcaggagatctgcaaggccgagacgctggtgcaggccaggaagcgaaagcggacctccatcgagaaccgcgttcgcgggaacctggagaacctgttcctgcagtgtcccaagcctacactgcagcagatctctcacatagcccagcagctgggcctggagaaggatgtggtgcgagtgtggttctgcaatcggaggcagaagggcaagcgctcttcctccgcctacgcccagagggccgccttcgccgcggcggggtcccccttcagcggcggccccgtgtccttccctctggcccccgggccacacttcgggactcccggctacggcagcccacacttcaccgcgctgtacagcagcgtgccattccctgccggggccgccttcccccccgtgagcgtgacgacgctgggcagccccatgcacagcaatggaagcggagccacgaacttctctctgttaaagcaagcaggagatgttgaagaaaaccccgggcctatggccgtgtccgacgccctgctgccctcattcagcaccttcgcctcaggccccgctggcagagaaaagacactgagacaggctggagcccctaacaaccgctggcgcgaggagctgagtcacatgaaacgcctgccccctgtcctgcctgggcggccatacgacctggccgccgccacggtggccaccgacctggagtcaggcggggccggagccgcctgtggcggctccaacctggcgcccctgccccgcagggagactgaggagttcaacgatctgctggatctggacttcatcctcagtaactctctgacccaccccccagagagtgttgctgctaccgtgagcagcagcgccagcgcgagctctagcagcagccctagcagctccgggcctgccagtgcccccagcacctgcagcttcacctaccccatcagggccggtaacgaccctggtgtggcccccggcggcaccgggggcggactcctgtacggccgggagtccgcccccccgcccaccgcccccttcaacctggcggacatcaacgatgtgagcccctccgggggcttcgtcgccgagctgctgcggccagagctcgaccctgtgtacatccccccacagcagccgcagcccccgggcggcggcctgatggggaagttcgtgctcaaggccagcctgagcgcacccggctctgagtacggaagcccctccgtgatcagtgtgagcaagggaagccccgacggctcacaccccgtggttgtggccccctacaacggcgggccgccacggacctgccccaagatcaagcaggaggcagtgagcagctgcacccatctgggtgcggggccaccactgtccaacggccaccgccccgctgcccatgacttccctctgggcaggcagctgcccagcaggaccacccctacgctgggcctggaggaggtcctgtcctccagggactgccacccggccctgcccctgcccccggggttccacccccaccccggacccaactaccccagcttcctgcctgaccagatgcagccgcaggttccgcccctgcattaccaggagctgatgcccccgggcagctgcatgcccgaggagcctaagcctaagcggggccggcgcagctggccccgcaagcggaccgccacccacacttgcgattacgccgggtgcggcaagacctacacaaagagttcgcacctgaaggcccacctgcgaactcacacgggcgagaagccctaccactgcgactgggacgggtgcggctggaagttcgcccggtccgatgagctgacccggcactatcggaagcacaccgggcacaggcccttccagtgccagaagtgtgaccgggccttcagccggtcagaccatctggcactgcacatgaagcgccacttcggaagcggagagggcaggggaagtcttctaacatgcggggacgtggaggaaaatcccggccccatgcccctgaatgtgtccttcaccaaccgcaactatgatctggactatgactctgtgcagccttacttctactgcgatgaggaggagaacttctaccagcagcagcagcagagcgaactgcagccacccgccccatccgaggatatctggaggaggttcgagctgctgccgacccctcctctcagcccctccaggaggagcgggctgtgcagtcccagctacgtggctgtgacccccttctccctgcgcggcgacaacgacggcgggggggggagcttcagcaccgctgaccagctggagatggtcaccgagctgctgggtggcgacatggtcaaccagagcttcatctgcgaccctgatgatgagacattcatcaggaacatcatcatccaggactgcatgtggtccggcttctcggccgctgccaggctggtcagcgagaggctggccagctaccaggccgcccggagggattccgggtcgcctaaccccgccaggggccacagcgtctgctccacgagcagcctgtacctgcaggatctgagcgccgccgccagcgagtgcatagatccttcagtggtgttcccatacccactgaacgacagcagctctcccaggagctgcgcctcgcaggacagcagcgccttcagcccctcgtccgactcgctgctgtccagcaccgagtcgagcccccagggctctcctgagcccctggtgctgcacgaggagacccctcctaccacctcctcggactccgaggaggagcaggaggatgaggaagagatcgacgtggtcagcgtggagaggcgccaggctcctggcaggcgcagcgagtctggcagcccctccgccgggggccacagcaggcccccgcacagcccgctggtgctgaggcggtgtcacgtgagcacccaccagcataactatgctgcgcctccttccaccaggagggactaccccgctgccaggcgggtgaggctggatagcgtccgggtgctgaggcagatcagcaataaccgtaggtgcacctcccccaggagcagtgacacagaggagaacgtgaggaggcggactcacaacgttctggagcgccagcgccggaacgagctgaggcggtccttcttcgctctgagggaccagatcccagagctggagaacaatgagagggcaccgagggtggtcatcctgaggagggccaccgcgtatatcctgagcgtgcaggctgaggagcagaggctgatcagcgaggaggacttgctgaggaggcggcgcgagcagctgaggcacaggctggagcagctgcgaaacagctgcgcctgatgataaaaaaaacaaaaaacaaaacggctattatgcgttaccggcgatgctcaatgtacctatttctatgggccttgcgccgggaaaccacgcaagggatggtgtcaaattcggcgaaacctaagcgcccgcccgggcgtatggcaacgccgagccaagcttcggcgccaattccatttatcagatttctagag

SEQ ID NO: 60 - DNA, 5073 bp, synthetic construct
  source 1..5073: mol_type = other DNA
gggagaccctcgaatggaatttgcgccgatgaaggtgtagagactagacggcacccacctaaggcaaacgctatggtgaaggcatagtccagggagtggcgaaagtcacacaaaccggaatattggactcgccggaaacgcaatagccgaaaaacaaaaaacaaaaaaaacaaaaaaaaaaccaaaaaaacaaaacacattaaaacagcctgtgggttgatcccacccacaggcccattgggcgctagcactctggtatcacggtacctttgtgcgcctgttttataccccctcccccaactgtaacttagaagtaacacacaccgatcaacagtcagcgtggcacaccagccacgttttgatcaagcacttctgttaccccggactgagtatcaatagactgctcacgcggttgaaggagaaagcgttcgttatccggccaactacttcgaaaaacctagtaacaccgtggaagttgcagagtgtttcgctcagcactaccccagtgtagatcaggtcgatgagtcaccgcattccccacgggcgaccgtggcggtggctgcgttggcggcctgcccatggggaaacccatgggacgctctaatacagacatggtgcgaagagtctattgagctagttggtagtcctccggcccctgaatgcggctaatcctaactgcggagcacacaccctcaagccagagggcagtgtgtcgtaacgggcaactctgcagcggaaccgactactttgggtgtccgtgtttcattttattcctatactggctgcttatggtgacaattgagagatcgttaccatatagctattggattggccatccggtgactaatagagctattatatatccctttgttgggtttataccacttagcttgaaagaggttaaaacattacaattcattgttaagttgaatacagcaaaatggctggccacctggcctctgacttcgccttctctcccccacctggcggcggcggtgacggccccggaggacccgagcctggatgggtggaccctagaacctggctgtcattccagggacctcctggcggacccggcatcggacctggcgtcgggcccggcagcgaggtgtggggcatacctccctgccctcccccctacgagttctgcgggggcatggcctactgtggcccccaggtcggggtcggcctggtgccccagggcggcctcgaaaccagccagcccgagggcgaggctggtgtcggagtggagagcaactccgacggggccagcccagagccatgcaccgtgactcccggcgcagtgaagctggaaaaggagaagctggagcagaatcctgaggagtctcaggacatcaaggcgctccagaaggagctggagcagttcgcgaagctgctgaagcagaagcggatcacgctggggtacacccaggccgacgtcggcctgaccctgggcgtcctgttcggcaaggtgttcagccagaccaccatctgccggttcgaggccctgcagcttagcttcaagaacatgtgcaagctgcgcccacttctgcagaagtgggtggaggaggcggataacaacgagaacctgcaggagatctgcaaggccgagacgctggtgcaggccaggaagcgaaagcggacctccatcgagaaccgcgttcgcgggaacctggagaacctgttcctgcagtgtcccaagcctacactgcagcagatctctcacatagcccagcagctgggcctggagaaggatgtggtgcgagtgtggttctgcaatcggaggcagaagggcaagcgctcttcctccgattacgcccagagggaggacttcgaggcggcggggtcccccttcagcggcggccccgtgtccttccctctggcccccgggccacacttcgggactcccggctacggcagcccacacttcaccgcgctgtacagcagcgtgccattccctgagggggaggccttcccccccgtgagcgtgacgacgctgggcagccccatgcacagcaatggaagcggagccacgaacttctctctgttaaagcaagcaggagatgttgaagaaaaccccgggcctatggccgtgtccgacgccctgctgccctcattcagcaccttcgcctcaggccccgctggcagagaaaagacactgagacaggctggagcccctaacaaccgctggcgcgaggagctgagtcacatgaaacgcctgccccctgtcctgcctgggcggccatacgacctggccgccgccacggtggccaccgacctggagtcaggcggggccggagccgcctgtggcggctccaacctggcgcccctgccccgcagggagactgaggagttcaacgatctgctggatctggacttcatcctcagtaactctctgacccaccccccagagagtgttgctgctaccgtgagcagcagcgccagcgcgagctctagcagcagccctagcagctccgggcctgccagtgcccccagcacctgcagcttcacctaccccatcagggccggtaacgaccctggtgtggcccccggcggcaccgggggcggactcctgtacggccgggagtccgcccccccgcccaccgcccccttcaacctggcggacatcaacgatgtgagcccctccgggggcttcgtcgccgagctgctgcggccagagctcgaccctgtgtacatccccccacagcagccgcagcccccgggcggcggcctgatggggaagttcgtgctcaaggccagcctgagcgcacccggctctgagtacggaagcccctccgtgatcagtgtgagcaagggaagccccgacggctcacaccccgtggttgtggccccctacaacggcgggccgccacggacctgccccaagatcaagcaggaggcagtgagcagctgcacccatctgggtgcggggccaccactgtccaacggccaccgccccgctgcccatgacttccctctgggcaggcagctgcccagcaggaccacccctacgctgggcctggaggaggtcctgtcctccagggactgccacccggccctgcccctgcccccggggttccacccccaccccggacccaactaccccagcttcctgcctgaccagatgcagccgcaggttccgcccctgcattaccaggagctgatgcccccgggcagctgcatgcccgaggagcctaagcctaagcggggccggcgcagctggccccgcaagcggaccgccacccacacttgcgattacgccgggtgcggcaagacctacacaaagagttcgcacctgaaggcccacctgcgaactcacacgggcgagaagccctaccactgcgactgggacgggtgcggctggaagttcgcccggtccgatgagctgacccggcactatcggaagcacaccgggcacaggcccttccagtgccagaagtgtgaccgggccttcagccggtcagaccatctggcactgcacatgaagcgccacttcggaagcggagagggcaggggaagtcttctaacatgcggggacgtggaggaaaatcccggccccatgcccctgaatgtgtccttcaccaaccgcaactatgatctggactatgactctgtgcagccttacttctactgcgatgaggaggagaacttctaccagcagcagcagcagagcgaactgcagccacccgccccatccgaggatatctggaagaagttcgagctgctgccgacccctcctctcagcccctccaggaggagcgggctgtgcagtcccagctacgtggctgtgacccccttctccctgcgcggcgacaacgacggcgggggggggagcttcagcaccgctgaccagctggagatggtcaccgagctgctgggtggcgacatggtcaaccagagcttcatctgcgaccctgatgatgagacattcatcaagaacatcatcatccaggactgcatgtggtccggcttctcggccgctgccaagctggtcagcgagaagctggccagctaccaggccgcccggaaggattccgggtcgcctaaccccgccaggggccacagcgtctgctccacgagcagcctgtacctgcaggatctgagcgccgccgccagcgagtgcatagatccttcagtggtgttcccatacccactgaacgacagcagctctcccaagagctgcgcctcgcaggacagcagcgccttcagcccctcgtccgactcgctgctgtccagcaccgagtcgagcccccagggctctcctgagcccctggtgctgcacgaggagacccctcctaccacctcctcggactccgaggaggagcaggaggatgaggaagagatcgacgtggtcagcgtggagaagcgccaggctcctggcaagcgcagcgagtctggcagcccctccgccgggggccacagcaagcccccgcacagcccgctggtgctgaagcggtgtcacgtgagcacccaccagcataactatgctgcgcctccttccaccaggaaggactaccccgctgccaagcgggtgaagctggatagcgtccgggtgctgaggcagatcagcaataaccgtaagtgcacctcccccaggagcagtgacacagaggagaacgtgaagaggcggactcacaacgttctggagcgccagcgccggaacgagctgaagcggtccttcttcgctctgagggaccagatcccagagctggagaacaatgagaaggcaccgaaggtggtcatcctgaagaaggccaccgcgtatatcctgagcgtgcaggctgaggagcagaagctgatcagcgaggaggacttgctgaggaagcggcgcgagcagctgaaacacaagctggagcagctgcgaaacagctgcgcctgatgataaaaaaaacaaaaaacaaaacggctattatgcgttaccggcgatgctcaatgtacctatttctatgggccttgcgccgggaaaccacgcaagggatggtgtcaaattcggcgaaacctaagcgcccgcccgggcgtatggcaacgccgagccaagcttcggcgccaattccatttatcagatttctagag

SEQ ID NO: 61 - DNA, 6093 bp, synthetic construct
  source 1..6093: mol_type = other DNA
gggagaccctcgaatggaatttgcgccgatgaaggtgtagagactagacggcacccacctaaggcaaacgctatggtgaaggcatagtccagggagtggcgaaagtcacacaaaccggaatattggactcgccggaaacgcaatagccgaaaaacaaaaaacaaaaaaaacaaaaaaaaaaccaaaaaaacaaaacacattaaaacagcctgtgggttgatcccacccacaggcccattgggcgctagcactctggtatcacggtacctttgtgcgcctgttttataccccctcccccaactgtaacttagaagtaacacacaccgatcaacagtcagcgtggcacaccagccacgttttgatcaagcacttctgttaccccggactgagtatcaatagactgctcacgcggttgaaggagaaagcgttcgttatccggccaactacttcgaaaaacctagtaacaccgtggaagttgcagagtgtttcgctcagcactaccccagtgtagatcaggtcgatgagtcaccgcattccccacgggcgaccgtggcggtggctgcgttggcggcctgcccatggggaaacccatgggacgctctaatacagacatggtgcgaagagtctattgagctagttggtagtcctccggcccctgaatgcggctaatcctaactgcggagcacacaccctcaagccagagggcagtgtgtcgtaacgggcaactctgcagcggaaccgactactttgggtgtccgtgtttcattttattcctatactggctgcttatggtgacaattgagagatcgttaccatatagctattggattggccatccggtgactaatagagctattatatatccctttgttgggtttataccacttagcttgaaagaggttaaaacattacaattcattgttaagttgaatacagcaaaatggctggccacctggcctctgccttcgccttctctcccccacctggcggcggcggtgccggccccggaggacccgcccctggatgggtggcccctagaacctggctgtcattccagggacctcctggcggacccggcatcggacctggcgtcgggcccggcagcgccgtgtggggcatacctccctgccctcccccctacgccttctgcgggggcatggcctactgtggcccccaggtcggggtcggcctggtgccccagggcggcctcgccaccagccagcccgccggcgccgctggtgtcggagtggccagcaactccgccggggccagcccagccccatgcaccgtgactcccggcgcagtgaagctggccaaggccaagctggcccagaatcctgccgcctctcaggccatcaaggcgctccagaaggagctggagcagttcgcgaagctgctgaagcagaagcggatcacgctggggtacacccaggccgacgtcggcctgaccctgggcgtcctgttcggcaaggtgttcagccagaccaccatctgccggttcgaggccctgcagcttagcttcaagaacatgtgcaagctgcgcccacttctgcagaagtgggtggaggaggcggataacaacgagaacctgcaggagatctgcaaggccgagacgctggtgcaggccaggaagcgaaagcggacctccatcgagaaccgcgttcgcgggaacctggagaacctgttcctgcagtgtcccaagcctacactgcagcagatctctcacatagcccagcagctgggcctggagaaggatgtggtgcgagtgtggttctgcaatcggaggcagaagggcaagcgctcttcctccgcctacgcccagagggccgccttcgccgcggcggggtcccccttcagcggcggccccgtgtccttccctctggcccccgggccacacttcgggactcccggctacggcagcccacacttcaccgcgctgtacagcagcgtgccattccctgccggggccgccttcccccccgtgagcgtgacgacgctgggcagccccatgcacagcaatggaagcggagccacgaacttctctctgttaaagcaagcaggagatgttgaagaaaaccccgggcctatggccgtgtccgacgccctgctgccctcattcagcaccttcgcctcaggccccgctggcagagaaaagacactgagacaggctggagcccctaacaaccgctggcgcgaggagctgagtcacatgaaacgcctgccccctgtcctgcctgggcggccatacgacctggccgccgccacggtggccaccgacctggagtcaggcggggccggagccgcctgtggcggctccaacctggcgcccctgccccgcagggagactgaggagttcaacgatctgctggatctggacttcatcctcagtaactctctgacccaccccccagagagtgttgctgctaccgtgagcagcagcgccagcgcgagctctagcagcagccctagcagctccgggcctgccagtgcccccagcacctgcagcttcacctaccccatcagggccggtaacgaccctggtgtggcccccggcggcaccgggggcggactcctgtacggccgggagtccgcccccccgcccaccgcccccttcaacctggcggacatcaacgatgtgagcccctccgggggcttcgtcgccgagctgctgcggccagagctcgaccctgtgtacatccccccacagcagccgcagcccccgggcggcggcctgatggggaagttcgtgctcaaggccagcctgagcgcacccggctctgagtacggaagcccctccgtgatcagtgtgagcaagggaagccccgacggctcacaccccgtggttgtggccccctacaacggcgggccgccacggacctgccccaagatcaagcaggaggcagtgagcagctgcacccatctgggtgcggggccaccactgtccaacggccaccgccccgctgcccatgacttccctctgggcaggcagctgcccagcaggaccacccctacgctgggcctggaggaggtcctgtcctccagggactgccacccggccctgcccctgcccccggggttccacccccaccccggacccaactaccccagcttcctgcctgaccagatgcagccgcaggttccgcccctgcattaccaggagctgatgcccccgggcagctgcatgcccgaggagcctaagcctaagcggggccggcgcagctggccccgcaagcggaccgccacccacacttgcgattacgccgggtgcggcaagacctacacaaagagttcgcacctgaaggcccacctgcgaactcacacgggcgagaagccctaccactgcgactgggacgggtgcggctggaagttcgcccggtccgatgagctgacccggcactatcggaagcacaccgggcacaggcccttccagtgccagaagtgtgaccgggccttcagccggtcagaccatctggcactgcacatgaagcgccacttcggaagcggagagggcaggggaagtcttctaacatgcggggacgtggaggaaaatcccggccccatgcccctgaatgtgtccttcaccaaccgcaactatgatctggactatgactctgtgcagccttacttctactgcgatgaggaggagaacttctaccagcagcagcagcagagcgaactgcagccacccgccccatccgaggatatctggaggaggttcgagctgctgccgacccctcctctcagcccctccaggaggagcgggctgtgcagtcccagctacgtggctgtgacccccttctccctgcgcggcgacaacgacggcgggggggggagcttcagcaccgctgaccagctggagatggtcaccgagctgctgggtggcgacatggtcaaccagagcttcatctgcgaccctgatgatgagacattcatcaggaacatcatcatccaggactgcatgtggtccggcttctcggccgctgccaggctggtcagcgagaggctggccagctaccaggccgcccggagggattccgggtcgcctaaccccgccaggggccacagcgtctgctccacgagcagcctgtacctgcaggatctgagcgccgccgccagcgagtgcatagatccttcagtggtgttcccatacccactgaacgacagcagctctcccaggagctgcgcctcgcaggacagcagcgccttcagcccctcgtccgactcgctgctgtccagcaccgagtcgagcccccagggctctcctgagcccctggtgctgcacgaggagacccctcctaccacctcctcggactccgaggaggagcaggaggatgaggaagagatcgacgtggtcagcgtggagaggcgccaggctcctggcaggcgcagcgagtctggcagcccctccgccgggggccacagcaggcccccgcacagcccgctggtgctgaggcggtgtcacgtgagcacccaccagcataactatgctgcgcctccttccaccaggagggactaccccgctgccaggcgggtgaggctggatagcgtccgggtgctgaggcagatcagcaataaccgtaggtgcacctcccccaggagcagtgacacagaggagaacgtgaggaggcggactcacaacgttctggagcgccagcgccggaacgagctgaggcggtccttcttcgctctgagggaccagatcccagagctggagaacaatgagagggcaccgagggtggtcatcctgaggagggccaccgcgtatatcctgagcgtgcaggctgaggagcagaggctgatcagcgaggaggacttgctgaggaggcggcgcgagcagctgaggcacaggctggagcagctgcgaaacagctgcgccggaagcggacagtgtactaattatgctctcttgaaattggctggagatgttgagagcaacccaggtcccatgtacaacatgatggagacagagctgaagccccccgggcctcagcagaccagcggcggcggcgggggcaactccaccgccgccgctgctgggggcaaccagaagaacagccccgatagggtgaagcgccctatgaacgccttcatggtgtggtcccgcggccagcgccgtaagatggctcaggagaaccctaagatgcacaactccgagatcagcaagcggctgggcgcggagtggaagctgctgtcggagaccgagaagcggccattcatcgacgaggccaagaggcttcgtgccctgcacatgaaggagcatcctgactacaagtaccggccccgccggaagaccaagacactgatgaagaaggacaagtacaccttgcctgggggcctgctggcccccgggggcaactccatggcttccggcgtgggcgtgggagccggtctaggcgctggcgtgaaccagcgcatggactcctacgctcacatgaacggctggagcaacgggtcctacagcatgatgcaggaccagttgggctacccccagcaccctgggctgaacgcccatggggctgcccagatgcagcccatgcatcggtacgacgtgagtgccctgcagtacaactccatgacatctagccagacctacatgaacgggagtcccacctacagcatgagctatagccagcaggggaccccaggcatggccctggggtccatgggctccgtggtgaagtcggaggccagctcctcacctcccgtggtgacaagctcctcccacagccgggccccctgccaggctggggatctgagggacatgatctccatgtacctcccgggcgccgaggtgcccgagcctgctgctcccagcaggctgcatatgagccagcattaccagtccgggcccgtgcccggcactgccatcaatgggacactgccactgtcccatatgtgatgataaaaaaaacaaaaaacaaaacggctattatgcgttaccggcgatgctcaatgtacctatttctatgggccttgcgccgggaaaccacgcaagggatggtgtcaaattcggcgaaacctaagcgcccgcccgggcgtatggcaacgccgagccaagcttcggcgccaattccatttatcagatttctagag

SEQ ID NO: 62 - DNA, 6093 bp, synthetic construct
  source 1..6093: mol_type = other DNA
gggagaccctcgaatggaatttgcgccgatgaaggtgtagagactagacggcacccacctaaggcaaacgctatggtgaaggcatagtccagggagtggcgaaagtcacacaaaccggaatattggactcgccggaaacgcaatagccgaaaaacaaaaaacaaaaaaaacaaaaaaaaaaccaaaaaaacaaaacacattaaaacagcctgtgggttgatcccacccacaggcccattgggcgctagcactctggtatcacggtacctttgtgcgcctgttttataccccctcccccaactgtaacttagaagtaacacacaccgatcaacagtcagcgtggcacaccagccacgttttgatcaagcacttctgttaccccggactgagtatcaatagactgctcacgcggttgaaggagaaagcgttcgttatccggccaactacttcgaaaaacctagtaacaccgtggaagttgcagagtgtttcgctcagcactaccccagtgtagatcaggtcgatgagtcaccgcattccccacgggcgaccgtggcggtggctgcgttggcggcctgcccatggggaaacccatgggacgctctaatacagacatggtgcgaagagtctattgagctagttggtagtcctccggcccctgaatgcggctaatcctaactgcggagcacacaccctcaagccagagggcagtgtgtcgtaacgggcaactctgcagcggaaccgactactttgggtgtccgtgtttcattttattcctatactggctgcttatggtgacaattgagagatcgttaccatatagctattggattggccatccggtgactaatagagctattatatatccctttgttgggtttataccacttagcttgaaagaggttaaaacattacaattcattgttaagttgaatacagcaaaatggctggccacctggcctctgacttcgccttctctcccccacctggcggcggcggtgacggccccggaggacccgagcctggatgggtggaccctagaacctggctgtcattccagggacctcctggcggacccggcatcggacctggcgtcgggcccggcagcgaggtgtggggcatacctccctgccctcccccctacgagttctgcgggggcatggcctactgtggcccccaggtcggggtcggcctggtgccccagggcggcctcgaaaccagccagcccgagggcgaggctggtgtcggagtggagagcaactccgacggggccagcccagagccatgcaccgtgactcccggcgcagtgaagctggaaaaggagaagctggagcagaatcctgaggagtctcaggacatcaaggcgctccagaaggagctggagcagttcgcgaagctgctgaagcagaagcggatcacgctggggtacacccaggccgacgtcggcctgaccctgggcgtcctgttcggcaaggtgttcagccagaccaccatctgccggttcgaggccctgcagcttagcttcaagaacatgtgcaagctgcgcccacttctgcagaagtgggtggaggaggcggataacaacgagaacctgcaggagatctgcaaggccgagacgctggtgcaggccaggaagcgaaagcggacctccatcgagaaccgcgttcgcgggaacctggagaacctgttcctgcagtgtcccaagcctacactgcagcagatctctcacatagcccagcagctgggcctggagaaggatgtggtgcgagtgtggttctgcaatcggaggcagaagggcaagcgctcttcctccgattacgcccagagggaggacttcgaggcggcggggtcccccttcagcggcggccccgtgtccttccctctggcccccgggccacacttcgggactcccggctacggcagcccacacttcaccgcgctgtacagcagcgtgccattccctgagggggaggccttcccccccgtgagcgtgacgacgctgggcagccccatgcacagcaatggaagcggagccacgaacttctctctgttaaagcaagcaggagatgttgaagaaaaccccgggcctatggccgtgtccgacgccctgctgccctcattcagcaccttcgcctcaggccccgctggcagagaaaagacactgagacaggctggagcccctaacaaccgctggcgcgaggagctgagtcacatgaaacgcctgccccctgtcctgcctgggcggccatacgacctggccgccgccacggtggccaccgacctggagtcaggcggggccggagccgcctgtggcggctccaacctggcgcccctgccccgcagggagactgaggagttcaacgatctgctggatctggacttcatcctcagtaactctctgacccaccccccagagagtgttgctgctaccgtgagcagcagcgccagcgcgagctctagcagcagccctagcagctccgggcctgccagtgcccccagcacctgcagcttcacctaccccatcagggccggtaacgaccctggtgtggcccccggcggcaccgggggcggactcctgtacggccgggagtccgcccccccgcccaccgcccccttcaacctggcggacatcaacgatgtgagcccctccgggggcttcgtcgccgagctgctgcggccagagctcgaccctgtgtacatccccccacagcagccgcagcccccgggcggcggcctgatggggaagttcgtgctcaaggccagcctgagcgcacccggctctgagtacggaagcccctccgtgatcagtgtgagcaagggaagccccgacggctcacaccccgtggttgtggccccctacaacggcgggccgccacggacctgccccaagatcaagcaggaggcagtgagcagctgcacccatctgggtgcggggccaccactgtccaacggccaccgccccgctgcccatgacttccctctgggcaggcagctgcccagcaggaccacccctacgctgggcctggaggaggtcctgtcctccagggactgccacccggccctgcccctgcccccggggttccacccccaccccggacccaactaccccagcttcctgcctgaccagatgcagccgcaggttccgcccctgcattaccaggagctgatgcccccgggcagctgcatgcccgaggagcctaagcctaagcggggccggcgcagctggccccgcaagcggaccgccacccacacttgcgattacgccgggtgcggcaagacctacacaaagagttcgcacctgaaggcccacctgcgaactcacacgggcgagaagccctaccactgcgactgggacgggtgcggctggaagttcgcccggtccgatgagctgacccggcactatcggaagcacaccgggcacaggcccttccagtgccagaagtgtgaccgggccttcagccggtcagaccatctggcactgcacatgaagcgccacttcggaagcggagagggcaggggaagtcttctaacatgcggggacgtggaggaaaatcccggccccatgcccctgaatgtgtccttcaccaaccgcaactatgatctggactatgactctgtgcagccttacttctactgcgatgaggaggagaacttctaccagcagcagcagcagagcgaactgcagccacccgccccatccgaggatatctggaagaagttcgagctgctgccgacccctcctctcagcccctccaggaggagcgggctgtgcagtcccagctacgtggctgtgacccccttctccctgcgcggcgacaacgacggcgggggggggagcttcagcaccgctgaccagctggagatggtcaccgagctgctgggtggcgacatggtcaaccagagcttcatctgcgaccctgatgatgagacattcatcaagaacatcatcatccaggactgcatgtggtccggcttctcggccgctgccaagctggtcagcgagaagctggccagctaccaggccgcccggaaggattccgggtcgcctaaccccgccaggggccacagcgtctgctccacgagcagcctgtacctgcaggatctgagcgccgccgccagcgagtgcatagatccttcagtggtgttcccatacccactgaacgacagcagctctcccaagagctgcgcctcgcaggacagcagcgccttcagcccctcgtccgactcgctgctgtccagcaccgagtcgagcccccagggctctcctgagcccctggtgctgcacgaggagacccctcctaccacctcctcggactccgaggaggagcaggaggatgaggaagagatcgacgtggtcagcgtggagaagcgccaggctcctggcaagcgcagcgagtctggcagcccctccgccgggggccacagcaagcccccgcacagcccgctggtgctgaagcggtgtcacgtgagcacccaccagcataactatgctgcgcctccttccaccaggaaggactaccccgctgccaagcgggtgaagctggatagcgtccgggtgctgaggcagatcagcaataaccgtaagtgcacctcccccaggagcagtgacacagaggagaacgtgaagaggcggactcacaacgttctggagcgccagcgccggaacgagctgaagcggtccttcttcgctctgagggaccagatcccagagctggagaacaatgagaaggcaccgaaggtggtcatcctgaagaaggccaccgcgtatatcctgagcgtgcaggctgaggagcagaagctgatcagcgaggaggacttgctgaggaagcggcgcgagcagctgaaacacaagctggagcagctgcgaaacagctgcgccggaagcggacagtgtactaattatgctctcttgaaattggctggagatgttgagagcaacccaggtcccatgtacaacatgatggagacagagctgaagccccccgggcctcagcagaccagcggcggcggcgggggcaactccaccgccgccgctgctgggggcaaccagaagaacagccccgatagggtgaagcgccctatgaacgccttcatggtgtggtcccgcggccagcgccgtaagatggctcaggagaaccctaagatgcacaactccgagatcagcaagcggctgggcgcggagtggaagctgctgtcggagaccgagaagcggccattcatcgacgaggccaagaggcttcgtgccctgcacatgaaggagcatcctgactacaagtaccggccccgccggaagaccaagacactgatgaagaaggacaagtacaccttgcctgggggcctgctggcccccgggggcaactccatggcttccggcgtgggcgtgggagccggtctaggcgctggcgtgaaccagcgcatggactcctacgctcacatgaacggctggagcaacgggtcctacagcatgatgcaggaccagttgggctacccccagcaccctgggctgaacgcccatggggctgcccagatgcagcccatgcatcggtacgacgtgagtgccctgcagtacaactccatgacatctagccagacctacatgaacgggagtcccacctacagcatgagctatagccagcaggggaccccaggcatggccctggggtccatgggctccgtggtgaagtcggaggccagctcctcacctcccgtggtgacaagctcctcccacagccgggccccctgccaggctggggatctgagggacatgatctccatgtacctcccgggcgccgaggtgcccgagcctgctgctcccagcaggctgcatatgagccagcattaccagtccgggcccgtgcccggcactgccatcaatgggacactgccactgtcccatatgtgatgataaaaaaaacaaaaaacaaaacggctattatgcgttaccggcgatgctcaatgtacctatttctatgggccttgcgccgggaaaccacgcaagggatggtgtcaaattcggcgaaacctaagcgcccgcccgggcgtatggcaacgccgagccaagcttcggcgccaattccatttatcagatttctagag

SEQ ID NO: 63 - DNA, 376 bp, synthetic construct
  source 1..376: mol_type = other DNA
tttactccctatcagtgatagagaacgtatgaagagtttactccctatcagtgatagagaacgtatgcagactttactccctatcagtgatagagaacgtataaggagtttactccctatcagtgatagagaacgtatgaccagtttactccctatcagtgatagagaacgtatctacagtttactccctatcagtgatagagaacgtatatccagtttactccctatcagtgatagagaacgtataagctttaggcgtgtacggtgggcgcctataaaagcagagctcgtttagtgaaccgtcagatcgcctggagcaattccacaacacttttgtcttataccaactttccgtaccacttcctaccctcgtaaa

SEQ ID NO: 64 - DNA, 122 bp, synthetic construct
  source 1..122: mol_type = other DNA
aacttgtttattgcagcttataatggttacaaataaagcaatagcatcacaaatttcacaaataaagcatttttttcactgcattctagttgtggtttgtccaaactcatcaatgtatctta

SEQ ID NO: 65 - DNA, 477 bp, synthetic construct
  source 1..477: mol_type = other DNA
gggtggcatccctgtgacccctccccagtgcctctcctggccctggaagttgccactccagtgcccaccagccttgtcctaataaaattaagttgcatcattttgtctgactaggtgtccttctataatattatggggtggaggggggtggtatggagcaaggggcaagttgggaagacaacctgtagggcctgcggggtctattgggaaccaagctggagtgcagtggcacaatcttggctcactgcaatctccgcctcctgggttcaagcgattctcctgcctcagcctcccgagttgttgggattccaggcatgcatgaccaggctcagctaatttttgtttttttggtagagacggggtttcaccatattggccaggctggtctccaactcctaatctcaggtgatctacccaccttggcctcccaaattgctgggattacaggcgtgaaccactgctcccttccctgtcctt